European Patent Application EP 4 184 168 A1, published May 24, 2023. Title: Probe and method for detecting membrane-associated molecules in living cells. Applicant: Ustav organicke chemie a biochemie AV CR, v. v. i. The sequence listing filed with the application follows.

SEQUENCE LISTING (65 sequences)

SEQ ID NO: 1 - protein, 7 aa, artificial
  linker
GSGGSGG

SEQ ID NO: 2 - protein, 8 aa, artificial
  linker
SSGSSGTG

SEQ ID NO: 3 - protein, 27 aa, artificial
  linker
GSKSSGSGSESKSTGKSTGSGTETGGS

SEQ ID NO: 4 - protein, 6 aa, artificial
  motif
GGVWLG

SEQ ID NO: 5 - protein, 273 aa, artificial
  KB1753-meGFP-GSGGSGG-hRas
MSSRGYYHGIWVGEEGRLSRGKGEELFTGVVPILVELDGDVNGHKFSVSGEGEGDATYGKLTLKFICTTGKLPVPWPTLVTTLTYGVQCFSRYPDHMKRHDFFKSAMPEGYVQERTIFFKDDGNYKTRAEVKFEGDTLVNRIELKGIDFKEDGNILGHKLEYNYNSHNVYIMADKQKNGIKANFKIRHNIESGGVQLADHYQQNTPIGDGPVLLPDNHYLSTQSKLSKDPNEKRDHMVLKERVTAAGITHGMDELYKGSGGSGGCMSCKCVLS

SEQ ID NO: 6 - DNA, 6229 bp, artificial
  KB1753-meGFP- GSGGSGG-hRas-pcDNA3.1+
gacggatcgggagatctcccgatcccctatggtgcactctcagtacaatctgctctgatgccgcatagttaagccagtatctgctccctgcttgtgtgttggaggtcgctgagtagtgcgcgagcaaaatttaagctacaacaaggcaaggcttgaccgacaattgcatgaagaatctgcttagggttaggcgttttgcgctgcttcgcgatgtacgggccagatatacgcgttgacattgattattgactagttattaatagtaatcaattacggggtcattagttcatagcccatatatggagttccgcgttacataacttacggtaaatggcccgcctggctgaccgcccaacgacccccgcccattgacgtcaataatgacgtatgttcccatagtaacgccaatagggactttccattgacgtcaatgggtggagtatttacggtaaactgcccacttggcagtacatcaagtgtatcatatgccaagtacgccccctattgacgtcaatgacggtaaatggcccgcctggcattatgcccagtacatgaccttatgggactttcctacttggcagtacatctacgtattagtcatcgctattaccatggtgatgcggttttggcagtacatcaatgggcgtggatagcggtttgactcacggggatttccaagtctccaccccattgacgtcaatgggagtttgttttggcaccaaaatcaacgggactttccaaaatgtcgtaacaactccgccccattgacgcaaatgggcggtaggcgtgtacggtgggaggtctatataagcagagctctctggctaactagagaacccactgcttactggcttatcgaaattaatacgactcactatagggagacccaagctggctagcggtaccgagctcggatcactagtccagtgtggtggaattcacgcggaccatgtcttctagaggttactaccatggtatttgggtgggtgaagaaggtcgactttctcgaggtaaaggagaagaacttttcactggagttgtcccaattcttgttgaattagatggtgatgttaatgggcacaaattttctgtcagtggagagggtgaaggtgatgcaacatacggaaaacttacccttaaatttatttgcactactggaaaactacctgttccttggccaacacttgtcactactttaacttatggtgttcaatgcttttcaagatacccagatcatatgaaacggcatgactttttcaagagtgccatgcccgaaggttatgtacaggaaagaactatatttttcaaagatgacgggaactacaagacacgtgctgaagtcaagtttgaaggtgatacccttgttaatagaatcgagttaaaaggtattgattttaaagaagatggaaacattcttggacacaaattggaatacaactataactcacacaatgtatacatcatggcagacaaacaaaagaatggaatcaaagctaacttcaaaattagacacaacattgagtccggaggcgttcaactagcagaccattatcaacaaaatactccaattggcgatggccctgtccttttaccagacaaccattacctgtccacacaatctaagctttcgaaagatcccaacgaaaagagagaccacatggtccttaaagagagggtaacagctgctgggattacacatggcatggacgagctgtacaagggatccggtggaagtggaggctgcatgagctgcaagtgtgtgctgtcctaatgagcggccgcactagagggcccgggcccgtttaaacccgctgatcagcctcgactgtgccttctagttgccagccatctgttgtttgcccctcccccgtgccttccttgaccctggaaggtgccactcccactgtcctttcctaataaaatgaggaaattgcatcgcattgtctgagtaggtgtcattctattctggggggtggggtggggcaggacagcaagggggaggattgggaagacaatagcaggcatgctggggatgcggtgggctctatggcttctgaggcggaaagaaccagctggggctctagggggtatccccacgcgccctgtagcggcgcattaagcgcggcgggtgtggtggttacgcgcagcgtgaccgctacacttgccagcgccctagcgcccgctcctttcgctttcttcccttcctttctcgccacgttcgccggctttccccgtcaagctctaaatcgggggctccctttagggttccgatttagtgctttacggcacctcgaccccaaaaaacttgattagggtgatggttcacgtagtgggccatcgccctgatagacggtttttcgccctttgacgttggagtccacgttctttaatagtggactcttgttccaaactggaacaacactcaaccctatctcggtctattcttttgatttataagggattttgccgatttcggcctattggttaaaaaatgagctgatttaacaaaaatttaacgcgaattaattctgtggaatgtgtgtcagttagggtgtggaaagtccccaggctccccagcaggcagaagtatgcaaagcatgcatctcaattagtcagcaaccaggtgtggaaagtccccaggctccccagcaggcagaagtatgcaaagcatgcatctcaattagtcagcaaccatagtcccgcccctaactccgcccatcccgcccctaactccgcccagttccgcccattctccgccccatggctgactaattttttttatttatgcagaggccgaggccgcctctgcctctgagctattccagaagtagtgaggaggcttttttggaggcctaggcttttgcaaaaagctcccgggagcttgtatatccattttcggatctgatcaagagacaggatgaggatcgtttcgcatgattgaacaagatggattgcacgcaggttctccggccgcttgggtggagaggctattcggctatgactgggcacaacagacaatcggctgctctgatgccgccgtgttccggctgtcagcgcaggggcgcccggttctttttgtcaagaccgacctgtccggtgccctgaatgaactgcaggacgaggcagcgcggctatcgtggctggccacgacgggcgttccttgcgcagctgtgctcgacgttgtcactgaagcgggaagggactggctgctattgggcgaagtgccggggcaggatctcctgtcatctcaccttgctcctgccgagaaagtatccatcatggctgatgcaatgcggcggctgcatacgcttgatccggctacctgcccattcgaccaccaagcgaaacatcgcatcgagcgagcacgtactcggatggaagccggtcttgtcgatcaggatgatctggacgaagagcatcaggggctcgcgccagccgaactgttcgccaggctcaaggcgcgcatgcccgacggcgaggatctcgtcgtgacccatggcgatgcctgcttgccgaatatcatggtggaaaatggccgcttttctggattcatcgactgtggccggctgggtgtggcggaccgctatcaggacatagcgttggctacccgtgatattgctgaagagcttggcggcgaatgggctgaccgcttcctcgtgctttacggtatcgccgctcccgattcgcagcgcatcgccttctatcgccttcttgacgagttcttctgagcgggactctggggttcgaaatgaccgaccaagcgacgcccaacctgccatcacgagatttcgattccaccgccgccttctatgaaaggttgggcttcggaatcgttttccgggacgccggctggatgatcctccagcgcggggatctcatgctggagttcttcgcccaccccaacttgtttattgcagcttataatggttacaaataaagcaatagcatcacaaatttcacaaataaagcatttttttcactgcattctagttgtggtttgtccaaactcatcaatgtatcttatcatgtctgtataccgtcgacctctagctagagcttggcgtaatcatggtcatagctgtttcctgtgtgaaattgttatccgctcacaattccacacaacatacgagccggaagcataaagtgtaaagcctggggtgcctaatgagtgagctaactcacattaattgcgttgcgctcactgcccgctttccagtcgggaaacctgtcgtgccagctgcattaatgaatcggccaacgcgcggggagaggcggtttgcgtattgggcgctcttccgcttcctcgctcactgactcgctgcgctcggtcgttcggctgcggcgagcggtatcagctcactcaaaggcggtaatacggttatccacagaatcaggggataacgcaggaaagaacatgtgagcaaaaggccagcaaaaggccaggaaccgtaaaaaggccgcgttgctggcgtttttccataggctccgcccccctgacgagcatcacaaaaatcgacgctcaagtcagaggtggcgaaacccgacaggactataaagataccaggcgtttccccctggaagctccctcgtgcgctctcctgttccgaccctgccgcttaccggatacctgtccgcctttctcccttcgggaagcgtggcgctttctcatagctcacgctgtaggtatctcagttcggtgtaggtcgttcgctccaagctgggctgtgtgcacgaaccccccgttcagcccgaccgctgcgccttatccggtaactatcgtcttgagtccaacccggtaagacacgacttatcgccactggcagcagccactggtaacaggattagcagagcgaggtatgtaggcggtgctacagagttcttgaagtggtggcctaactacggctacactagaagaacagtatttggtatctgcgctctgctgaagccagttaccttcggaaaaagagttggtagctcttgatccggcaaacaaaccaccgctggtagcggtggtttttttgtttgcaagcagcagattacgcgcagaaaaaaaggatctcaagaagatcctttgatcttttctacggggtctgacgctcagtggaacgaaaactcacgttaagggattttggtcatgagattatcaaaaaggatcttcacctagatccttttaaattaaaaatgaagttttaaatcaatctaaagtatatatgagtaaacttggtctgacagttaccaatgcttaatcagtgaggcacctatctcagcgatctgtctatttcgttcatccatagttgcctgactccccgtcgtgtagataactacgatacgggagggcttaccatctggccccagtgctgcaatgataccgcgagacccacgctcaccggctccagatttatcagcaataaaccagccagccggaagggccgagcgcagaagtggtcctgcaactttatccgcctccatccagtctattaattgttgccgggaagctagagtaagtagttcgccagttaatagtttgcgcaacgttgttgccattgctacaggcatcgtggtgtcacgctcgtcgtttggtatggcttcattcagctccggttcccaacgatcaaggcgagttacatgatcccccatgttgtgcaaaaaagcggttagctccttcggtcctccgatcgttgtcagaagtaagttggccgcagtgttatcactcatggttatggcagcactgcataattctcttactgtcatgccatccgtaagatgcttttctgtgactggtgagtactcaaccaagtcattctgagaatagtgtatgcggcgaccgagttgctcttgcccggcgtcaatacgggataataccgcgccacatagcagaactttaaaagtgctcatcattggaaaacgttcttcggggcgaaaactctcaaggatcttaccgctgttgagatccagttcgatgtaacccactcgtgcacccaactgatcttcagcatcttttactttcaccagcgtttctgggtgagcaaaaacaggaaggcaaaatgccgcaaaaaagggaataagggcgacacggaaatgttgaatactcatactcttcctttttcaatattattgaagcatttatcagggttattgtctcatgagcggatacatatttgaatgtatttagaaaaataaacaaataggggttccgcgcacatttccccgaaaagtgccacctgacgtc

SEQ ID NO: 7 - protein, 354 aa, artificial
  G i1(Q204L)
MGCTLSAEDKAAVERSKMIDRNLREDGEKAAREVKLLLLGAGESGKSTIVKQMKIIHEAGYSEEECKQYKAVVYSNTIQSIIAIIRAMGRLKIDFGDSARADDARQLFVLAGAAEEGFMTAELAGVIKRLWKDSGVQACFNRSREYQLNDSAAYYLNDLDRIAQPNYIPTQQDVLRTRVKTTGIVETHFTFKDLHFKMFDVGGLRSERKKWIHCFEGVTAIIFCVALSDYDLVLAEDEEMNRMHESMKLFDSICNNKWFTDTSIILFLNKKDLFEEKIKKSPLTICYPEYAGSNTYEEAAAYIQCQFEDLNKRKDTKEIYTHFTCATDTKNVQFVFDAVTDVIIKNNLKDCGLF

SEQ ID NO: 8 - DNA, 7111 bp, artificial
  Galfa-i1(Q204L)-pcDNA3.1
tagttattaatagtaatcaattacggggtcattagttcatagcccatatatggagttccgcgttacataacttacggtaaatggcccgcctggctgaccgcccaacgacccccgcccattgacgtcaataatgacgtatgttcccatagtaacgccaatagggactttccattgacgtcaatgggtggagtatttacggtaaactgcccacttggcagtacatcaagtgtatcatatgccaagtacgccccctattgacgtcaatgacggtaaatggcccgcctggcattatgcccagtacatgaccttatgggactttcctacttggcagtacatctacgtattagtcatcgctattaccatggtgatgcggttttggcagtacatcaatgggcgtggatagcggtttgactcacggggatttccaagtctccaccccattgacgtcaatgggagtttgttttggcaccaaaatcaacgggactttccaaaatgtcgtaacaactccgccccattgacgcaaatgggcggtaggcgtgtacggtgggaggtctatataagcagagctggtttagtgaaccgtcagatccgctagcctcgacttgagctctctggctaactagagaacccactgcttactggcttatcgaaattaatacgactcactatagggagacccaagctggctagcgtttaaacttaagcttggtaccaccatgggctgcacgctgagcgccgaggacaaggcggcggtggagcggagtaagatgatcgaccgcaacctccgtgaggacggcgagaaggcggcgcgcgaggtcaagctgctgctgctcggtgctggtgaatctggtaaaagtacaattgtgaagcagatgaaaattatccatgaagctggttattcagaagaggagtgtaaacaatacaaagcagtggtctacagtaacaccatccagtcaattattgctatcattagggctatggggaggttgaagatagactttggtgactcagcccgggcggatgatgcacgccaactctttgtgctagctggagctgctgaagaaggctttatgactgcagaacttgctggagttataaagagattgtggaaagatagtggtgtacaagcctgtttcaacagatcccgagagtaccagcttaatgattctgcagcatactatttgaatgacttggacagaatagctcaaccaaattacatcccgactcaacaagatgttctcagaactagagtgaaaactacaggaattgttgaaacccattttactttcaaagatcttcattttaaaatgtttgatgtgggaggtctgagatctgagcggaagaagtggattcattgcttcgaaggagtgacggcgatcatcttctgtgtagcactgagtgactacgacctggttctagctgaagatgaagaaatgaaccgaatgcatgaaagcatgaaattgtttgacagcatatgtaacaacaagtggtttacagatacatccattatactttttctaaacaagaaggatctctttgaagaaaaaatcaaaaagagccctctcactatatgctatccagaatatgcaggatcaaacacatatgaagaggcagctgcatatattcaatgtcagtttgaagacctcaataaaagaaaggacacaaaggaaatatacacccacttcacatgtgccacagatactaagaatgtgcagtttgtttttgatgctgtaacagatgtcatcataaaaaataatctaaaagattgtggtctcttttaactcgagtctagaactagtttgagtcgagccgcggcaattccgcccccccccccccccctctccctcccccccccctaacgttactggccgaagccgcttggaataaggccggtgtgcgtttgtctatatgttattttccaccatattgccgtcttttggcaatgtgagggcccggaaacctggccctgtcttcttgacgagcattcctaggggtctttcccctctcgccaaaggaatgcaaggtctgttgaatgtcgtgaaggaagcagttcctctggaagcttcttgaagacaaacaacgtctgtagcgaccctttgcaggcagcggaaccccccacctggcaacaggtgcctctgcggccaaaagccacgtgtataagatacacctgcaaaggcggcacaaccccagtgccacgttgtgagttggatagttgtggaaagagtcaaatggctctcctcaagcgtattcaacaaggggctgaaggatgcccagaaggtaccccattgtatgggatctgatctggggcctcggtgcacatgctttacatgtgtttagtcgaggttaaaaaaacgtctaggccccccgaaccacggggacgtggttttcctttgaaaaacacgatgataatatggtgagcaagggcgaggaggataacatggccatcatcaaggagttcatgcgcttcaaggtgcacatggagggctccgtgaacggccacgagttcgagatcgagggcgagggcgagggccgcccctacgagggcacccagaccgccaagctgaaggtgaccaagggtggccccctgcccttcgcctgggacatcctgtcccctcagttcatgtacggctccaaggcctacgtgaagcaccccgccgacatccccgactacttgaagctgtccttccccgagggcttcaagtgggagcgcgtgatgaacttcgaggacggcggcgtggtgaccgtgacccaggactcctccctgcaggacggcgagttcatctacaaggtgaagctgcgcggcaccaacttcccctccgacggccccgtaatgcagaagaagaccatgggctgggaggcctcctccgagcggatgtaccccgaggacggcgccctgaagggcgagatcaagcagaggctgaagctgaaggacggcggccactacgacgctgaggtcaagaccacctacaaggccaagaagcccgtgcagctgcccggcgcctacaacgtcaacatcaagttggacatcacctcccacaacgaggactacaccatcgtggaacagtacgaacgcgccgagggccgccactccaccggcggcatggacgagctgtacaagtaaccgcggtcgacggtaccgcgggcccgggatctaagcttatcgataatcaacctctggattacaaaatttgtgaaagattgactggtattcttaactatgttgctccttttacgctatgtggatacgctgctttaatgcctttgtatcatgctattgcttcccgtatggctttcattttctcctccttgtataaatcctggttgctgtctctttatgaggagttgtggcccgttgtcaggcaacgtggcgtggtgtgcactgtgtttgctgacgcaacccccactggttggggcattgccaccacctgtcagctcctttccgggactttcgctttccccctccctattgccacggcggaactcatcgccgcctgccttgcccgctgctggacaggggctcggctgttgggcactgacaattccgtggtgttgtcggggaaatcatcgtcctttccttggctgctcgcctgtgttgccacctggattctgcgcgggacgtccttctgctacgtcccttcggccctcaatccagcggaccttccttcccgcggcctgctgccggctctgcggcctcttccgcgtcttcgccttcgccctcagacgagtcggatctccctttgggccgcctccccgcatcgataccgtggatcgatccaccggatctagataactgatcataatcagccataccacatttgtagaggttttacttgctttaaaaaacctcccacacctccccctgaacctgaaacataaaatgaatgcaattgttgttgttaacttgtttattgcagcttataatggttacaaataaagcaatagcatcacaaatttcacaaataaagcatttttttcactgcattctagttgtggtttgtccaaactcatcaatgtatcttaacgcgtaaattgtaagcgttaatattttgttaaaattcgcgttaaatttttgttaaatcagctcattttttaaccaataggccgaaatcggcaaaatcccttataaatcaaaagaatagaccgagatagggttgagtgttgttccagtttggaacaagagtccactattaaagaacgtggactccaacgtcaaagggcgaaaaaccgtctatcagggcgatggcccactacgtgaaccatcaccctaatcaagttttttggggtcgaggtgccgtaaagcactaaatcggaaccctaaagggagcccccgatttagagcttgacggggaaagccggcgaacgtggcgagaaaggaagggaagaaagcgaaaggagcgggcgctagggcgctggcaagtgtagcggtcacgctgcgcgtaaccaccacacccgccgcgcttaatgcgccgctacagggcgcgtcaggtggcacttttcggggaaatgtgcgcggaacccctatttgtttatttttctaaatacattcaaatatgtatccgctcatgagacaataaccctgataaatgcttcaataatattgaaaaaggaagagtcctgaggcggaaagaaccagctgtggaatgtgtgtcagttagggtgtggaaagtccccaggctccccagcaggcagaagtatgcaaagcatgcatctcaattagtcagcaaccaggtgtggaaagtccccaggctccccagcaggcagaagtatgcaaagcatgcatctcaattagtcagcaaccatagtcccgcccctaactccgcccatcccgcccctaactccgcccagttccgcccattctccgccccatggctgactaattttttttatttatgcagaggccgaggccgcctcggcctctgagctattccagaagtagtgaggaggcttttttggaggcctaggcttttgcaaagatcgatcaagagacaggatgaggatcgtttcgcatgattgaacaagatggattgcacgcaggttctccggccgcttgggtggagaggctattcggctatgactgggcacaacagacaatcggctgctctgatgccgccgtgttccggctgtcagcgcaggggcgcccggttctttttgtcaagaccgacctgtccggtgccctgaatgaactgcaagacgaggcagcgcggctatcgtggctggccacgacgggcgttccttgcgcagctgtgctcgacgttgtcactgaagcgggaagggactggctgctattgggcgaagtgccggggcaggatctcctgtcatctcaccttgctcctgccgagaaagtatccatcatggctgatgcaatgcggcggctgcatacgcttgatccggctacctgcccattcgaccaccaagcgaaacatcgcatcgagcgagcacgtactcggatggaagccggtcttgtcgatcaggatgatctggacgaagagcatcaggggctcgcgccagccgaactgttcgccaggctcaaggcgagcatgcccgacggcgaggatctcgtcgtgacccatggcgatgcctgcttgccgaatatcatggtggaaaatggccgcttttctggattcatcgactgtggccggctgggtgtggcggaccgctatcaggacatagcgttggctacccgtgatattgctgaagagcttggcggcgaatgggctgaccgcttcctcgtgctttacggtatcgccgctcccgattcgcagcgcatcgccttctatcgccttcttgacgagttcttctgagcgggactctggggttcgaaatgaccgaccaagcgacgcccaacctgccatcacgagatttcgattccaccgccgccttctatgaaaggttgggcttcggaatcgttttccgggacgccggctggatgatcctccagcgcggggatctcatgctggagttcttcgcccaccctagggggaggctaactgaaacacggaaggagacaataccggaaggaacccgcgctatgacggcaataaaaagacagaataaaacgcacggtgttgggtcgtttgttcataaacgcggggttcggtcccagggctggcactctgtcgataccccaccgagaccccattggggccaatacgcccgcgtttcttccttttccccaccccaccccccaagttcgggtgaaggcccagggctcgcagccaacgtcggggcggcaggccctgccatagcctcaggttactcatatatactttagattgatttaaaacttcatttttaatttaaaaggatctaggtgaagatcctttttgataatctcatgaccaaaatcccttaacgtgagttttcgttccactgagcgtcagaccccgtagaaaagatcaaaggatcttcttgagatcctttttttctgcgcgtaatctgctgcttgcaaacaaaaaaaccaccgctaccagcggtggtttgtttgccggatcaagagctaccaactctttttccgaaggtaactggcttcagcagagcgcagataccaaatactgtccttctagtgtagccgtagttaggccaccacttcaagaactctgtagcaccgcctacatacctcgctctgctaatcctgttaccagtggctgctgccagtggcgataagtcgtgtcttaccgggttggactcaagacgatagttaccggataaggcgcagcggtcgggctgaacggggggttcgtgcacacagcccagcttggagcgaacgacctacaccgaactgagatacctacagcgtgagctatgagaaagcgccacgcttcccgaagggagaaaggcggacaggtatccggtaagcggcagggtcggaacaggagagcgcacgagggagcttccagggggaaacgcctggtatctttatagtcctgtcgggtttcgccacctctgacttgagcgtcgatttttgtgatgctcgtcaggggggcggagcctatggaaaaacgccagcaacgcggcctttttacggttcctggccttttgctggccttttgctcacatgttctttcctgcgttatcccctgattctgtggataaccgtattaccgccatgcat

SEQ ID NO: 9 - protein, 278 aa, artificial
  KB1753-meGFP-GSGGSGG-kRas
MSSRGYYHGIWVGEEGRLSRGKGEELFTGVVPILVELDGDVNGHKFSVSGEGEGDATYGKLTLKFICTTGKLPVPWPTLVTTLTYGVQCFSRYPDHMKRHDFFKSAMPEGYVQERTIFFKDDGNYKTRAEVKFEGDTLVNRIELKGIDFKEDGNILGHKLEYNYNSHNVYIMADKQKNGIKANFKIRHNIESGGVQLADHYQQNTPIGDGPVLLPDNHYLSTQSKLSKDPNEKRDHMVLKERVTAAGITHGMDELYKGSGGSGGKKKKKKSKTKCVIM

SEQ ID NO: 10 - DNA, 6244 bp, artificial
  KB1753-meGFP-GSGGSGG-kRas
gacggatcgggagatctcccgatcccctatggtgcactctcagtacaatctgctctgatgccgcatagttaagccagtatctgctccctgcttgtgtgttggaggtcgctgagtagtgcgcgagcaaaatttaagctacaacaaggcaaggcttgaccgacaattgcatgaagaatctgcttagggttaggcgttttgcgctgcttcgcgatgtacgggccagatatacgcgttgacattgattattgactagttattaatagtaatcaattacggggtcattagttcatagcccatatatggagttccgcgttacataacttacggtaaatggcccgcctggctgaccgcccaacgacccccgcccattgacgtcaataatgacgtatgttcccatagtaacgccaatagggactttccattgacgtcaatgggtggagtatttacggtaaactgcccacttggcagtacatcaagtgtatcatatgccaagtacgccccctattgacgtcaatgacggtaaatggcccgcctggcattatgcccagtacatgaccttatgggactttcctacttggcagtacatctacgtattagtcatcgctattaccatggtgatgcggttttggcagtacatcaatgggcgtggatagcggtttgactcacggggatttccaagtctccaccccattgacgtcaatgggagtttgttttggcaccaaaatcaacgggactttccaaaatgtcgtaacaactccgccccattgacgcaaatgggcggtaggcgtgtacggtgggaggtctatataagcagagctctctggctaactagagaacccactgcttactggcttatcgaaattaatacgactcactatagggagacccaagctggctagcggtaccgagctcggatcactagtccagtgtggtggaattcacgcggaccatgtcttctagaggttactaccatggtatttgggtgggtgaagaaggtcgactttctcgaggtaaaggagaagaacttttcactggagttgtcccaattcttgttgaattagatggtgatgttaatgggcacaaattttctgtcagtggagagggtgaaggtgatgcaacatacggaaaacttacccttaaatttatttgcactactggaaaactacctgttccttggccaacacttgtcactactttaacttatggtgttcaatgcttttcaagatacccagatcatatgaaacggcatgactttttcaagagtgccatgcccgaaggttatgtacaggaaagaactatatttttcaaagatgacgggaactacaagacacgtgctgaagtcaagtttgaaggtgatacccttgttaatagaatcgagttaaaaggtattgattttaaagaagatggaaacattcttggacacaaattggaatacaactataactcacacaatgtatacatcatggcagacaaacaaaagaatggaatcaaagctaacttcaaaattagacacaacattgagtccggaggcgttcaactagcagaccattatcaacaaaatactccaattggcgatggccctgtccttttaccagacaaccattacctgtccacacaatctaagctttcgaaagatcccaacgaaaagagagaccacatggtccttaaagagagggtaacagctgctgggattacacatggcatggacgagctgtacaagggatccggtggaagtggaggcaagaaaaagaaaaagaagagcaaaactaagtgtgtaatcatgtaatgagcggccgcactagagggcccgggcccgtttaaacccgctgatcagcctcgactgtgccttctagttgccagccatctgttgtttgcccctcccccgtgccttccttgaccctggaaggtgccactcccactgtcctttcctaataaaatgaggaaattgcatcgcattgtctgagtaggtgtcattctattctggggggtggggtggggcaggacagcaagggggaggattgggaagacaatagcaggcatgctggggatgcggtgggctctatggcttctgaggcggaaagaaccagctggggctctagggggtatccccacgcgccctgtagcggcgcattaagcgcggcgggtgtggtggttacgcgcagcgtgaccgctacacttgccagcgccctagcgcccgctcctttcgctttcttcccttcctttctcgccacgttcgccggctttccccgtcaagctctaaatcgggggctccctttagggttccgatttagtgctttacggcacctcgaccccaaaaaacttgattagggtgatggttcacgtagtgggccatcgccctgatagacggtttttcgccctttgacgttggagtccacgttctttaatagtggactcttgttccaaactggaacaacactcaaccctatctcggtctattcttttgatttataagggattttgccgatttcggcctattggttaaaaaatgagctgatttaacaaaaatttaacgcgaattaattctgtggaatgtgtgtcagttagggtgtggaaagtccccaggctccccagcaggcagaagtatgcaaagcatgcatctcaattagtcagcaaccaggtgtggaaagtccccaggctccccagcaggcagaagtatgcaaagcatgcatctcaattagtcagcaaccatagtcccgcccctaactccgcccatcccgcccctaactccgcccagttccgcccattctccgccccatggctgactaattttttttatttatgcagaggccgaggccgcctctgcctctgagctattccagaagtagtgaggaggcttttttggaggcctaggcttttgcaaaaagctcccgggagcttgtatatccattttcggatctgatcaagagacaggatgaggatcgtttcgcatgattgaacaagatggattgcacgcaggttctccggccgcttgggtggagaggctattcggctatgactgggcacaacagacaatcggctgctctgatgccgccgtgttccggctgtcagcgcaggggcgcccggttctttttgtcaagaccgacctgtccggtgccctgaatgaactgcaggacgaggcagcgcggctatcgtggctggccacgacgggcgttccttgcgcagctgtgctcgacgttgtcactgaagcgggaagggactggctgctattgggcgaagtgccggggcaggatctcctgtcatctcaccttgctcctgccgagaaagtatccatcatggctgatgcaatgcggcggctgcatacgcttgatccggctacctgcccattcgaccaccaagcgaaacatcgcatcgagcgagcacgtactcggatggaagccggtcttgtcgatcaggatgatctggacgaagagcatcaggggctcgcgccagccgaactgttcgccaggctcaaggcgcgcatgcccgacggcgaggatctcgtcgtgacccatggcgatgcctgcttgccgaatatcatggtggaaaatggccgcttttctggattcatcgactgtggccggctgggtgtggcggaccgctatcaggacatagcgttggctacccgtgatattgctgaagagcttggcggcgaatgggctgaccgcttcctcgtgctttacggtatcgccgctcccgattcgcagcgcatcgccttctatcgccttcttgacgagttcttctgagcgggactctggggttcgaaatgaccgaccaagcgacgcccaacctgccatcacgagatttcgattccaccgccgccttctatgaaaggttgggcttcggaatcgttttccgggacgccggctggatgatcctccagcgcggggatctcatgctggagttcttcgcccaccccaacttgtttattgcagcttataatggttacaaataaagcaatagcatcacaaatttcacaaataaagcatttttttcactgcattctagttgtggtttgtccaaactcatcaatgtatcttatcatgtctgtataccgtcgacctctagctagagcttggcgtaatcatggtcatagctgtttcctgtgtgaaattgttatccgctcacaattccacacaacatacgagccggaagcataaagtgtaaagcctggggtgcctaatgagtgagctaactcacattaattgcgttgcgctcactgcccgctttccagtcgggaaacctgtcgtgccagctgcattaatgaatcggccaacgcgcggggagaggcggtttgcgtattgggcgctcttccgcttcctcgctcactgactcgctgcgctcggtcgttcggctgcggcgagcggtatcagctcactcaaaggcggtaatacggttatccacagaatcaggggataacgcaggaaagaacatgtgagcaaaaggccagcaaaaggccaggaaccgtaaaaaggccgcgttgctggcgtttttccataggctccgcccccctgacgagcatcacaaaaatcgacgctcaagtcagaggtggcgaaacccgacaggactataaagataccaggcgtttccccctggaagctccctcgtgcgctctcctgttccgaccctgccgcttaccggatacctgtccgcctttctcccttcgggaagcgtggcgctttctcatagctcacgctgtaggtatctcagttcggtgtaggtcgttcgctccaagctgggctgtgtgcacgaaccccccgttcagcccgaccgctgcgccttatccggtaactatcgtcttgagtccaacccggtaagacacgacttatcgccactggcagcagccactggtaacaggattagcagagcgaggtatgtaggcggtgctacagagttcttgaagtggtggcctaactacggctacactagaagaacagtatttggtatctgcgctctgctgaagccagttaccttcggaaaaagagttggtagctcttgatccggcaaacaaaccaccgctggtagcggtggtttttttgtttgcaagcagcagattacgcgcagaaaaaaaggatctcaagaagatcctttgatcttttctacggggtctgacgctcagtggaacgaaaactcacgttaagggattttggtcatgagattatcaaaaaggatcttcacctagatccttttaaattaaaaatgaagttttaaatcaatctaaagtatatatgagtaaacttggtctgacagttaccaatgcttaatcagtgaggcacctatctcagcgatctgtctatttcgttcatccatagttgcctgactccccgtcgtgtagataactacgatacgggagggcttaccatctggccccagtgctgcaatgataccgcgagacccacgctcaccggctccagatttatcagcaataaaccagccagccggaagggccgagcgcagaagtggtcctgcaactttatccgcctccatccagtctattaattgttgccgggaagctagagtaagtagttcgccagttaatagtttgcgcaacgttgttgccattgctacaggcatcgtggtgtcacgctcgtcgtttggtatggcttcattcagctccggttcccaacgatcaaggcgagttacatgatcccccatgttgtgcaaaaaagcggttagctccttcggtcctccgatcgttgtcagaagtaagttggccgcagtgttatcactcatggttatggcagcactgcataattctcttactgtcatgccatccgtaagatgcttttctgtgactggtgagtactcaaccaagtcattctgagaatagtgtatgcggcgaccgagttgctcttgcccggcgtcaatacgggataataccgcgccacatagcagaactttaaaagtgctcatcattggaaaacgttcttcggggcgaaaactctcaaggatcttaccgctgttgagatccagttcgatgtaacccactcgtgcacccaactgatcttcagcatcttttactttcaccagcgtttctgggtgagcaaaaacaggaaggcaaaatgccgcaaaaaagggaataagggcgacacggaaatgttgaatactcatactcttcctttttcaatattattgaagcatttatcagggttattgtctcatgagcggatacatatttgaatgtatttagaaaaataaacaaataggggttccgcgcacatttccccgaaaagtgccacctgacgtc

SEQ ID NO: 11 - protein, 285 aa, artificial
  GAP43-SSGSSGTG-meGFP-KB1753
MLCCMRRTKQVEKNDEDQNSSGSSGTGSKGEELFTGVVPILVELDGDVNGHKFSVSGEGEGDATYGKLTLKFICTTGKLPVPWPTLVTTLTYGVQCFSRYPDHMKRHDFFKSAMPEGYVQERTIFFKDDGNYKTRAEVKFEGDTLVNRIELKGIDFKEDGNILGHKLEYNYNSHNVYIMADKQKNGIKANFKIRHNIESGGVQLADHYQQNTPIGDGPVLLPDNHYLSTQSKLSKDPNEKRDHMVLKERVTAAGITHGMDELYKGSSRGYYHGIWVGEEGRLSRG

SEQ ID NO: 12 - DNA, 6250 bp, artificial
  GAP43-SSGSSGTG-meGFP-KB1753
gacggatcgggagatctcccgatcccctatggtgcactctcagtacaatctgctctgatgccgcatagttaagccagtatctgctccctgcttgtgtgttggaggtcgctgagtagtgcgcgagcaaaatttaagctacaacaaggcaaggcttgaccgacaattgcatgaagaatctgcttagggttaggcgttttgcgctgcttcgcgatgtacgggccagatatacgcgttgacattgattattgactagttattaatagtaatcaattacggggtcattagttcatagcccatatatggagttccgcgttacataacttacggtaaatggcccgcctggctgaccgcccaacgacccccgcccattgacgtcaataatgacgtatgttcccatagtaacgccaatagggactttccattgacgtcaatgggtggagtatttacggtaaactgcccacttggcagtacatcaagtgtatcatatgccaagtacgccccctattgacgtcaatgacggtaaatggcccgcctggcattatgcccagtacatgaccttatgggactttcctacttggcagtacatctacgtattagtcatcgctattaccatggtgatgcggttttggcagtacatcaatgggcgtggatagcggtttgactcacggggatttccaagtctccaccccattgacgtcaatgggagtttgttttggcaccaaaatcaacgggactttccaaaatgtcgtaacaactccgccccattgacgcaaatgggcggtaggcgtgtacggtgggaggtctatataagcagagctctctggctaactagagaacccactgcttactggcttatcgaaattaatacgactcactatagggagacccaagctggctagcgtttaaacttaagcttggtaccgacggaccatgctgtgctgtatgagaagaaccaaacaggttgaaaagaatgatgaggaccagaattcctccggatcgtctggaaccggttctaaaggagaagaacttttcactggagttgtcccaattcttgttgaattagatggtgatgttaatgggcacaaattttctgtcagtggagagggtgaaggtgatgcaacatacggaaaacttacccttaaatttatttgcactactggaaaactacctgttccttggccaacacttgtcactactttaacttatggtgttcaatgcttttcaagatacccagatcatatgaaacggcatgactttttcaagagtgccatgcccgaaggttatgtacaggaaagaactatatttttcaaagatgacgggaactacaagacacgtgctgaagtcaagtttgaaggtgatacccttgttaatagaatcgagttaaaaggtattgattttaaagaagatggaaacattcttggacacaaattggaatacaactataactcacacaatgtatacatcatggcagacaaacaaaagaatggaatcaaagctaacttcaaaattagacacaacattgagtccggaggcgttcaactagcagaccattatcaacaaaatactccaattggcgatggccctgtccttttaccagacaaccattacctgtccacacaatctaagctttcgaaagatcccaacgaaaagagagaccacatggtccttaaagagagggtaacagctgctgggattacacatggcatggacgagctgtacaagggatcctctagaggttactaccatggtatttgggtgggtgaagaaggtcgactttctcgaggataatgaaggtggcggccgctcgaaactagagggcccgtttaaacccgctgatcagcctcgactgtgccttctagttgccagccatctgttgtttgcccctcccccgtgccttccttgaccctggaaggtgccactcccactgtcctttcctaataaaatgaggaaattgcatcgcattgtctgagtaggtgtcattctattctggggggtggggtggggcaggacagcaagggggaggattgggaagacaatagcaggcatgctggggatgcggtgggctctatggcttctgaggcggaaagaaccagctggggctctagggggtatccccacgcgccctgtagcggcgcattaagcgcggcgggtgtggtggttacgcgcagcgtgaccgctacacttgccagcgccctagcgcccgctcctttcgctttcttcccttcctttctcgccacgttcgccggctttccccgtcaagctctaaatcgggggctccctttagggttccgatttagtgctttacggcacctcgaccccaaaaaacttgattagggtgatggttcacgtagtgggccatcgccctgatagacggtttttcgccctttgacgttggagtccacgttctttaatagtggactcttgttccaaactggaacaacactcaaccctatctcggtctattcttttgatttataagggattttgccgatttcggcctattggttaaaaaatgagctgatttaacaaaaatttaacgcgaattaattctgtggaatgtgtgtcagttagggtgtggaaagtccccaggctccccagcaggcagaagtatgcaaagcatgcatctcaattagtcagcaaccaggtgtggaaagtccccaggctccccagcaggcagaagtatgcaaagcatgcatctcaattagtcagcaaccatagtcccgcccctaactccgcccatcccgcccctaactccgcccagttccgcccattctccgccccatggctgactaattttttttatttatgcagaggccgaggccgcctctgcctctgagctattccagaagtagtgaggaggcttttttggaggcctaggcttttgcaaaaagctcccgggagcttgtatatccattttcggatctgatcaagagacaggatgaggatcgtttcgcatgattgaacaagatggattgcacgcaggttctccggccgcttgggtggagaggctattcggctatgactgggcacaacagacaatcggctgctctgatgccgccgtgttccggctgtcagcgcaggggcgcccggttctttttgtcaagaccgacctgtccggtgccctgaatgaactgcaggacgaggcagcgcggctatcgtggctggccacgacgggcgttccttgcgcagctgtgctcgacgttgtcactgaagcgggaagggactggctgctattgggcgaagtgccggggcaggatctcctgtcatctcaccttgctcctgccgagaaagtatccatcatggctgatgcaatgcggcggctgcatacgcttgatccggctacctgcccattcgaccaccaagcgaaacatcgcatcgagcgagcacgtactcggatggaagccggtcttgtcgatcaggatgatctggacgaagagcatcaggggctcgcgccagccgaactgttcgccaggctcaaggcgcgcatgcccgacggcgaggatctcgtcgtgacccatggcgatgcctgcttgccgaatatcatggtggaaaatggccgcttttctggattcatcgactgtggccggctgggtgtggcggaccgctatcaggacatagcgttggctacccgtgatattgctgaagagcttggcggcgaatgggctgaccgcttcctcgtgctttacggtatcgccgctcccgattcgcagcgcatcgccttctatcgccttcttgacgagttcttctgagcgggactctggggttcgaaatgaccgaccaagcgacgcccaacctgccatcacgagatttcgattccaccgccgccttctatgaaaggttgggcttcggaatcgttttccgggacgccggctggatgatcctccagcgcggggatctcatgctggagttcttcgcccaccccaacttgtttattgcagcttataatggttacaaataaagcaatagcatcacaaatttcacaaataaagcatttttttcactgcattctagttgtggtttgtccaaactcatcaatgtatcttatcatgtctgtataccgtcgacctctagctagagcttggcgtaatcatggtcatagctgtttcctgtgtgaaattgttatccgctcacaattccacacaacatacgagccggaagcataaagtgtaaagcctggggtgcctaatgagtgagctaactcacattaattgcgttgcgctcactgcccgctttccagtcgggaaacctgtcgtgccagctgcattaatgaatcggccaacgcgcggggagaggcggtttgcgtattgggcgctcttccgcttcctcgctcactgactcgctgcgctcggtcgttcggctgcggcgagcggtatcagctcactcaaaggcggtaatacggttatccacagaatcaggggataacgcaggaaagaacatgtgagcaaaaggccagcaaaaggccaggaaccgtaaaaaggccgcgttgctggcgtttttccataggctccgcccccctgacgagcatcacaaaaatcgacgctcaagtcagaggtggcgaaacccgacaggactataaagataccaggcgtttccccctggaagctccctcgtgcgctctcctgttccgaccctgccgcttaccggatacctgtccgcctttctcccttcgggaagcgtggcgctttctcatagctcacgctgtaggtatctcagttcggtgtaggtcgttcgctccaagctgggctgtgtgcacgaaccccccgttcagcccgaccgctgcgccttatccggtaactatcgtcttgagtccaacccggtaagacacgacttatcgccactggcagcagccactggtaacaggattagcagagcgaggtatgtaggcggtgctacagagttcttgaagtggtggcctaactacggctacactagaagaacagtatttggtatctgcgctctgctgaagccagttaccttcggaaaaagagttggtagctcttgatccggcaaacaaaccaccgctggtagcggtggtttttttgtttgcaagcagcagattacgcgcagaaaaaaaggatctcaagaagatcctttgatcttttctacggggtctgacgctcagtggaacgaaaactcacgttaagggattttggtcatgagattatcaaaaaggatcttcacctagatccttttaaattaaaaatgaagttttaaatcaatctaaagtatatatgagtaaacttggtctgacagttaccaatgcttaatcagtgaggcacctatctcagcgatctgtctatttcgttcatccatagttgcctgactccccgtcgtgtagataactacgatacgggagggcttaccatctggccccagtgctgcaatgataccgcgagacccacgctcaccggctccagatttatcagcaataaaccagccagccggaagggccgagcgcagaagtggtcctgcaactttatccgcctccatccagtctattaattgttgccgggaagctagagtaagtagttcgccagttaatagtttgcgcaacgttgttgccattgctacaggcatcgtggtgtcacgctcgtcgtttggtatggcttcattcagctccggttcccaacgatcaaggcgagttacatgatcccccatgttgtgcaaaaaagcggttagctccttcggtcctccgatcgttgtcagaagtaagttggccgcagtgttatcactcatggttatggcagcactgcataattctcttactgtcatgccatccgtaagatgcttttctgtgactggtgagtactcaaccaagtcattctgagaatagtgtatgcggcgaccgagttgctcttgcccggcgtcaatacgggataataccgcgccacatagcagaactttaaaagtgctcatcattggaaaacgttcttcggggcgaaaactctcaaggatcttaccgctgttgagatccagttcgatgtaacccactcgtgcacccaactgatcttcagcatcttttactttcaccagcgtttctgggtgagcaaaaacaggaaggcaaaatgccgcaaaaaagggaataagggcgacacggaaatgttgaatactcatactcttcctttttcaatattattgaagcatttatcagggttattgtctcatgagcggatacatatttgaatgtatttagaaaaataaacaaataggggttccgcgcacatttccccgaaaagtgccacctgacgtc

SEQ ID NO: 13 - protein, 341 aa, artificial
  IL4R-SSGSSGTG-meGFP-KB1753
MAAGPRTSLLLAFALLCLPWTNGGVAFPAMSSDPDGTDTEQHLLLGVSVSCIVILAVCLLCYVSITVEKNDEDQNSSGSSGTGSKGEELFTGVVPILVELDGDVNGHKFSVSGEGEGDATYGKLTLKFICTTGKLPVPWPTLVTTLTYGVQCFSRYPDHMKRHDFFKSAMPEGYVQERTIFFKDDGNYKTRAEVKFEGDTLVNRIELKGIDFKEDGNILGHKLEYNYNSHNVYIMADKQKNGIKANFKIRHNIESGGVQLADHYQQNTPIGDGPVLLPDNHYLSTQSKLSKDPNEKRDHMVLKERVTAAGITHGMDELYKGSSRGYYHGIWVGEEGRLSRG

SEQ ID NO: 14 - DNA, 6418 bp, artificial
  IL4R-SSGSSGTG-meGFP-KB1753
gacggatcgggagatctcccgatcccctatggtgcactctcagtacaatctgctctgatgccgcatagttaagccagtatctgctccctgcttgtgtgttggaggtcgctgagtagtgcgcgagcaaaatttaagctacaacaaggcaaggcttgaccgacaattgcatgaagaatctgcttagggttaggcgttttgcgctgcttcgcgatgtacgggccagatatacgcgttgacattgattattgactagttattaatagtaatcaattacggggtcattagttcatagcccatatatggagttccgcgttacataacttacggtaaatggcccgcctggctgaccgcccaacgacccccgcccattgacgtcaataatgacgtatgttcccatagtaacgccaatagggactttccattgacgtcaatgggtggagtatttacggtaaactgcccacttggcagtacatcaagtgtatcatatgccaagtacgccccctattgacgtcaatgacggtaaatggcccgcctggcattatgcccagtacatgaccttatgggactttcctacttggcagtacatctacgtattagtcatcgctattaccatggtgatgcggttttggcagtacatcaatgggcgtggatagcggtttgactcacggggatttccaagtctccaccccattgacgtcaatgggagtttgttttggcaccaaaatcaacgggactttccaaaatgtcgtaacaactccgccccattgacgcaaatgggcggtaggcgtgtacggtgggaggtctatataagcagagctctctggctaactagagaacccactgcttactggcttatcgaaattaatacgactcactatagggagacccaagctggctagcgtttaaacttaagcttggtaccgacggaccatggccgccggccccaggaccagcctgctgctggccttcgccctgctgtgcctgccctggaccaacggcggcgtggccttccccgccatgagcagcgaccccgacggcaccgacaccgagcagcacctgctgctgggcgtgagcgtgagctgcatcgtgatcctggccgtgtgcctgctgtgctacgtgagcatcaccgtggagaagaacgacgaggaccagaattcctccggatcgtctggaaccggttctaaaggagaagaacttttcactggagttgtcccaattcttgttgaattagatggtgatgttaatgggcacaaattttctgtcagtggagagggtgaaggtgatgcaacatacggaaaacttacccttaaatttatttgcactactggaaaactacctgttccttggccaacacttgtcactactttaacttatggtgttcaatgcttttcaagatacccagatcatatgaaacggcatgactttttcaagagtgccatgcccgaaggttatgtacaggaaagaactatatttttcaaagatgacgggaactacaagacacgtgctgaagtcaagtttgaaggtgatacccttgttaatagaatcgagttaaaaggtattgattttaaagaagatggaaacattcttggacacaaattggaatacaactataactcacacaatgtatacatcatggcagacaaacaaaagaatggaatcaaagctaacttcaaaattagacacaacattgagtccggaggcgttcaactagcagaccattatcaacaaaatactccaattggcgatggccctgtccttttaccagacaaccattacctgtccacacaatctaagctttcgaaagatcccaacgaaaagagagaccacatggtccttaaagagagggtaacagctgctgggattacacatggcatggacgagctgtacaagggatcctctagaggttactaccatggtatttgggtgggtgaagaaggtcgactttctcgaggataatgaaggtggcggccgctcgaaactagagggcccgtttaaacccgctgatcagcctcgactgtgccttctagttgccagccatctgttgtttgcccctcccccgtgccttccttgaccctggaaggtgccactcccactgtcctttcctaataaaatgaggaaattgcatcgcattgtctgagtaggtgtcattctattctggggggtggggtggggcaggacagcaagggggaggattgggaagacaatagcaggcatgctggggatgcggtgggctctatggcttctgaggcggaaagaaccagctggggctctagggggtatccccacgcgccctgtagcggcgcattaagcgcggcgggtgtggtggttacgcgcagcgtgaccgctacacttgccagcgccctagcgcccgctcctttcgctttcttcccttcctttctcgccacgttcgccggctttccccgtcaagctctaaatcgggggctccctttagggttccgatttagtgctttacggcacctcgaccccaaaaaacttgattagggtgatggttcacgtagtgggccatcgccctgatagacggtttttcgccctttgacgttggagtccacgttctttaatagtggactcttgttccaaactggaacaacactcaaccctatctcggtctattcttttgatttataagggattttgccgatttcggcctattggttaaaaaatgagctgatttaacaaaaatttaacgcgaattaattctgtggaatgtgtgtcagttagggtgtggaaagtccccaggctccccagcaggcagaagtatgcaaagcatgcatctcaattagtcagcaaccaggtgtggaaagtccccaggctccccagcaggcagaagtatgcaaagcatgcatctcaattagtcagcaaccatagtcccgcccctaactccgcccatcccgcccctaactccgcccagttccgcccattctccgccccatggctgactaattttttttatttatgcagaggccgaggccgcctctgcctctgagctattccagaagtagtgaggaggcttttttggaggcctaggcttttgcaaaaagctcccgggagcttgtatatccattttcggatctgatcaagagacaggatgaggatcgtttcgcatgattgaacaagatggattgcacgcaggttctccggccgcttgggtggagaggctattcggctatgactgggcacaacagacaatcggctgctctgatgccgccgtgttccggctgtcagcgcaggggcgcccggttctttttgtcaagaccgacctgtccggtgccctgaatgaactgcaggacgaggcagcgcggctatcgtggctggccacgacgggcgttccttgcgcagctgtgctcgacgttgtcactgaagcgggaagggactggctgctattgggcgaagtgccggggcaggatctcctgtcatctcaccttgctcctgccgagaaagtatccatcatggctgatgcaatgcggcggctgcatacgcttgatccggctacctgcccattcgaccaccaagcgaaacatcgcatcgagcgagcacgtactcggatggaagccggtcttgtcgatcaggatgatctggacgaagagcatcaggggctcgcgccagccgaactgttcgccaggctcaaggcgcgcatgcccgacggcgaggatctcgtcgtgacccatggcgatgcctgcttgccgaatatcatggtggaaaatggccgcttttctggattcatcgactgtggccggctgggtgtggcggaccgctatcaggacatagcgttggctacccgtgatattgctgaagagcttggcggcgaatgggctgaccgcttcctcgtgctttacggtatcgccgctcccgattcgcagcgcatcgccttctatcgccttcttgacgagttcttctgagcgggactctggggttcgaaatgaccgaccaagcgacgcccaacctgccatcacgagatttcgattccaccgccgccttctatgaaaggttgggcttcggaatcgttttccgggacgccggctggatgatcctccagcgcggggatctcatgctggagttcttcgcccaccccaacttgtttattgcagcttataatggttacaaataaagcaatagcatcacaaatttcacaaataaagcatttttttcactgcattctagttgtggtttgtccaaactcatcaatgtatcttatcatgtctgtataccgtcgacctctagctagagcttggcgtaatcatggtcatagctgtttcctgtgtgaaattgttatccgctcacaattccacacaacatacgagccggaagcataaagtgtaaagcctggggtgcctaatgagtgagctaactcacattaattgcgttgcgctcactgcccgctttccagtcgggaaacctgtcgtgccagctgcattaatgaatcggccaacgcgcggggagaggcggtttgcgtattgggcgctcttccgcttcctcgctcactgactcgctgcgctcggtcgttcggctgcggcgagcggtatcagctcactcaaaggcggtaatacggttatccacagaatcaggggataacgcaggaaagaacatgtgagcaaaaggccagcaaaaggccaggaaccgtaaaaaggccgcgttgctggcgtttttccataggctccgcccccctgacgagcatcacaaaaatcgacgctcaagtcagaggtggcgaaacccgacaggactataaagataccaggcgtttccccctggaagctccctcgtgcgctctcctgttccgaccctgccgcttaccggatacctgtccgcctttctcccttcgggaagcgtggcgctttctcatagctcacgctgtaggtatctcagttcggtgtaggtcgttcgctccaagctgggctgtgtgcacgaaccccccgttcagcccgaccgctgcgccttatccggtaactatcgtcttgagtccaacccggtaagacacgacttatcgccactggcagcagccactggtaacaggattagcagagcgaggtatgtaggcggtgctacagagttcttgaagtggtggcctaactacggctacactagaagaacagtatttggtatctgcgctctgctgaagccagttaccttcggaaaaagagttggtagctcttgatccggcaaacaaaccaccgctggtagcggtggtttttttgtttgcaagcagcagattacgcgcagaaaaaaaggatctcaagaagatcctttgatcttttctacggggtctgacgctcagtggaacgaaaactcacgttaagggattttggtcatgagattatcaaaaaggatcttcacctagatccttttaaattaaaaatgaagttttaaatcaatctaaagtatatatgagtaaacttggtctgacagttaccaatgcttaatcagtgaggcacctatctcagcgatctgtctatttcgttcatccatagttgcctgactccccgtcgtgtagataactacgatacgggagggcttaccatctggccccagtgctgcaatgataccgcgagacccacgctcaccggctccagatttatcagcaataaaccagccagccggaagggccgagcgcagaagtggtcctgcaactttatccgcctccatccagtctattaattgttgccgggaagctagagtaagtagttcgccagttaatagtttgcgcaacgttgttgccattgctacaggcatcgtggtgtcacgctcgtcgtttggtatggcttcattcagctccggttcccaacgatcaaggcgagttacatgatcccccatgttgtgcaaaaaagcggttagctccttcggtcctccgatcgttgtcagaagtaagttggccgcagtgttatcactcatggttatggcagcactgcataattctcttactgtcatgccatccgtaagatgcttttctgtgactggtgagtactcaaccaagtcattctgagaatagtgtatgcggcgaccgagttgctcttgcccggcgtcaatacgggataataccgcgccacatagcagaactttaaaagtgctcatcattggaaaacgttcttcggggcgaaaactctcaaggatcttaccgctgttgagatccagttcgatgtaacccactcgtgcacccaactgatcttcagcatcttttactttcaccagcgtttctgggtgagcaaaaacaggaaggcaaaatgccgcaaaaaagggaataagggcgacacggaaatgttgaatactcatactcttcctttttcaatattattgaagcatttatcagggttattgtctcatgagcggatacatatttgaatgtatttagaaaaataaacaaataggggttccgcgcacatttccccgaaaagtgccacctgacgtc

SEQ ID NO: 15 - protein, 293 aa, artificial
  KB1753-meGFP-GS24-hRas
MSSRGYYHGIWVGEEGRLSRGKGEELFTGVVPILVELDGDVNGHKFSVSGEGEGDATYGKLTLKFICTTGKLPVPWPTLVTTLTYGVQCFSRYPDHMKRHDFFKSAMPEGYVQERTIFFKDDGNYKTRAEVKFEGDTLVNRIELKGIDFKEDGNILGHKLEYNYNSHNVYIMADKQKNGIKANFKIRHNIESGGVQLADHYQQNTPIGDGPVLLPDNHYLSTQSKLSKDPNEKRDHMVLKERVTAAGITHGMDELYKGSKSSGSGSESKSTGKSTGSGTETGGSCMSCKCVLS

SEQ ID NO: 16 - DNA, 6289 bp, artificial
  KB1753-meGFP-GS24-hRas
gacggatcgggagatctcccgatcccctatggtgcactctcagtacaatctgctctgatgccgcatagttaagccagtatctgctccctgcttgtgtgttggaggtcgctgagtagtgcgcgagcaaaatttaagctacaacaaggcaaggcttgaccgacaattgcatgaagaatctgcttagggttaggcgttttgcgctgcttcgcgatgtacgggccagatatacgcgttgacattgattattgactagttattaatagtaatcaattacggggtcattagttcatagcccatatatggagttccgcgttacataacttacggtaaatggcccgcctggctgaccgcccaacgacccccgcccattgacgtcaataatgacgtatgttcccatagtaacgccaatagggactttccattgacgtcaatgggtggagtatttacggtaaactgcccacttggcagtacatcaagtgtatcatatgccaagtacgccccctattgacgtcaatgacggtaaatggcccgcctggcattatgcccagtacatgaccttatgggactttcctacttggcagtacatctacgtattagtcatcgctattaccatggtgatgcggttttggcagtacatcaatgggcgtggatagcggtttgactcacggggatttccaagtctccaccccattgacgtcaatgggagtttgttttggcaccaaaatcaacgggactttccaaaatgtcgtaacaactccgccccattgacgcaaatgggcggtaggcgtgtacggtgggaggtctatataagcagagctctctggctaactagagaacccactgcttactggcttatcgaaattaatacgactcactatagggagacccaagctggctagcggtaccgagctcggatcactagtccagtgtggtggaattcacgcggaccatgtcttctagaggttactaccatggtatttgggtgggtgaagaaggtcgactttctcgaggtaaaggagaagaacttttcactggagttgtcccaattcttgttgaattagatggtgatgttaatgggcacaaattttctgtcagtggagagggtgaaggtgatgcaacatacggaaaacttacccttaaatttatttgcactactggaaaactacctgttccttggccaacacttgtcactactttaacttatggtgttcaatgcttttcaagatacccagatcatatgaaacggcatgactttttcaagagtgccatgcccgaaggttatgtacaggaaagaactatatttttcaaagatgacgggaactacaagacacgtgctgaagtcaagtttgaaggtgatacccttgttaatagaatcgagttaaaaggtattgattttaaagaagatggaaacattcttggacacaaattggaatacaactataactcacacaatgtatacatcatggcagacaaacaaaagaatggaatcaaagctaacttcaaaattagacacaacattgagtcaggaggcgttcaactagcagaccattatcaacaaaatactccaattggcgatggccctgtccttttaccagacaaccattacctgtccacacaatctaagctttcgaaagatcccaacgaaaagagagaccacatggtccttaaagagagggtaacagctgctgggattacacatggcatggacgagctgtacaagggatccaagtcttccggaagcgggagcgagtctaaatcaacaggcaagagcacaggttccgggaccgagacgggtggatcctgcatgagctgcaagtgtgtgctgtcctaatgagcggccgcactagagggcccgggcccgtttaaacccgctgatcagcctcgactgtgccttctagttgccagccatctgttgtttgcccctcccccgtgccttccttgaccctggaaggtgccactcccactgtcctttcctaataaaatgaggaaattgcatcgcattgtctgagtaggtgtcattctattctggggggtggggtggggcaggacagcaagggggaggattgggaagacaatagcaggcatgctggggatgcggtgggctctatggcttctgaggcggaaagaaccagctggggctctagggggtatccccacgcgccctgtagcggcgcattaagcgcggcgggtgtggtggttacgcgcagcgtgaccgctacacttgccagcgccctagcgcccgctcctttcgctttcttcccttcctttctcgccacgttcgccggctttccccgtcaagctctaaatcgggggctccctttagggttccgatttagtgctttacggcacctcgaccccaaaaaacttgattagggtgatggttcacgtagtgggccatcgccctgatagacggtttttcgccctttgacgttggagtccacgttctttaatagtggactcttgttccaaactggaacaacactcaaccctatctcggtctattcttttgatttataagggattttgccgatttcggcctattggttaaaaaatgagctgatttaacaaaaatttaacgcgaattaattctgtggaatgtgtgtcagttagggtgtggaaagtccccaggctccccagcaggcagaagtatgcaaagcatgcatctcaattagtcagcaaccaggtgtggaaagtccccaggctccccagcaggcagaagtatgcaaagcatgcatctcaattagtcagcaaccatagtcccgcccctaactccgcccatcccgcccctaactccgcccagttccgcccattctccgccccatggctgactaattttttttatttatgcagaggccgaggccgcctctgcctctgagctattccagaagtagtgaggaggcttttttggaggcctaggcttttgcaaaaagctcccgggagcttgtatatccattttcggatctgatcaagagacaggatgaggatcgtttcgcatgattgaacaagatggattgcacgcaggttctccggccgcttgggtggagaggctattcggctatgactgggcacaacagacaatcggctgctctgatgccgccgtgttccggctgtcagcgcaggggcgcccggttctttttgtcaagaccgacctgtccggtgccctgaatgaactgcaggacgaggcagcgcggctatcgtggctggccacgacgggcgttccttgcgcagctgtgctcgacgttgtcactgaagcgggaagggactggctgctattgggcgaagtgccggggcaggatctcctgtcatctcaccttgctcctgccgagaaagtatccatcatggctgatgcaatgcggcggctgcatacgcttgatccggctacctgcccattcgaccaccaagcgaaacatcgcatcgagcgagcacgtactcggatggaagccggtcttgtcgatcaggatgatctggacgaagagcatcaggggctcgcgccagccgaactgttcgccaggctcaaggcgcgcatgcccgacggcgaggatctcgtcgtgacccatggcgatgcctgcttgccgaatatcatggtggaaaatggccgcttttctggattcatcgactgtggccggctgggtgtggcggaccgctatcaggacatagcgttggctacccgtgatattgctgaagagcttggcggcgaatgggctgaccgcttcctcgtgctttacggtatcgccgctcccgattcgcagcgcatcgccttctatcgccttcttgacgagttcttctgagcgggactctggggttcgaaatgaccgaccaagcgacgcccaacctgccatcacgagatttcgattccaccgccgccttctatgaaaggttgggcttcggaatcgttttccgggacgccggctggatgatcctccagcgcggggatctcatgctggagttcttcgcccaccccaacttgtttattgcagcttataatggttacaaataaagcaatagcatcacaaatttcacaaataaagcatttttttcactgcattctagttgtggtttgtccaaactcatcaatgtatcttatcatgtctgtataccgtcgacctctagctagagcttggcgtaatcatggtcatagctgtttcctgtgtgaaattgttatccgctcacaattccacacaacatacgagccggaagcataaagtgtaaagcctggggtgcctaatgagtgagctaactcacattaattgcgttgcgctcactgcccgctttccagtcgggaaacctgtcgtgccagctgcattaatgaatcggccaacgcgcggggagaggcggtttgcgtattgggcgctcttccgcttcctcgctcactgactcgctgcgctcggtcgttcggctgcggcgagcggtatcagctcactcaaaggcggtaatacggttatccacagaatcaggggataacgcaggaaagaacatgtgagcaaaaggccagcaaaaggccaggaaccgtaaaaaggccgcgttgctggcgtttttccataggctccgcccccctgacgagcatcacaaaaatcgacgctcaagtcagaggtggcgaaacccgacaggactataaagataccaggcgtttccccctggaagctccctcgtgcgctctcctgttccgaccctgccgcttaccggatacctgtccgcctttctcccttcgggaagcgtggcgctttctcatagctcacgctgtaggtatctcagttcggtgtaggtcgttcgctccaagctgggctgtgtgcacgaaccccccgttcagcccgaccgctgcgccttatccggtaactatcgtcttgagtccaacccggtaagacacgacttatcgccactggcagcagccactggtaacaggattagcagagcgaggtatgtaggcggtgctacagagttcttgaagtggtggcctaactacggctacactagaagaacagtatttggtatctgcgctctgctgaagccagttaccttcggaaaaagagttggtagctcttgatccggcaaacaaaccaccgctggtagcggtggtttttttgtttgcaagcagcagattacgcgcagaaaaaaaggatctcaagaagatcctttgatcttttctacggggtctgacgctcagtggaacgaaaactcacgttaagggattttggtcatgagattatcaaaaaggatcttcacctagatccttttaaattaaaaatgaagttttaaatcaatctaaagtatatatgagtaaacttggtctgacagttaccaatgcttaatcagtgaggcacctatctcagcgatctgtctatttcgttcatccatagttgcctgactccccgtcgtgtagataactacgatacgggagggcttaccatctggccccagtgctgcaatgataccgcgagacccacgctcaccggctccagatttatcagcaataaaccagccagccggaagggccgagcgcagaagtggtcctgcaactttatccgcctccatccagtctattaattgttgccgggaagctagagtaagtagttcgccagttaatagtttgcgcaacgttgttgccattgctacaggcatcgtggtgtcacgctcgtcgtttggtatggcttcattcagctccggttcccaacgatcaaggcgagttacatgatcccccatgttgtgcaaaaaagcggttagctccttcggtcctccgatcgttgtcagaagtaagttggccgcagtgttatcactcatggttatggcagcactgcataattctcttactgtcatgccatccgtaagatgcttttctgtgactggtgagtactcaaccaagtcattctgagaatagtgtatgcggcgaccgagttgctcttgcccggcgtcaatacgggataataccgcgccacatagcagaactttaaaagtgctcatcattggaaaacgttcttcggggcgaaaactctcaaggatcttaccgctgttgagatccagttcgatgtaacccactcgtgcacccaactgatcttcagcatcttttactttcaccagcgtttctgggtgagcaaaaacaggaaggcaaaatgccgcaaaaaagggaataagggcgacacggaaatgttgaatactcatactcttcctttttcaatattattgaagcatttatcagggttattgtctcatgagcggatacatatttgaatgtatttagaaaaataaacaaataggggttccgcgcacatttccccgaaaagtgccacctgacgtc

SEQ ID NO: 17 - protein, 267 aa, artificial
  KB1753-mScarlet-GSGGSGG-hRas
MSSRGYYHGIWVGEEGRLSRVSKGEAVIKEFMRFKVHMEGSMNGHEFEIEGEGEGRPYEGTQTAKLKVTKGGPLPFSWDILSPQFMYGSRAFTKHPADIPDYYKQSFPEGFKWERVMNFEDGGAVTVTQDTSLEDGTLIYKVKLRGTNFPPDGPVMQKKTMGWEASTERLYPEDGVLKGDIKMALRLKDGGRYLADFKTTYKAKKPVQMPGAYNVDRKLDITSHNEDYTVVEQYERSEGRHSTGGMDELYKGSGGSGGCMSCKCVLS

SEQ ID NO: 18 - DNA, 6211 bp, artificial
  KB1753-mScarlet-GSGGSGG-hRas
gacggatcgggagatctcccgatcccctatggtgcactctcagtacaatctgctctgatgccgcatagttaagccagtatctgctccctgcttgtgtgttggaggtcgctgagtagtgcgcgagcaaaatttaagctacaacaaggcaaggcttgaccgacaattgcatgaagaatctgcttagggttaggcgttttgcgctgcttcgcgatgtacgggccagatatacgcgttgacattgattattgactagttattaatagtaatcaattacggggtcattagttcatagcccatatatggagttccgcgttacataacttacggtaaatggcccgcctggctgaccgcccaacgacccccgcccattgacgtcaataatgacgtatgttcccatagtaacgccaatagggactttccattgacgtcaatgggtggagtatttacggtaaactgcccacttggcagtacatcaagtgtatcatatgccaagtacgccccctattgacgtcaatgacggtaaatggcccgcctggcattatgcccagtacatgaccttatgggactttcctacttggcagtacatctacgtattagtcatcgctattaccatggtgatgcggttttggcagtacatcaatgggcgtggatagcggtttgactcacggggatttccaagtctccaccccattgacgtcaatgggagtttgttttggcaccaaaatcaacgggactttccaaaatgtcgtaacaactccgccccattgacgcaaatgggcggtaggcgtgtacggtgggaggtctatataagcagagctctctggctaactagagaacccactgcttactggcttatcgaaattaatacgactcactatagggagacccaagctggctagcggtaccgagctcggatcactagtccagtgtggtggaattcacgcggaccatgtcttctagaggttactaccatggtatttgggtgggtgaagaaggtcgactttctcgagtgagcaagggcgaggcagtgatcaaggagttcatgcggttcaaggtgcacatggagggctccatgaacggccacgagttcgagatcgagggcgagggcgagggccgcccctacgagggcacccagaccgccaagctgaaggtgaccaagggtggccccctgcccttctcctgggacatcctgtcccctcagttcatgtacggctccagggccttcaccaagcaccccgccgacatccccgactactataagcagtccttccccgagggcttcaagtgggagcgcgtgatgaacttcgaggacggcggcgccgtgaccgtgacccaggacacctccctggaggacggcaccctgatctacaaggtgaagctccgcggcaccaacttccctcctgacggccccgtaatgcagaagaagacaatgggctgggaagcgtccaccgagcggttgtaccccgaggacggcgtgctgaagggcgacattaagatggccctgcgcctgaaggacggcggccgctacctggcggacttcaagaccacctacaaggccaagaagcccgtgcagatgcccggcgcctacaacgtcgaccgcaagttggacatcacctcccacaacgaggactacaccgtggtggaacagtacgaacgctccgagggccgccactccaccggcggcatggacgagctgtacaagggatccggtggaagtggaggctgcatgagctgcaagtgtgtgctgtcctaatgagcggccgcactagagggcccgggcccgtttaaacccgctgatcagcctcgactgtgccttctagttgccagccatctgttgtttgcccctcccccgtgccttccttgaccctggaaggtgccactcccactgtcctttcctaataaaatgaggaaattgcatcgcattgtctgagtaggtgtcattctattctggggggtggggtggggcaggacagcaagggggaggattgggaagacaatagcaggcatgctggggatgcggtgggctctatggcttctgaggcggaaagaaccagctggggctctagggggtatccccacgcgccctgtagcggcgcattaagcgcggcgggtgtggtggttacgcgcagcgtgaccgctacacttgccagcgccctagcgcccgctcctttcgctttcttcccttcctttctcgccacgttcgccggctttccccgtcaagctctaaatcgggggctccctttagggttccgatttagtgctttacggcacctcgaccccaaaaaacttgattagggtgatggttcacgtagtgggccatcgccctgatagacggtttttcgccctttgacgttggagtccacgttctttaatagtggactcttgttccaaactggaacaacactcaaccctatctcggtctattcttttgatttataagggattttgccgatttcggcctattggttaaaaaatgagctgatttaacaaaaatttaacgcgaattaattctgtggaatgtgtgtcagttagggtgtggaaagtccccaggctccccagcaggcagaagtatgcaaagcatgcatctcaattagtcagcaaccaggtgtggaaagtccccaggctccccagcaggcagaagtatgcaaagcatgcatctcaattagtcagcaaccatagtcccgcccctaactccgcccatcccgcccctaactccgcccagttccgcccattctccgccccatggctgactaattttttttatttatgcagaggccgaggccgcctctgcctctgagctattccagaagtagtgaggaggcttttttggaggcctaggcttttgcaaaaagctcccgggagcttgtatatccattttcggatctgatcaagagacaggatgaggatcgtttcgcatgattgaacaagatggattgcacgcaggttctccggccgcttgggtggagaggctattcggctatgactgggcacaacagacaatcggctgctctgatgccgccgtgttccggctgtcagcgcaggggcgcccggttctttttgtcaagaccgacctgtccggtgccctgaatgaactgcaggacgaggcagcgcggctatcgtggctggccacgacgggcgttccttgcgcagctgtgctcgacgttgtcactgaagcgggaagggactggctgctattgggcgaagtgccggggcaggatctcctgtcatctcaccttgctcctgccgagaaagtatccatcatggctgatgcaatgcggcggctgcatacgcttgatccggctacctgcccattcgaccaccaagcgaaacatcgcatcgagcgagcacgtactcggatggaagccggtcttgtcgatcaggatgatctggacgaagagcatcaggggctcgcgccagccgaactgttcgccaggctcaaggcgcgcatgcccgacggcgaggatctcgtcgtgacccatggcgatgcctgcttgccgaatatcatggtggaaaatggccgcttttctggattcatcgactgtggccggctgggtgtggcggaccgctatcaggacatagcgttggctacccgtgatattgctgaagagcttggcggcgaatgggctgaccgcttcctcgtgctttacggtatcgccgctcccgattcgcagcgcatcgccttctatcgccttcttgacgagttcttctgagcgggactctggggttcgaaatgaccgaccaagcgacgcccaacctgccatcacgagatttcgattccaccgccgccttctatgaaaggttgggcttcggaatcgttttccgggacgccggctggatgatcctccagcgcggggatctcatgctggagttcttcgcccaccccaacttgtttattgcagcttataatggttacaaataaagcaatagcatcacaaatttcacaaataaagcatttttttcactgcattctagttgtggtttgtccaaactcatcaatgtatcttatcatgtctgtataccgtcgacctctagctagagcttggcgtaatcatggtcatagctgtttcctgtgtgaaattgttatccgctcacaattccacacaacatacgagccggaagcataaagtgtaaagcctggggtgcctaatgagtgagctaactcacattaattgcgttgcgctcactgcccgctttccagtcgggaaacctgtcgtgccagctgcattaatgaatcggccaacgcgcggggagaggcggtttgcgtattgggcgctcttccgcttcctcgctcactgactcgctgcgctcggtcgttcggctgcggcgagcggtatcagctcactcaaaggcggtaatacggttatccacagaatcaggggataacgcaggaaagaacatgtgagcaaaaggccagcaaaaggccaggaaccgtaaaaaggccgcgttgctggcgtttttccataggctccgcccccctgacgagcatcacaaaaatcgacgctcaagtcagaggtggcgaaacccgacaggactataaagataccaggcgtttccccctggaagctccctcgtgcgctctcctgttccgaccctgccgcttaccggatacctgtccgcctttctcccttcgggaagcgtggcgctttctcatagctcacgctgtaggtatctcagttcggtgtaggtcgttcgctccaagctgggctgtgtgcacgaaccccccgttcagcccgaccgctgcgccttatccggtaactatcgtcttgagtccaacccggtaagacacgacttatcgccactggcagcagccactggtaacaggattagcagagcgaggtatgtaggcggtgctacagagttcttgaagtggtggcctaactacggctacactagaagaacagtatttggtatctgcgctctgctgaagccagttaccttcggaaaaagagttggtagctcttgatccggcaaacaaaccaccgctggtagcggtggtttttttgtttgcaagcagcagattacgcgcagaaaaaaaggatctcaagaagatcctttgatcttttctacggggtctgacgctcagtggaacgaaaactcacgttaagggattttggtcatgagattatcaaaaaggatcttcacctagatccttttaaattaaaaatgaagttttaaatcaatctaaagtatatatgagtaaacttggtctgacagttaccaatgcttaatcagtgaggcacctatctcagcgatctgtctatttcgttcatccatagttgcctgactccccgtcgtgtagataactacgatacgggagggcttaccatctggccccagtgctgcaatgataccgcgagacccacgctcaccggctccagatttatcagcaataaaccagccagccggaagggccgagcgcagaagtggtcctgcaactttatccgcctccatccagtctattaattgttgccgggaagctagagtaagtagttcgccagttaatagtttgcgcaacgttgttgccattgctacaggcatcgtggtgtcacgctcgtcgtttggtatggcttcattcagctccggttcccaacgatcaaggcgagttacatgatcccccatgttgtgcaaaaaagcggttagctccttcggtcctccgatcgttgtcagaagtaagttggccgcagtgttatcactcatggttatggcagcactgcataattctcttactgtcatgccatccgtaagatgcttttctgtgactggtgagtactcaaccaagtcattctgagaatagtgtatgcggcgaccgagttgctcttgcccggcgtcaatacgggataataccgcgccacatagcagaactttaaaagtgctcatcattggaaaacgttcttcggggcgaaaactctcaaggatcttaccgctgttgagatccagttcgatgtaacccactcgtgcacccaactgatcttcagcatcttttactttcaccagcgtttctgggtgagcaaaaacaggaaggcaaaatgccgcaaaaaagggaataagggcgacacggaaatgttgaatactcatactcttcctttttcaatattattgaagcatttatcagggttattgtctcatgagcggatacatatttgaatgtatttagaaaaataaacaaataggggttccgcgcacatttccccgaaaagtgccacctgacgtc

SEQ ID NO: 19 - protein, 279 aa, artificial
  KB1753-cpmTurquoise2-GSGGSGG-hRas
MSSRGYYHGIWVGEEGRLSRVPVPWPTLVTTLSWGVQCFARYPDHMKQHDFFKSAMPEGYVQERTISFKDDGTYKTRAEVKFEGDTLVNRIELKGIDFKEDGNILGHKLEYNYFSDNVYITADKQKNGIKANFKIRHNVEDGGVQLADHYQQNTPIGDGPVLLPDNHYLSTQSKLSKDPNEKRDHMVLLEFVTAAGITLGMDELYKGGGSGSKGEELFTGVVPILVELDGDVNGHKFSVRGEGEGDATNGKLTLKFICTTGKLGSGGSGGCMSCKCVLS

SEQ ID NO: 20 - DNA, 6247 bp, artificial
  KB1753-cpmTurquoise2-GSGGSGG-hRas
gacggatcgggagatctcccgatcccctatggtgcactctcagtacaatctgctctgatgccgcatagttaagccagtatctgctccctgcttgtgtgttggaggtcgctgagtagtgcgcgagcaaaatttaagctacaacaaggcaaggcttgaccgacaattgcatgaagaatctgcttagggttaggcgttttgcgctgcttcgcgatgtacgggccagatatacgcgttgacattgattattgactagttattaatagtaatcaattacggggtcattagttcatagcccatatatggagttccgcgttacataacttacggtaaatggcccgcctggctgaccgcccaacgacccccgcccattgacgtcaataatgacgtatgttcccatagtaacgccaatagggactttccattgacgtcaatgggtggagtatttacggtaaactgcccacttggcagtacatcaagtgtatcatatgccaagtacgccccctattgacgtcaatgacggtaaatggcccgcctggcattatgcccagtacatgaccttatgggactttcctacttggcagtacatctacgtattagtcatcgctattaccatggtgatgcggttttggcagtacatcaatgggcgtggatagcggtttgactcacggggatttccaagtctccaccccattgacgtcaatgggagtttgttttggcaccaaaatcaacgggactttccaaaatgtcgtaacaactccgccccattgacgcaaatgggcggtaggcgtgtacggtgggaggtctatataagcagagctctctggctaactagagaacccactgcttactggcttatcgaaattaatacgactcactatagggagacccaagctggctagcggtaccgagctcggatcactagtccagtgtggtggaattcacgcggaccatgtcttctagaggttactaccatggtatttgggtgggtgaagaaggtcgactttctcgagtgccagtgccttggccaaccctcgtgaccaccctgtcctggggcgtgcagtgcttcgcccgctaccccgaccacatgaagcagcacgacttcttcaagtccgccatgcccgaaggctacgtccaggagcgcaccatcagcttcaaggacgacggcacatacaagacccgcgccgaggtgaagttcgagggcgacaccctggtgaaccgcatcgagctgaagggcatcgacttcaaggaggacggcaacatcctggggcacaagctggagtacaactactttagcgacaacgtctatatcaccgccgacaagcagaagaacggcatcaaggccaacttcaagatccgccacaacgtggaggacggcggcgtgcagctcgccgaccactaccagcagaacacccccatcggcgacggccccgtgctgctgcccgacaaccactacctgagcacccagtccaagctgagcaaagaccccaacgagaagcgcgatcacatggtcctgctggagttcgtgaccgccgccgggatcactctcggcatggacgagctgtacaagggcggtggcagcgggagcaagggcgaggagctgttcaccggggtggtgcccatcctggtcgagctggacggcgacgtaaacggccacaagttcagcgtgcgcggcgagggcgagggcgatgccaccaatggcaagctgaccctgaagttcatctgcaccaccggcaagctgggatccggtggaagtggaggctgcatgagctgcaagtgtgtgctgtcctaatgagcggccgcactagagggcccgggcccgtttaaacccgctgatcagcctcgactgtgccttctagttgccagccatctgttgtttgcccctcccccgtgccttccttgaccctggaaggtgccactcccactgtcctttcctaataaaatgaggaaattgcatcgcattgtctgagtaggtgtcattctattctggggggtggggtggggcaggacagcaagggggaggattgggaagacaatagcaggcatgctggggatgcggtgggctctatggcttctgaggcggaaagaaccagctggggctctagggggtatccccacgcgccctgtagcggcgcattaagcgcggcgggtgtggtggttacgcgcagcgtgaccgctacacttgccagcgccctagcgcccgctcctttcgctttcttcccttcctttctcgccacgttcgccggctttccccgtcaagctctaaatcgggggctccctttagggttccgatttagtgctttacggcacctcgaccccaaaaaacttgattagggtgatggttcacgtagtgggccatcgccctgatagacggtttttcgccctttgacgttggagtccacgttctttaatagtggactcttgttccaaactggaacaacactcaaccctatctcggtctattcttttgatttataagggattttgccgatttcggcctattggttaaaaaatgagctgatttaacaaaaatttaacgcgaattaattctgtggaatgtgtgtcagttagggtgtggaaagtccccaggctccccagcaggcagaagtatgcaaagcatgcatctcaattagtcagcaaccaggtgtggaaagtccccaggctccccagcaggcagaagtatgcaaagcatgcatctcaattagtcagcaaccatagtcccgcccctaactccgcccatcccgcccctaactccgcccagttccgcccattctccgccccatggctgactaattttttttatttatgcagaggccgaggccgcctctgcctctgagctattccagaagtagtgaggaggcttttttggaggcctaggcttttgcaaaaagctcccgggagcttgtatatccattttcggatctgatcaagagacaggatgaggatcgtttcgcatgattgaacaagatggattgcacgcaggttctccggccgcttgggtggagaggctattcggctatgactgggcacaacagacaatcggctgctctgatgccgccgtgttccggctgtcagcgcaggggcgcccggttctttttgtcaagaccgacctgtccggtgccctgaatgaactgcaggacgaggcagcgcggctatcgtggctggccacgacgggcgttccttgcgcagctgtgctcgacgttgtcactgaagcgggaagggactggctgctattgggcgaagtgccggggcaggatctcctgtcatctcaccttgctcctgccgagaaagtatccatcatggctgatgcaatgcggcggctgcatacgcttgatccggctacctgcccattcgaccaccaagcgaaacatcgcatcgagcgagcacgtactcggatggaagccggtcttgtcgatcaggatgatctggacgaagagcatcaggggctcgcgccagccgaactgttcgccaggctcaaggcgcgcatgcccgacggcgaggatctcgtcgtgacccatggcgatgcctgcttgccgaatatcatggtggaaaatggccgcttttctggattcatcgactgtggccggctgggtgtggcggaccgctatcaggacatagcgttggctacccgtgatattgctgaagagcttggcggcgaatgggctgaccgcttcctcgtgctttacggtatcgccgctcccgattcgcagcgcatcgccttctatcgccttcttgacgagttcttctgagcgggactctggggttcgaaatgaccgaccaagcgacgcccaacctgccatcacgagatttcgattccaccgccgccttctatgaaaggttgggcttcggaatcgttttccgggacgccggctggatgatcctccagcgcggggatctcatgctggagttcttcgcccaccccaacttgtttattgcagcttataatggttacaaataaagcaatagcatcacaaatttcacaaataaagcatttttttcactgcattctagttgtggtttgtccaaactcatcaatgtatcttatcatgtctgtataccgtcgacctctagctagagcttggcgtaatcatggtcatagctgtttcctgtgtgaaattgttatccgctcacaattccacacaacatacgagccggaagcataaagtgtaaagcctggggtgcctaatgagtgagctaactcacattaattgcgttgcgctcactgcccgctttccagtcgggaaacctgtcgtgccagctgcattaatgaatcggccaacgcgcggggagaggcggtttgcgtattgggcgctcttccgcttcctcgctcactgactcgctgcgctcggtcgttcggctgcggcgagcggtatcagctcactcaaaggcggtaatacggttatccacagaatcaggggataacgcaggaaagaacatgtgagcaaaaggccagcaaaaggccaggaaccgtaaaaaggccgcgttgctggcgtttttccataggctccgcccccctgacgagcatcacaaaaatcgacgctcaagtcagaggtggcgaaacccgacaggactataaagataccaggcgtttccccctggaagctccctcgtgcgctctcctgttccgaccctgccgcttaccggatacctgtccgcctttctcccttcgggaagcgtggcgctttctcatagctcacgctgtaggtatctcagttcggtgtaggtcgttcgctccaagctgggctgtgtgcacgaaccccccgttcagcccgaccgctgcgccttatccggtaactatcgtcttgagtccaacccggtaagacacgacttatcgccactggcagcagccactggtaacaggattagcagagcgaggtatgtaggcggtgctacagagttcttgaagtggtggcctaactacggctacactagaagaacagtatttggtatctgcgctctgctgaagccagttaccttcggaaaaagagttggtagctcttgatccggcaaacaaaccaccgctggtagcggtggtttttttgtttgcaagcagcagattacgcgcagaaaaaaaggatctcaagaagatcctttgatcttttctacggggtctgacgctcagtggaacgaaaactcacgttaagggattttggtcatgagattatcaaaaaggatcttcacctagatccttttaaattaaaaatgaagttttaaatcaatctaaagtatatatgagtaaacttggtctgacagttaccaatgcttaatcagtgaggcacctatctcagcgatctgtctatttcgttcatccatagttgcctgactccccgtcgtgtagataactacgatacgggagggcttaccatctggccccagtgctgcaatgataccgcgagacccacgctcaccggctccagatttatcagcaataaaccagccagccggaagggccgagcgcagaagtggtcctgcaactttatccgcctccatccagtctattaattgttgccgggaagctagagtaagtagttcgccagttaatagtttgcgcaacgttgttgccattgctacaggcatcgtggtgtcacgctcgtcgtttggtatggcttcattcagctccggttcccaacgatcaaggcgagttacatgatcccccatgttgtgcaaaaaagcggttagctccttcggtcctccgatcgttgtcagaagtaagttggccgcagtgttatcactcatggttatggcagcactgcataattctcttactgtcatgccatccgtaagatgcttttctgtgactggtgagtactcaaccaagtcattctgagaatagtgtatgcggcgaccgagttgctcttgcccggcgtcaatacgggataataccgcgccacatagcagaactttaaaagtgctcatcattggaaaacgttcttcggggcgaaaactctcaaggatcttaccgctgttgagatccagttcgatgtaacccactcgtgcacccaactgatcttcagcatcttttactttcaccagcgtttctgggtgagcaaaaacaggaaggcaaaatgccgcaaaaaagggaataagggcgacacggaaatgttgaatactcatactcttcctttttcaatattattgaagcatttatcagggttattgtctcatgagcggatacatatttgaatgtatttagaaaaataaacaaataggggttccgcgcacatttccccgaaaagtgccacctgacgtc

SEQ ID NO: 21 - protein, 332 aa, artificial
  KB1753-HALO-GSGGSGG-hRas
MSSRGYYHGIWVGEEGRLSRAEIGTGFPFDPHYVEVLGERMHYVDVGPRDGTPVLFLHGNPTSSYVWRNIIPHVAPTHRCIAPDLIGMGKSDKPDLGYFFDDHVRFMDAFIEALGLEEVVLVIHDWGSALGFHWAKRNPERVKGIAFMEFIRPIPTWDEWPEFARETFQAFRTTDVGRKLIIDQNVFIEGTLPMGVVRPLTEVEMDHYREPFLNPVDREPLWRFPNELPIAGEPANIVALVEEYMDWLHQSPVPKLLFWGTPGVLIPPAEAARLAKSLPNCKAVDIGPGLNLLQEDNPDLIGSEIARWLSTLEISGGSGGSGGCMSCKCVLS

SEQ ID NO: 22 - DNA, 6406 bp, artificial
  KB1753-HALO-GSGGSGG-hRas
gacggatcgggagatctcccgatcccctatggtgcactctcagtacaatctgctctgatgccgcatagttaagccagtatctgctccctgcttgtgtgttggaggtcgctgagtagtgcgcgagcaaaatttaagctacaacaaggcaaggcttgaccgacaattgcatgaagaatctgcttagggttaggcgttttgcgctgcttcgcgatgtacgggccagatatacgcgttgacattgattattgactagttattaatagtaatcaattacggggtcattagttcatagcccatatatggagttccgcgttacataacttacggtaaatggcccgcctggctgaccgcccaacgacccccgcccattgacgtcaataatgacgtatgttcccatagtaacgccaatagggactttccattgacgtcaatgggtggagtatttacggtaaactgcccacttggcagtacatcaagtgtatcatatgccaagtacgccccctattgacgtcaatgacggtaaatggcccgcctggcattatgcccagtacatgaccttatgggactttcctacttggcagtacatctacgtattagtcatcgctattaccatggtgatgcggttttggcagtacatcaatgggcgtggatagcggtttgactcacggggatttccaagtctccaccccattgacgtcaatgggagtttgttttggcaccaaaatcaacgggactttccaaaatgtcgtaacaactccgccccattgacgcaaatgggcggtaggcgtgtacggtgggaggtctatataagcagagctctctggctaactagagaacccactgcttactggcttatcgaaattaatacgactcactatagggagacccaagctggctagcggtaccgagctcggatcactagtccagtgtggtggaattcacgcggaccatgtcttctagaggttactaccatggtatttgggtgggtgaagaaggtcgactttctcgagcagaaatcggtactggctttccattcgacccccattatgtggaagtcctgggcgagcgcatgcactacgtcgatgttggtccgcgcgatggcacccctgtgctgttcctgcacggtaacccgacctcctcctacgtgtggcgcaacatcatcccgcatgttgcaccgacccatcgctgcattgctccagacctgatcggtatgggcaaatccgacaaaccagacctgggttatttcttcgacgaccacgtccgcttcatggatgccttcatcgaagccctgggtctggaagaggtcgtcctggtcattcacgactggggctccgctctgggtttccactgggccaagcgcaatccagagcgcgtcaaaggtattgcatttatggagttcatccgccctatcccgacctgggacgaatggccagaatttgcccgcgagaccttccaggccttccgcaccaccgacgtcggccgcaagctgatcatcgatcagaacgtttttatcgagggtacgctgccgatgggtgtcgtccgcccgctgactgaagtcgagatggaccattaccgcgagccgttcctgaatcctgttgaccgcgagccactgtggcgcttcccaaacgagctgccaatcgccggtgagccagcgaacatcgtcgcgctggtcgaagaatacatggactggctgcaccagtcccctgtcccgaagctgctgttctggggcaccccaggcgttctgatcccaccggccgaagccgctcgcctggccaaaagcctgcctaactgcaaggctgtggacatcggcccgggtctgaatctgctgcaagaagacaacccggacctgatcggcagcgagatcgcgcgctggctgtcgacgctcgaaatttccggcggatccggtggaagtggaggctgcatgagctgcaagtgtgtgctgtcctaatgagcggccgcactagagggcccgggcccgtttaaacccgctgatcagcctcgactgtgccttctagttgccagccatctgttgtttgcccctcccccgtgccttccttgaccctggaaggtgccactcccactgtcctttcctaataaaatgaggaaattgcatcgcattgtctgagtaggtgtcattctattctggggggtggggtggggcaggacagcaagggggaggattgggaagacaatagcaggcatgctggggatgcggtgggctctatggcttctgaggcggaaagaaccagctggggctctagggggtatccccacgcgccctgtagcggcgcattaagcgcggcgggtgtggtggttacgcgcagcgtgaccgctacacttgccagcgccctagcgcccgctcctttcgctttcttcccttcctttctcgccacgttcgccggctttccccgtcaagctctaaatcgggggctccctttagggttccgatttagtgctttacggcacctcgaccccaaaaaacttgattagggtgatggttcacgtagtgggccatcgccctgatagacggtttttcgccctttgacgttggagtccacgttctttaatagtggactcttgttccaaactggaacaacactcaaccctatctcggtctattcttttgatttataagggattttgccgatttcggcctattggttaaaaaatgagctgatttaacaaaaatttaacgcgaattaattctgtggaatgtgtgtcagttagggtgtggaaagtccccaggctccccagcaggcagaagtatgcaaagcatgcatctcaattagtcagcaaccaggtgtggaaagtccccaggctccccagcaggcagaagtatgcaaagcatgcatctcaattagtcagcaaccatagtcccgcccctaactccgcccatcccgcccctaactccgcccagttccgcccattctccgccccatggctgactaattttttttatttatgcagaggccgaggccgcctctgcctctgagctattccagaagtagtgaggaggcttttttggaggcctaggcttttgcaaaaagctcccgggagcttgtatatccattttcggatctgatcaagagacaggatgaggatcgtttcgcatgattgaacaagatggattgcacgcaggttctccggccgcttgggtggagaggctattcggctatgactgggcacaacagacaatcggctgctctgatgccgccgtgttccggctgtcagcgcaggggcgcccggttctttttgtcaagaccgacctgtccggtgccctgaatgaactgcaggacgaggcagcgcggctatcgtggctggccacgacgggcgttccttgcgcagctgtgctcgacgttgtcactgaagcgggaagggactggctgctattgggcgaagtgccggggcaggatctcctgtcatctcaccttgctcctgccgagaaagtatccatcatggctgatgcaatgcggcggctgcatacgcttgatccggctacctgcccattcgaccaccaagcgaaacatcgcatcgagcgagcacgtactcggatggaagccggtcttgtcgatcaggatgatctggacgaagagcatcaggggctcgcgccagccgaactgttcgccaggctcaaggcgcgcatgcccgacggcgaggatctcgtcgtgacccatggcgatgcctgcttgccgaatatcatggtggaaaatggccgcttttctggattcatcgactgtggccggctgggtgtggcggaccgctatcaggacatagcgttggctacccgtgatattgctgaagagcttggcggcgaatgggctgaccgcttcctcgtgctttacggtatcgccgctcccgattcgcagcgcatcgccttctatcgccttcttgacgagttcttctgagcgggactctggggttcgaaatgaccgaccaagcgacgcccaacctgccatcacgagatttcgattccaccgccgccttctatgaaaggttgggcttcggaatcgttttccgggacgccggctggatgatcctccagcgcggggatctcatgctggagttcttcgcccaccccaacttgtttattgcagcttataatggttacaaataaagcaatagcatcacaaatttcacaaataaagcatttttttcactgcattctagttgtggtttgtccaaactcatcaatgtatcttatcatgtctgtataccgtcgacctctagctagagcttggcgtaatcatggtcatagctgtttcctgtgtgaaattgttatccgctcacaattccacacaacatacgagccggaagcataaagtgtaaagcctggggtgcctaatgagtgagctaactcacattaattgcgttgcgctcactgcccgctttccagtcgggaaacctgtcgtgccagctgcattaatgaatcggccaacgcgcggggagaggcggtttgcgtattgggcgctcttccgcttcctcgctcactgactcgctgcgctcggtcgttcggctgcggcgagcggtatcagctcactcaaaggcggtaatacggttatccacagaatcaggggataacgcaggaaagaacatgtgagcaaaaggccagcaaaaggccaggaaccgtaaaaaggccgcgttgctggcgtttttccataggctccgcccccctgacgagcatcacaaaaatcgacgctcaagtcagaggtggcgaaacccgacaggactataaagataccaggcgtttccccctggaagctccctcgtgcgctctcctgttccgaccctgccgcttaccggatacctgtccgcctttctcccttcgggaagcgtggcgctttctcatagctcacgctgtaggtatctcagttcggtgtaggtcgttcgctccaagctgggctgtgtgcacgaaccccccgttcagcccgaccgctgcgccttatccggtaactatcgtcttgagtccaacccggtaagacacgacttatcgccactggcagcagccactggtaacaggattagcagagcgaggtatgtaggcggtgctacagagttcttgaagtggtggcctaactacggctacactagaagaacagtatttggtatctgcgctctgctgaagccagttaccttcggaaaaagagttggtagctcttgatccggcaaacaaaccaccgctggtagcggtggtttttttgtttgcaagcagcagattacgcgcagaaaaaaaggatctcaagaagatcctttgatcttttctacggggtctgacgctcagtggaacgaaaactcacgttaagggattttggtcatgagattatcaaaaaggatcttcacctagatccttttaaattaaaaatgaagttttaaatcaatctaaagtatatatgagtaaacttggtctgacagttaccaatgcttaatcagtgaggcacctatctcagcgatctgtctatttcgttcatccatagttgcctgactccccgtcgtgtagataactacgatacgggagggcttaccatctggccccagtgctgcaatgataccgcgagacccacgctcaccggctccagatttatcagcaataaaccagccagccggaagggccgagcgcagaagtggtcctgcaactttatccgcctccatccagtctattaattgttgccgggaagctagagtaagtagttcgccagttaatagtttgcgcaacgttgttgccattgctacaggcatcgtggtgtcacgctcgtcgtttggtatggcttcattcagctccggttcccaacgatcaaggcgagttacatgatcccccatgttgtgcaaaaaagcggttagctccttcggtcctccgatcgttgtcagaagtaagttggccgcagtgttatcactcatggttatggcagcactgcataattctcttactgtcatgccatccgtaagatgcttttctgtgactggtgagtactcaaccaagtcattctgagaatagtgtatgcggcgaccgagttgctcttgcccggcgtcaatacgggataataccgcgccacatagcagaactttaaaagtgctcatcattggaaaacgttcttcggggcgaaaactctcaaggatcttaccgctgttgagatccagttcgatgtaacccactcgtgcacccaactgatcttcagcatcttttactttcaccagcgtttctgggtgagcaaaaacaggaaggcaaaatgccgcaaaaaagggaataagggcgacacggaaatgttgaatactcatactcttcctttttcaatattattgaagcatttatcagggttattgtctcatgagcggatacatatttgaatgtatttagaaaaataaacaaataggggttccgcgcacatttccccgaaaagtgccacctgacgtc

SEQ ID NO: 23 - protein, 216 aa, artificial
  KB1753-SNAP-GSGGSGG-hRas
MSSRGYYHGIWVGEEGRLSRDKDCEMKRTTLDSPLGKLELSGCEQGLHRIIFLGKGTSAADAVEVPAPAAVLGGPEPLMQATAWLNAYFHQPEAIEEFPVPALHHPVFQQESFTRQVLWKLLKVVKFGEVISYSHLAALAGNPAATAAVKTALSGNPVPILIPCHRVVQGDLDVGGYEGGLAVKEWLLAHEGHRLGKPGLGSGGSGGCMSCKCVLS

SEQ ID NO: 24 - DNA, 6058 bp, artificial
  KB1753-SNAP-GSGGSGG-hRas
gacggatcgggagatctcccgatcccctatggtgcactctcagtacaatctgctctgatgccgcatagttaagccagtatctgctccctgcttgtgtgttggaggtcgctgagtagtgcgcgagcaaaatttaagctacaacaaggcaaggcttgaccgacaattgcatgaagaatctgcttagggttaggcgttttgcgctgcttcgcgatgtacgggccagatatacgcgttgacattgattattgactagttattaatagtaatcaattacggggtcattagttcatagcccatatatggagttccgcgttacataacttacggtaaatggcccgcctggctgaccgcccaacgacccccgcccattgacgtcaataatgacgtatgttcccatagtaacgccaatagggactttccattgacgtcaatgggtggagtatttacggtaaactgcccacttggcagtacatcaagtgtatcatatgccaagtacgccccctattgacgtcaatgacggtaaatggcccgcctggcattatgcccagtacatgaccttatgggactttcctacttggcagtacatctacgtattagtcatcgctattaccatggtgatgcggttttggcagtacatcaatgggcgtggatagcggtttgactcacggggatttccaagtctccaccccattgacgtcaatgggagtttgttttggcaccaaaatcaacgggactttccaaaatgtcgtaacaactccgccccattgacgcaaatgggcggtaggcgtgtacggtgggaggtctatataagcagagctctctggctaactagagaacccactgcttactggcttatcgaaattaatacgactcactatagggagacccaagctggctagcggtaccgagctcggatcactagtccagtgtggtggaattcacgcggaccatgtcttctagaggttactaccatggtatttgggtgggtgaagaaggtcgactttctcgagacaaagactgcgaaatgaagcgcaccaccctggatagccctctgggcaagctggaactgtctgggtgcgaacagggcctgcaccgtatcatcttcctgggcaaaggaacatctgccgccgacgccgtggaagtgcctgccccagccgccgtgctgggcggaccagagccactgatgcaggccaccgcctggctcaacgcctactttcaccagcctgaggccatcgaggagttccctgtgccagccctgcaccacccagtgttccagcaggagagctttacccgccaggtgctgtggaaactgctgaaagtggtgaagttcggagaggtcatcagctacagccacctggccgccctggccggcaatcccgccgccaccgccgccgtgaaaaccgccctgagcggaaatcccgtgcccattctgatcccctgccaccgggtggtgcagggcgacctggacgtggggggctacgagggcgggctcgccgtgaaagagtggctgctggcccacgagggccacagactgggcaagcctgggctgggatccggtggaagtggaggctgcatgagctgcaagtgtgtgctgtcctaatgagcggccgcactagagggcccgggcccgtttaaacccgctgatcagcctcgactgtgccttctagttgccagccatctgttgtttgcccctcccccgtgccttccttgaccctggaaggtgccactcccactgtcctttcctaataaaatgaggaaattgcatcgcattgtctgagtaggtgtcattctattctggggggtggggtggggcaggacagcaagggggaggattgggaagacaatagcaggcatgctggggatgcggtgggctctatggcttctgaggcggaaagaaccagctggggctctagggggtatccccacgcgccctgtagcggcgcattaagcgcggcgggtgtggtggttacgcgcagcgtgaccgctacacttgccagcgccctagcgcccgctcctttcgctttcttcccttcctttctcgccacgttcgccggctttccccgtcaagctctaaatcgggggctccctttagggttccgatttagtgctttacggcacctcgaccccaaaaaacttgattagggtgatggttcacgtagtgggccatcgccctgatagacggtttttcgccctttgacgttggagtccacgttctttaatagtggactcttgttccaaactggaacaacactcaaccctatctcggtctattcttttgatttataagggattttgccgatttcggcctattggttaaaaaatgagctgatttaacaaaaatttaacgcgaattaattctgtggaatgtgtgtcagttagggtgtggaaagtccccaggctccccagcaggcagaagtatgcaaagcatgcatctcaattagtcagcaaccaggtgtggaaagtccccaggctccccagcaggcagaagtatgcaaagcatgcatctcaattagtcagcaaccatagtcccgcccctaactccgcccatcccgcccctaactccgcccagttccgcccattctccgccccatggctgactaattttttttatttatgcagaggccgaggccgcctctgcctctgagctattccagaagtagtgaggaggcttttttggaggcctaggcttttgcaaaaagctcccgggagcttgtatatccattttcggatctgatcaagagacaggatgaggatcgtttcgcatgattgaacaagatggattgcacgcaggttctccggccgcttgggtggagaggctattcggctatgactgggcacaacagacaatcggctgctctgatgccgccgtgttccggctgtcagcgcaggggcgcccggttctttttgtcaagaccgacctgtccggtgccctgaatgaactgcaggacgaggcagcgcggctatcgtggctggccacgacgggcgttccttgcgcagctgtgctcgacgttgtcactgaagcgggaagggactggctgctattgggcgaagtgccggggcaggatctcctgtcatctcaccttgctcctgccgagaaagtatccatcatggctgatgcaatgcggcggctgcatacgcttgatccggctacctgcccattcgaccaccaagcgaaacatcgcatcgagcgagcacgtactcggatggaagccggtcttgtcgatcaggatgatctggacgaagagcatcaggggctcgcgccagccgaactgttcgccaggctcaaggcgcgcatgcccgacggcgaggatctcgtcgtgacccatggcgatgcctgcttgccgaatatcatggtggaaaatggccgcttttctggattcatcgactgtggccggctgggtgtggcggaccgctatcaggacatagcgttggctacccgtgatattgctgaagagcttggcggcgaatgggctgaccgcttcctcgtgctttacggtatcgccgctcccgattcgcagcgcatcgccttctatcgccttcttgacgagttcttctgagcgggactctggggttcgaaatgaccgaccaagcgacgcccaacctgccatcacgagatttcgattccaccgccgccttctatgaaaggttgggcttcggaatcgttttccgggacgccggctggatgatcctccagcgcggggatctcatgctggagttcttcgcccaccccaacttgtttattgcagcttataatggttacaaataaagcaatagcatcacaaatttcacaaataaagcatttttttcactgcattctagttgtggtttgtccaaactcatcaatgtatcttatcatgtctgtataccgtcgacctctagctagagcttggcgtaatcatggtcatagctgtttcctgtgtgaaattgttatccgctcacaattccacacaacatacgagccggaagcataaagtgtaaagcctggggtgcctaatgagtgagctaactcacattaattgcgttgcgctcactgcccgctttccagtcgggaaacctgtcgtgccagctgcattaatgaatcggccaacgcgcggggagaggcggtttgcgtattgggcgctcttccgcttcctcgctcactgactcgctgcgctcggtcgttcggctgcggcgagcggtatcagctcactcaaaggcggtaatacggttatccacagaatcaggggataacgcaggaaagaacatgtgagcaaaaggccagcaaaaggccaggaaccgtaaaaaggccgcgttgctggcgtttttccataggctccgcccccctgacgagcatcacaaaaatcgacgctcaagtcagaggtggcgaaacccgacaggactataaagataccaggcgtttccccctggaagctccctcgtgcgctctcctgttccgaccctgccgcttaccggatacctgtccgcctttctcccttcgggaagcgtggcgctttctcatagctcacgctgtaggtatctcagttcggtgtaggtcgttcgctccaagctgggctgtgtgcacgaaccccccgttcagcccgaccgctgcgccttatccggtaactatcgtcttgagtccaacccggtaagacacgacttatcgccactggcagcagccactggtaacaggattagcagagcgaggtatgtaggcggtgctacagagttcttgaagtggtggcctaactacggctacactagaagaacagtatttggtatctgcgctctgctgaagccagttaccttcggaaaaagagttggtagctcttgatccggcaaacaaaccaccgctggtagcggtggtttttttgtttgcaagcagcagattacgcgcagaaaaaaaggatctcaagaagatcctttgatcttttctacggggtctgacgctcagtggaacgaaaactcacgttaagggattttggtcatgagattatcaaaaaggatcttcacctagatccttttaaattaaaaatgaagttttaaatcaatctaaagtatatatgagtaaacttggtctgacagttaccaatgcttaatcagtgaggcacctatctcagcgatctgtctatttcgttcatccatagttgcctgactccccgtcgtgtagataactacgatacgggagggcttaccatctggccccagtgctgcaatgataccgcgagacccacgctcaccggctccagatttatcagcaataaaccagccagccggaagggccgagcgcagaagtggtcctgcaactttatccgcctccatccagtctattaattgttgccgggaagctagagtaagtagttcgccagttaatagtttgcgcaacgttgttgccattgctacaggcatcgtggtgtcacgctcgtcgtttggtatggcttcattcagctccggttcccaacgatcaaggcgagttacatgatcccccatgttgtgcaaaaaagcggttagctccttcggtcctccgatcgttgtcagaagtaagttggccgcagtgttatcactcatggttatggcagcactgcataattctcttactgtcatgccatccgtaagatgcttttctgtgactggtgagtactcaaccaagtcattctgagaatagtgtatgcggcgaccgagttgctcttgcccggcgtcaatacgggataataccgcgccacatagcagaactttaaaagtgctcatcattggaaaacgttcttcggggcgaaaactctcaaggatcttaccgctgttgagatccagttcgatgtaacccactcgtgcacccaactgatcttcagcatcttttactttcaccagcgtttctgggtgagcaaaaacaggaaggcaaaatgccgcaaaaaagggaataagggcgacacggaaatgttgaatactcatactcttcctttttcaatattattgaagcatttatcagggttattgtctcatgagcggatacatatttgaatgtatttagaaaaataaacaaataggggttccgcgcacatttccccgaaaagtgccacctgacgtc

SEQ ID NO: 25 - protein, 379 aa, artificial
  NB80-meGFP-GSGGSGG-hRas
MSSRGQVQLQESGGGLVQAGGSLRLSCAASGSIFSINTMGWYRQAPGKQRELVAAIHSGGSTNYANSVKGRFTISRDNAANTVYLQMNSLKPEDTAVYYCNVKDYGAVLYEYDYWGQGTQVTVSSRGKGEELFTGVVPILVELDGDVNGHKFSVSGEGEGDATYGKLTLKFICTTGKLPVPWPTLVTTLTYGVQCFSRYPDHMKRHDFFKSAMPEGYVQERTIFFKDDGNYKTRAEVKFEGDTLVNRIELKGIDFKEDGNILGHKLEYNYNSHNVYIMADKQKNGIKANFKIRHNIESGGVQLADHYQQNTPIGDGPVLLPDNHYLSTQSKLSKDPNEKRDHMVLKERVTAAGITHGMDELYKGSGGSGGCMSCKCVLS

SEQ ID NO: 26 - DNA, 6547 bp, artificial
  NB80-meGFP-GSGGSGG-hRas
gacggatcgggagatctcccgatcccctatggtgcactctcagtacaatctgctctgatgccgcatagttaagccagtatctgctccctgcttgtgtgttggaggtcgctgagtagtgcgcgagcaaaatttaagctacaacaaggcaaggcttgaccgacaattgcatgaagaatctgcttagggttaggcgttttgcgctgcttcgcgatgtacgggccagatatacgcgttgacattgattattgactagttattaatagtaatcaattacggggtcattagttcatagcccatatatggagttccgcgttacataacttacggtaaatggcccgcctggctgaccgcccaacgacccccgcccattgacgtcaataatgacgtatgttcccatagtaacgccaatagggactttccattgacgtcaatgggtggagtatttacggtaaactgcccacttggcagtacatcaagtgtatcatatgccaagtacgccccctattgacgtcaatgacggtaaatggcccgcctggcattatgcccagtacatgaccttatgggactttcctacttggcagtacatctacgtattagtcatcgctattaccatggtgatgcggttttggcagtacatcaatgggcgtggatagcggtttgactcacggggatttccaagtctccaccccattgacgtcaatgggagtttgttttggcaccaaaatcaacgggactttccaaaatgtcgtaacaactccgccccattgacgcaaatgggcggtaggcgtgtacggtgggaggtctatataagcagagctctctggctaactagagaacccactgcttactggcttatcgaaattaatacgactcactatagggagacccaagctggctagcggtaccgagctcggatcactagtccagtgtggtggaattcacgcggaccatgtcttctagaggacaggtgcagctgcaggagtctgggggaggcttggtgcaggctggggggtctctgagactctcctgtgcagcctctggaagcatcttcagtatcaataccatgggctggtaccgccaggctccagggaagcagcgcgagttggtcgcagctattcatagtggtggtagcacaaactatgccaactccgtgaagggccgattcaccatctccagagacaatgccgcgaacacggtgtatctgcaaatgaacagcctgaaacctgaggacacggccgtctattactgtaatgtaaaggactacggggcggtcctatatgagtatgactactggggccaggggacccaggtcaccgtctcctctcgaggtaaaggagaagaacttttcactggagttgtcccaattcttgttgaattagatggtgatgttaatgggcacaaattttctgtcagtggagagggtgaaggtgatgcaacatacggaaaacttacccttaaatttatttgcactactggaaaactacctgttccttggccaacacttgtcactactttaacttatggtgttcaatgcttttcaagatacccagatcatatgaaacggcatgactttttcaagagtgccatgcccgaaggttatgtacaggaaagaactatatttttcaaagatgacgggaactacaagacacgtgctgaagtcaagtttgaaggtgatacccttgttaatagaatcgagttaaaaggtattgattttaaagaagatggaaacattcttggacacaaattggaatacaactataactcacacaatgtatacatcatggcagacaaacaaaagaatggaatcaaagctaacttcaaaattagacacaacattgagtccggaggcgttcaactagcagaccattatcaacaaaatactccaattggcgatggccctgtccttttaccagacaaccattacctgtccacacaatctaagctttcgaaagatcccaacgaaaagagagaccacatggtccttaaagagagggtaacagctgctgggattacacatggcatggacgagctgtacaagggatccggtggaagtggaggctgcatgagctgcaagtgtgtgctgtcctaatgagcggccgcactagagggcccgggcccgtttaaacccgctgatcagcctcgactgtgccttctagttgccagccatctgttgtttgcccctcccccgtgccttccttgaccctggaaggtgccactcccactgtcctttcctaataaaatgaggaaattgcatcgcattgtctgagtaggtgtcattctattctggggggtggggtggggcaggacagcaagggggaggattgggaagacaatagcaggcatgctggggatgcggtgggctctatggcttctgaggcggaaagaaccagctggggctctagggggtatccccacgcgccctgtagcggcgcattaagcgcggcgggtgtggtggttacgcgcagcgtgaccgctacacttgccagcgccctagcgcccgctcctttcgctttcttcccttcctttctcgccacgttcgccggctttccccgtcaagctctaaatcgggggctccctttagggttccgatttagtgctttacggcacctcgaccccaaaaaacttgattagggtgatggttcacgtagtgggccatcgccctgatagacggtttttcgccctttgacgttggagtccacgttctttaatagtggactcttgttccaaactggaacaacactcaaccctatctcggtctattcttttgatttataagggattttgccgatttcggcctattggttaaaaaatgagctgatttaacaaaaatttaacgcgaattaattctgtggaatgtgtgtcagttagggtgtggaaagtccccaggctccccagcaggcagaagtatgcaaagcatgcatctcaattagtcagcaaccaggtgtggaaagtccccaggctccccagcaggcagaagtatgcaaagcatgcatctcaattagtcagcaaccatagtcccgcccctaactccgcccatcccgcccctaactccgcccagttccgcccattctccgccccatggctgactaattttttttatttatgcagaggccgaggccgcctctgcctctgagctattccagaagtagtgaggaggcttttttggaggcctaggcttttgcaaaaagctcccgggagcttgtatatccattttcggatctgatcaagagacaggatgaggatcgtttcgcatgattgaacaagatggattgcacgcaggttctccggccgcttgggtggagaggctattcggctatgactgggcacaacagacaatcggctgctctgatgccgccgtgttccggctgtcagcgcaggggcgcccggttctttttgtcaagaccgacctgtccggtgccctgaatgaactgcaggacgaggcagcgcggctatcgtggctggccacgacgggcgttccttgcgcagctgtgctcgacgttgtcactgaagcgggaagggactggctgctattgggcgaagtgccggggcaggatctcctgtcatctcaccttgctcctgccgagaaagtatccatcatggctgatgcaatgcggcggctgcatacgcttgatccggctacctgcccattcgaccaccaagcgaaacatcgcatcgagcgagcacgtactcggatggaagccggtcttgtcgatcaggatgatctggacgaagagcatcaggggctcgcgccagccgaactgttcgccaggctcaaggcgcgcatgcccgacggcgaggatctcgtcgtgacccatggcgatgcctgcttgccgaatatcatggtggaaaatggccgcttttctggattcatcgactgtggccggctgggtgtggcggaccgctatcaggacatagcgttggctacccgtgatattgctgaagagcttggcggcgaatgggctgaccgcttcctcgtgctttacggtatcgccgctcccgattcgcagcgcatcgccttctatcgccttcttgacgagttcttctgagcgggactctggggttcgaaatgaccgaccaagcgacgcccaacctgccatcacgagatttcgattccaccgccgccttctatgaaaggttgggcttcggaatcgttttccgggacgccggctggatgatcctccagcgcggggatctcatgctggagttcttcgcccaccccaacttgtttattgcagcttataatggttacaaataaagcaatagcatcacaaatttcacaaataaagcatttttttcactgcattctagttgtggtttgtccaaactcatcaatgtatcttatcatgtctgtataccgtcgacctctagctagagcttggcgtaatcatggtcatagctgtttcctgtgtgaaattgttatccgctcacaattccacacaacatacgagccggaagcataaagtgtaaagcctggggtgcctaatgagtgagctaactcacattaattgcgttgcgctcactgcccgctttccagtcgggaaacctgtcgtgccagctgcattaatgaatcggccaacgcgcggggagaggcggtttgcgtattgggcgctcttccgcttcctcgctcactgactcgctgcgctcggtcgttcggctgcggcgagcggtatcagctcactcaaaggcggtaatacggttatccacagaatcaggggataacgcaggaaagaacatgtgagcaaaaggccagcaaaaggccaggaaccgtaaaaaggccgcgttgctggcgtttttccataggctccgcccccctgacgagcatcacaaaaatcgacgctcaagtcagaggtggcgaaacccgacaggactataaagataccaggcgtttccccctggaagctccctcgtgcgctctcctgttccgaccctgccgcttaccggatacctgtccgcctttctcccttcgggaagcgtggcgctttctcatagctcacgctgtaggtatctcagttcggtgtaggtcgttcgctccaagctgggctgtgtgcacgaaccccccgttcagcccgaccgctgcgccttatccggtaactatcgtcttgagtccaacccggtaagacacgacttatcgccactggcagcagccactggtaacaggattagcagagcgaggtatgtaggcggtgctacagagttcttgaagtggtggcctaactacggctacactagaagaacagtatttggtatctgcgctctgctgaagccagttaccttcggaaaaagagttggtagctcttgatccggcaaacaaaccaccgctggtagcggtggtttttttgtttgcaagcagcagattacgcgcagaaaaaaaggatctcaagaagatcctttgatcttttctacggggtctgacgctcagtggaacgaaaactcacgttaagggattttggtcatgagattatcaaaaaggatcttcacctagatccttttaaattaaaaatgaagttttaaatcaatctaaagtatatatgagtaaacttggtctgacagttaccaatgcttaatcagtgaggcacctatctcagcgatctgtctatttcgttcatccatagttgcctgactccccgtcgtgtagataactacgatacgggagggcttaccatctggccccagtgctgcaatgataccgcgagacccacgctcaccggctccagatttatcagcaataaaccagccagccggaagggccgagcgcagaagtggtcctgcaactttatccgcctccatccagtctattaattgttgccgggaagctagagtaagtagttcgccagttaatagtttgcgcaacgttgttgccattgctacaggcatcgtggtgtcacgctcgtcgtttggtatggcttcattcagctccggttcccaacgatcaaggcgagttacatgatcccccatgttgtgcaaaaaagcggttagctccttcggtcctccgatcgttgtcagaagtaagttggccgcagtgttatcactcatggttatggcagcactgcataattctcttactgtcatgccatccgtaagatgcttttctgtgactggtgagtactcaaccaagtcattctgagaatagtgtatgcggcgaccgagttgctcttgcccggcgtcaatacgggataataccgcgccacatagcagaactttaaaagtgctcatcattggaaaacgttcttcggggcgaaaactctcaaggatcttaccgctgttgagatccagttcgatgtaacccactcgtgcacccaactgatcttcagcatcttttactttcaccagcgtttctgggtgagcaaaaacaggaaggcaaaatgccgcaaaaaagggaataagggcgacacggaaatgttgaatactcatactcttcctttttcaatattattgaagcatttatcagggttattgtctcatgagcggatacatatttgaatgtatttagaaaaataaacaaataggggttccgcgcacatttccccgaaaagtgccacctgacgtc

SEQ ID NO: 27 - protein, 413 aa, artificial
  beta2-adrenergic receptor
MGQPGNGSAFLLAPNRSHAPDHDVTQQRDEVWVVGMGIVMSLIVLAIVFGNVLVITAIAKFERLQTVTNYFITSLACADLVMGLAVVPFGAAHILMKMWTFGNFWCEFWTSIDVLCVTASIETLCVIAVDRYFAITSPFKYQSLLTKNKARVIILMVWIVSGLTSFLPIQMHWYRATHQEAINCYANETCCDFFTNQAYAIASSIVSFYVPLVIMVFVYSRVFQEAKRQLQKIDKSEGRFHVQNLSQVEQDGRTGHGLRRSSKFCLKEHKALKTLGIIMGTFTLCWLPFFIVNIVHVIQDNLIRKEVYILLNWIGYVNSGFNPLIYCRSPDFRIAFQELLCLRRSSLKAYGNGYSSNGNTGEQSGYHVEQEKENKLLCEDLPGTEDFVGHQGTVPSDNIDSQGRNCSTNDSLL

SEQ ID NO: 28 - DNA, 7211 bp, artificial
  beta2-adrenergic receptor-IRES-mCherry
tagttattaatagtaatcaattacggggtcattagttcatagcccatatatggagttccgcgttacataacttacggtaaatggcccgcctggctgaccgcccaacgacccccgcccattgacgtcaataatgacgtatgttcccatagtaacgccaatagggactttccattgacgtcaatgggtggagtatttacggtaaactgcccacttggcagtacatcaagtgtatcatatgccaagtacgccccctattgacgtcaatgacggtaaatggcccgcctggcattatgcccagtacatgaccttatgggactttcctacttggcagtacatctacgtattagtcatcgctattaccatggtgatgcggttttggcagtacatcaatgggcgtggatagcggtttgactcacggggatttccaagtctccaccccattgacgtcaatgggagtttgttttggcaccaaaatcaacgggactttccaaaatgtcgtaacaactccgccccattgacgcaaatgggcggtaggcgtgtacggtgggaggtctatataagcagagctggtttagtgaaccgtcagatccgctagcctcgacttgagctcggatccacggtggaattcgattatccaccatggggcaacccgggaacggcagcgccttcttgctggcacccaatagaagccatgcgccggaccacgacgtcacgcagcaaagggacgaggtgtgggtggtgggcatgggcatcgtcatgtctctcatcgtcctggccatcgtgtttggcaatgtgctggtcatcacagccattgccaagttcgagcgtctgcagacggtcaccaactacttcatcacttcactggcctgtgctgatctggtcatgggcctggcagtggtgccctttggggccgcccatattcttatgaaaatgtggacttttggcaacttctggtgcgagttttggacttccattgatgtgctgtgcgtcacggccagcattgagaccctgtgcgtgatcgcagtggatcgctactttgccattacttcacctttcaagtaccagagcctgctgaccaagaataaggcccgggtgatcattctgatggtgtggattgtgtcaggccttacctccttcttgcccattcagatgcactggtaccgggccacccaccaggaagccatcaactgctatgccaatgagacctgctgtgacttcttcacgaaccaagcctatgccattgcctcttccatcgtgtccttctacgttcccctggtgatcatggtcttcgtctactccagggtctttcaggaggccaaaaggcagctccagaagattgacaaatctgagggccgcttccatgtccagaaccttagccaggtggagcaggatgggcggacggggcatggactccgcagatcttccaagttctgcttgaaggagcacaaagccctcaagacgttaggcatcatcatgggcactttcaccctctgctggctgcccttcttcatcgttaacattgtgcatgtgatccaggataacctcatccgtaaggaagtttacatcctcctaaattggataggctatgtcaattctggtttcaatccccttatctactgccggagcccagatttcaggattgccttccaggagcttctgtgcctgcgcaggtcttctttgaaggcctatgggaatggctactccagcaacggcaacacaggggagcagagtggatatcacgtggaacaggagaaagaaaataaactgctgtgtgaagacctcccaggcacggaagactttgtgggccatcaaggtactgtgcctagcgataacattgattcacaagggaggaattgtagtacaaatgactcactgctgtaactcgagtctagaactagtttgagtcgagccgcggcaattccgcccccccccccccccctctccctcccccccccctaacgttactggccgaagccgcttggaataaggccggtgtgcgtttgtctatatgttattttccaccatattgccgtcttttggcaatgtgagggcccggaaacctggccctgtcttcttgacgagcattcctaggggtctttcccctctcgccaaaggaatgcaaggtctgttgaatgtcgtgaaggaagcagttcctctggaagcttcttgaagacaaacaacgtctgtagcgaccctttgcaggcagcggaaccccccacctggcaacaggtgcctctgcggccaaaagccacgtgtataagatacacctgcaaaggcggcacaaccccagtgccacgttgtgagttggatagttgtggaaagagtcaaatggctctcctcaagcgtattcaacaaggggctgaaggatgcccagaaggtaccccattgtatgggatctgatctggggcctcggtgcacatgctttacatgtgtttagtcgaggttaaaaaaacgtctaggccccccgaaccacggggacgtggttttcctttgaaaaacacgatgataatatggtgagcaagggcgaggaggataacatggccatcatcaaggagttcatgcgcttcaaggtgcacatggagggctccgtgaacggccacgagttcgagatcgagggcgagggcgagggccgcccctacgagggcacccagaccgccaagctgaaggtgaccaagggtggccccctgcccttcgcctgggacatcctgtcccctcagttcatgtacggctccaaggcctacgtgaagcaccccgccgacatccccgactacttgaagctgtccttccccgagggcttcaagtgggagcgcgtgatgaacttcgaggacggcggcgtggtgaccgtgacccaggactcctccctgcaggacggcgagttcatctacaaggtgaagctgcgcggcaccaacttcccctccgacggccccgtaatgcagaagaagaccatgggctgggaggcctcctccgagcggatgtaccccgaggacggcgccctgaagggcgagatcaagcagaggctgaagctgaaggacggcggccactacgacgctgaggtcaagaccacctacaaggccaagaagcccgtgcagctgcccggcgcctacaacgtcaacatcaagttggacatcacctcccacaacgaggactacaccatcgtggaacagtacgaacgcgccgagggccgccactccaccggcggcatggacgagctgtacaagtaaccgcggtcgacggtaccgcgggcccgggatctaagcttatcgataatcaacctctggattacaaaatttgtgaaagattgactggtattcttaactatgttgctccttttacgctatgtggatacgctgctttaatgcctttgtatcatgctattgcttcccgtatggctttcattttctcctccttgtataaatcctggttgctgtctctttatgaggagttgtggcccgttgtcaggcaacgtggcgtggtgtgcactgtgtttgctgacgcaacccccactggttggggcattgccaccacctgtcagctcctttccgggactttcgctttccccctccctattgccacggcggaactcatcgccgcctgccttgcccgctgctggacaggggctcggctgttgggcactgacaattccgtggtgttgtcggggaaatcatcgtcctttccttggctgctcgcctgtgttgccacctggattctgcgcgggacgtccttctgctacgtcccttcggccctcaatccagcggaccttccttcccgcggcctgctgccggctctgcggcctcttccgcgtcttcgccttcgccctcagacgagtcggatctccctttgggccgcctccccgcatcgataccgtggatcgatccaccggatctagataactgatcataatcagccataccacatttgtagaggttttacttgctttaaaaaacctcccacacctccccctgaacctgaaacataaaatgaatgcaattgttgttgttaacttgtttattgcagcttataatggttacaaataaagcaatagcatcacaaatttcacaaataaagcatttttttcactgcattctagttgtggtttgtccaaactcatcaatgtatcttaacgcgtaaattgtaagcgttaatattttgttaaaattcgcgttaaatttttgttaaatcagctcattttttaaccaataggccgaaatcggcaaaatcccttataaatcaaaagaatagaccgagatagggttgagtgttgttccagtttggaacaagagtccactattaaagaacgtggactccaacgtcaaagggcgaaaaaccgtctatcagggcgatggcccactacgtgaaccatcaccctaatcaagttttttggggtcgaggtgccgtaaagcactaaatcggaaccctaaagggagcccccgatttagagcttgacggggaaagccggcgaacgtggcgagaaaggaagggaagaaagcgaaaggagcgggcgctagggcgctggcaagtgtagcggtcacgctgcgcgtaaccaccacacccgccgcgcttaatgcgccgctacagggcgcgtcaggtggcacttttcggggaaatgtgcgcggaacccctatttgtttatttttctaaatacattcaaatatgtatccgctcatgagacaataaccctgataaatgcttcaataatattgaaaaaggaagagtcctgaggcggaaagaaccagctgtggaatgtgtgtcagttagggtgtggaaagtccccaggctccccagcaggcagaagtatgcaaagcatgcatctcaattagtcagcaaccaggtgtggaaagtccccaggctccccagcaggcagaagtatgcaaagcatgcatctcaattagtcagcaaccatagtcccgcccctaactccgcccatcccgcccctaactccgcccagttccgcccattctccgccccatggctgactaattttttttatttatgcagaggccgaggccgcctcggcctctgagctattccagaagtagtgaggaggcttttttggaggcctaggcttttgcaaagatcgatcaagagacaggatgaggatcgtttcgcatgattgaacaagatggattgcacgcaggttctccggccgcttgggtggagaggctattcggctatgactgggcacaacagacaatcggctgctctgatgccgccgtgttccggctgtcagcgcaggggcgcccggttctttttgtcaagaccgacctgtccggtgccctgaatgaactgcaagacgaggcagcgcggctatcgtggctggccacgacgggcgttccttgcgcagctgtgctcgacgttgtcactgaagcgggaagggactggctgctattgggcgaagtgccggggcaggatctcctgtcatctcaccttgctcctgccgagaaagtatccatcatggctgatgcaatgcggcggctgcatacgcttgatccggctacctgcccattcgaccaccaagcgaaacatcgcatcgagcgagcacgtactcggatggaagccggtcttgtcgatcaggatgatctggacgaagagcatcaggggctcgcgccagccgaactgttcgccaggctcaaggcgagcatgcccgacggcgaggatctcgtcgtgacccatggcgatgcctgcttgccgaatatcatggtggaaaatggccgcttttctggattcatcgactgtggccggctgggtgtggcggaccgctatcaggacatagcgttggctacccgtgatattgctgaagagcttggcggcgaatgggctgaccgcttcctcgtgctttacggtatcgccgctcccgattcgcagcgcatcgccttctatcgccttcttgacgagttcttctgagcgggactctggggttcgaaatgaccgaccaagcgacgcccaacctgccatcacgagatttcgattccaccgccgccttctatgaaaggttgggcttcggaatcgttttccgggacgccggctggatgatcctccagcgcggggatctcatgctggagttcttcgcccaccctagggggaggctaactgaaacacggaaggagacaataccggaaggaacccgcgctatgacggcaataaaaagacagaataaaacgcacggtgttgggtcgtttgttcataaacgcggggttcggtcccagggctggcactctgtcgataccccaccgagaccccattggggccaatacgcccgcgtttcttccttttccccaccccaccccccaagttcgggtgaaggcccagggctcgcagccaacgtcggggcggcaggccctgccatagcctcaggttactcatatatactttagattgatttaaaacttcatttttaatttaaaaggatctaggtgaagatcctttttgataatctcatgaccaaaatcccttaacgtgagttttcgttccactgagcgtcagaccccgtagaaaagatcaaaggatcttcttgagatcctttttttctgcgcgtaatctgctgcttgcaaacaaaaaaaccaccgctaccagcggtggtttgtttgccggatcaagagctaccaactctttttccgaaggtaactggcttcagcagagcgcagataccaaatactgtccttctagtgtagccgtagttaggccaccacttcaagaactctgtagcaccgcctacatacctcgctctgctaatcctgttaccagtggctgctgccagtggcgataagtcgtgtcttaccgggttggactcaagacgatagttaccggataaggcgcagcggtcgggctgaacggggggttcgtgcacacagcccagcttggagcgaacgacctacaccgaactgagatacctacagcgtgagctatgagaaagcgccacgcttcccgaagggagaaaggcggacaggtatccggtaagcggcagggtcggaacaggagagcgcacgagggagcttccagggggaaacgcctggtatctttatagtcctgtcgggtttcgccacctctgacttgagcgtcgatttttgtgatgctcgtcaggggggcggagcctatggaaaaacgccagcaacgcggcctttttacggttcctggccttttgctggccttttgctcacatgttctttcctgcgttatcccctgattctgtggataaccgtattaccgccatgcat

SEQ ID NO: 29 - protein, 782 aa, artificial
  beta2AR-SSGSSGTG-meGFP-NB80
MGQPGNGSAFLLAPNRSHAPDHDVTQQRDEVWVVGMGIVMSLIVLAIVFGNVLVITAIAKFERLQTVTNYFITSLACADLVMGLAVVPFGAAHILMKMWTFGNFWCEFWTSIDVLCVTASIETLCVIAVDRYFAITSPFKYQSLLTKNKARVIILMVWIVSGLTSFLPIQMHWYRATHQEAINCYANETCCDFFTNQAYAIASSIVSFYVPLVIMVFVYSRVFQEAKRQLQKIDKSEGRFHVQNLSQVEQDGRTGHGLRRSSKFCLKEHKALKTLGIIMGTFTLCWLPFFIVNIVHVIQDNLIRKEVYILLNWIGYVNSGFNPLIYCRSPDFRIAFQELLCLRRSSLKAYGNGYSSNGNTGEQSGYHVEQEKENKLLCEDLPGTEDFVGHQGTVPSDNIDSQGRNCSTNDSLLSSGSSGTGSKGEELFTGVVPILVELDGDVNGHKFSVSGEGEGDATYGKLTLKFICTTGKLPVPWPTLVTTLTYGVQCFSRYPDHMKRHDFFKSAMPEGYVQERTIFFKDDGNYKTRAEVKFEGDTLVNRIELKGIDFKEDGNILGHKLEYNYNSHNVYIMADKQKNGIKANFKIRHNIESGGVQLADHYQQNTPIGDGPVLLPDNHYLSTQSKLSKDPNEKRDHMVLKERVTAAGITHGMDELYKGSSRGQVQLQESGGGLVQAGGSLRLSCAASGSIFSINTMGWYRQAPGKQRELVAAIHSGGSTNYANSVKGRFTISRDNAANTVYLQMNSLKPEDTAVYYCNVKDYGAVLYEYDYWGQGTQVTVS

SEQ ID NO: 30 - DNA, 7750 bp, artificial
  b2AR-SSGSSGTG-meGFP-NB80
gacggatcgggagatctcccgatcccctatggtgcactctcagtacaatctgctctgatgccgcatagttaagccagtatctgctccctgcttgtgtgttggaggtcgctgagtagtgcgcgagcaaaatttaagctacaacaaggcaaggcttgaccgacaattgcatgaagaatctgcttagggttaggcgttttgcgctgcttcgcgatgtacgggccagatatacgcgttgacattgattattgactagttattaatagtaatcaattacggggtcattagttcatagcccatatatggagttccgcgttacataacttacggtaaatggcccgcctggctgaccgcccaacgacccccgcccattgacgtcaataatgacgtatgttcccatagtaacgccaatagggactttccattgacgtcaatgggtggagtatttacggtaaactgcccacttggcagtacatcaagtgtatcatatgccaagtacgccccctattgacgtcaatgacggtaaatggcccgcctggcattatgcccagtacatgaccttatgggactttcctacttggcagtacatctacgtattagtcatcgctattaccatggtgatgcggttttggcagtacatcaatgggcgtggatagcggtttgactcacggggatttccaagtctccaccccattgacgtcaatgggagtttgttttggcaccaaaatcaacgggactttccaaaatgtcgtaacaactccgccccattgacgcaaatgggcggtaggcgtgtacggtgggaggtctatataagcagagctctctggctaactagagaacccactgcttactggcttatcgaaattaatacgactcactatagggagacccaagctggctagcgtttaaacttaagcttggtaccgacggaccatggggcaacccgggaacggcagcgccttcttgctggcacccaatagaagccatgcgccggaccacgacgtcacgcagcaaagggacgaggtgtgggtggtgggcatgggcatcgtcatgtctctcatcgtcctggccatcgtgtttggcaatgtgctggtcatcacagccattgccaagttcgagcgtctgcagacggtcaccaactacttcatcacttcactggcctgtgctgatctggtcatgggcctggcagtggtgccctttggggccgcccatattcttatgaaaatgtggacttttggcaacttctggtgcgagttttggacttccattgatgtgctgtgcgtcacggccagcattgagaccctgtgcgtgatcgcagtggatcgctactttgccattacttcacctttcaagtaccagagcctgctgaccaagaataaggcccgggtgatcattctgatggtgtggattgtgtcaggccttacctccttcttgcccattcagatgcactggtatcgggccacccaccaggaagccatcaactgctatgccaatgagacctgctgtgacttcttcacgaaccaagcctatgccattgcctcttccatcgtgtccttctacgttcccctggtgatcatggtcttcgtctactccagggtctttcaggaggccaaaaggcagctccagaagattgacaaatctgagggccgcttccatgtccagaaccttagccaggtggagcaggatgggcggacggggcatggactccgcagatcttccaagttctgcttgaaggagcacaaagccctcaagacgttaggcatcatcatgggcactttcaccctctgctggctgcccttcttcatcgttaacattgtgcatgtgatccaggataacctcatccgtaaggaagtttacatcctcctaaattggataggctatgtcaattctggtttcaatccccttatctactgccggagcccagatttcaggattgccttccaggagcttctgtgcctgcgcaggtcttctttgaaggcctatgggaatggctactccagcaacggcaacacaggggagcagagtggatatcacgtggaacaggagaaagaaaataaactgctgtgtgaagacctcccaggcacggaagactttgtgggccatcaaggtactgtgcctagcgataacattgattcacaagggaggaattgtagtacaaatgactcactgctgtcctccggatcgtctggaaccggttctaaaggagaagaacttttcactggagttgtcccaattcttgttgaattagatggtgatgttaatgggcacaaattttctgtcagtggagagggtgaaggtgatgcaacatacggaaaacttacccttaaatttatttgcactactggaaaactacctgttccttggccaacacttgtcactactttaacttatggtgttcaatgcttttcaagatacccagatcatatgaaacggcatgactttttcaagagtgccatgcccgaaggttatgtacaggaaagaactatatttttcaaagatgacgggaactacaagacacgtgctgaagtcaagtttgaaggtgatacccttgttaatagaatcgagttaaaaggtattgattttaaagaagatggaaacattcttggacacaaattggaatacaactataactcacacaatgtatacatcatggcagacaaacaaaagaatggaatcaaagctaacttcaaaattagacacaacattgagtccggaggcgttcaactagcagaccattatcaacaaaatactccaattggcgatggccctgtccttttaccagacaaccattacctgtccacacaatctaagctttcgaaagatcccaacgaaaagagagaccacatggtccttaaagagagggtaacagctgctgggattacacatggcatggacgagctgtacaagggatcctctagaggacaggtgcagctgcaggagtctgggggaggcttggtgcaggctggggggtctctgagactctcctgtgcagcctctggaagcatcttcagtatcaataccatgggctggtaccgccaggctccagggaagcagcgcgagttggtcgcagctattcatagtggtggtagcacaaactatgccaactccgtgaagggccgattcaccatctccagagacaatgccgcgaacacggtgtatctgcaaatgaacagcctgaaacctgaggacacggccgtctattactgtaatgtaaaggactacggggcggtcctatatgagtatgactactggggccaggggacccaggtcaccgtctcctctcgaggataatgaaggtggcggccgctcgaaactagagggcccgtttaaacccgctgatcagcctcgactgtgccttctagttgccagccatctgttgtttgcccctcccccgtgccttccttgaccctggaaggtgccactcccactgtcctttcctaataaaatgaggaaattgcatcgcattgtctgagtaggtgtcattctattctggggggtggggtggggcaggacagcaagggggaggattgggaagacaatagcaggcatgctggggatgcggtgggctctatggcttctgaggcggaaagaaccagctggggctctagggggtatccccacgcgccctgtagcggcgcattaagcgcggcgggtgtggtggttacgcgcagcgtgaccgctacacttgccagcgccctagcgcccgctcctttcgctttcttcccttcctttctcgccacgttcgccggctttccccgtcaagctctaaatcgggggctccctttagggttccgatttagtgctttacggcacctcgaccccaaaaaacttgattagggtgatggttcacgtagtgggccatcgccctgatagacggtttttcgccctttgacgttggagtccacgttctttaatagtggactcttgttccaaactggaacaacactcaaccctatctcggtctattcttttgatttataagggattttgccgatttcggcctattggttaaaaaatgagctgatttaacaaaaatttaacgcgaattaattctgtggaatgtgtgtcagttagggtgtggaaagtccccaggctccccagcaggcagaagtatgcaaagcatgcatctcaattagtcagcaaccaggtgtggaaagtccccaggctccccagcaggcagaagtatgcaaagcatgcatctcaattagtcagcaaccatagtcccgcccctaactccgcccatcccgcccctaactccgcccagttccgcccattctccgccccatggctgactaattttttttatttatgcagaggccgaggccgcctctgcctctgagctattccagaagtagtgaggaggcttttttggaggcctaggcttttgcaaaaagctcccgggagcttgtatatccattttcggatctgatcaagagacaggatgaggatcgtttcgcatgattgaacaagatggattgcacgcaggttctccggccgcttgggtggagaggctattcggctatgactgggcacaacagacaatcggctgctctgatgccgccgtgttccggctgtcagcgcaggggcgcccggttctttttgtcaagaccgacctgtccggtgccctgaatgaactgcaggacgaggcagcgcggctatcgtggctggccacgacgggcgttccttgcgcagctgtgctcgacgttgtcactgaagcgggaagggactggctgctattgggcgaagtgccggggcaggatctcctgtcatctcaccttgctcctgccgagaaagtatccatcatggctgatgcaatgcggcggctgcatacgcttgatccggctacctgcccattcgaccaccaagcgaaacatcgcatcgagcgagcacgtactcggatggaagccggtcttgtcgatcaggatgatctggacgaagagcatcaggggctcgcgccagccgaactgttcgccaggctcaaggcgcgcatgcccgacggcgaggatctcgtcgtgacccatggcgatgcctgcttgccgaatatcatggtggaaaatggccgcttttctggattcatcgactgtggccggctgggtgtggcggaccgctatcaggacatagcgttggctacccgtgatattgctgaagagcttggcggcgaatgggctgaccgcttcctcgtgctttacggtatcgccgctcccgattcgcagcgcatcgccttctatcgccttcttgacgagttcttctgagcgggactctggggttcgaaatgaccgaccaagcgacgcccaacctgccatcacgagatttcgattccaccgccgccttctatgaaaggttgggcttcggaatcgttttccgggacgccggctggatgatcctccagcgcggggatctcatgctggagttcttcgcccaccccaacttgtttattgcagcttataatggttacaaataaagcaatagcatcacaaatttcacaaataaagcatttttttcactgcattctagttgtggtttgtccaaactcatcaatgtatcttatcatgtctgtataccgtcgacctctagctagagcttggcgtaatcatggtcatagctgtttcctgtgtgaaattgttatccgctcacaattccacacaacatacgagccggaagcataaagtgtaaagcctggggtgcctaatgagtgagctaactcacattaattgcgttgcgctcactgcccgctttccagtcgggaaacctgtcgtgccagctgcattaatgaatcggccaacgcgcggggagaggcggtttgcgtattgggcgctcttccgcttcctcgctcactgactcgctgcgctcggtcgttcggctgcggcgagcggtatcagctcactcaaaggcggtaatacggttatccacagaatcaggggataacgcaggaaagaacatgtgagcaaaaggccagcaaaaggccaggaaccgtaaaaaggccgcgttgctggcgtttttccataggctccgcccccctgacgagcatcacaaaaatcgacgctcaagtcagaggtggcgaaacccgacaggactataaagataccaggcgtttccccctggaagctccctcgtgcgctctcctgttccgaccctgccgcttaccggatacctgtccgcctttctcccttcgggaagcgtggcgctttctcatagctcacgctgtaggtatctcagttcggtgtaggtcgttcgctccaagctgggctgtgtgcacgaaccccccgttcagcccgaccgctgcgccttatccggtaactatcgtcttgagtccaacccggtaagacacgacttatcgccactggcagcagccactggtaacaggattagcagagcgaggtatgtaggcggtgctacagagttcttgaagtggtggcctaactacggctacactagaagaacagtatttggtatctgcgctctgctgaagccagttaccttcggaaaaagagttggtagctcttgatccggcaaacaaaccaccgctggtagcggtggtttttttgtttgcaagcagcagattacgcgcagaaaaaaaggatctcaagaagatcctttgatcttttctacggggtctgacgctcagtggaacgaaaactcacgttaagggattttggtcatgagattatcaaaaaggatcttcacctagatccttttaaattaaaaatgaagttttaaatcaatctaaagtatatatgagtaaacttggtctgacagttaccaatgcttaatcagtgaggcacctatctcagcgatctgtctatttcgttcatccatagttgcctgactccccgtcgtgtagataactacgatacgggagggcttaccatctggccccagtgctgcaatgataccgcgagacccacgctcaccggctccagatttatcagcaataaaccagccagccggaagggccgagcgcagaagtggtcctgcaactttatccgcctccatccagtctattaattgttgccgggaagctagagtaagtagttcgccagttaatagtttgcgcaacgttgttgccattgctacaggcatcgtggtgtcacgctcgtcgtttggtatggcttcattcagctccggttcccaacgatcaaggcgagttacatgatcccccatgttgtgcaaaaaagcggttagctccttcggtcctccgatcgttgtcagaagtaagttggccgcagtgttatcactcatggttatggcagcactgcataattctcttactgtcatgccatccgtaagatgcttttctgtgactggtgagtactcaaccaagtcattctgagaatagtgtatgcggcgaccgagttgctcttgcccggcgtcaatacgggataataccgcgccacatagcagaactttaaaagtgctcatcattggaaaacgttcttcggggcgaaaactctcaaggatcttaccgctgttgagatccagttcgatgtaacccactcgtgcacccaactgatcttcagcatcttttactttcaccagcgtttctgggtgagcaaaaacaggaaggcaaaatgccgcaaaaaagggaataagggcgacacggaaatgttgaatactcatactcttcctttttcaatattattgaagcatttatcagggttattgtctcatgagcggatacatatttgaatgtatttagaaaaataaacaaataggggttccgcgcacatttccccgaaaagtgccacctgacgtc

SEQ ID NO: 31 - protein, 383 aa, artificial
  NB33-meGFP-GSGGSGG-hRas
MSSRAQVQLVESGGGLVRPGGSRRLSCVDSERTSYPMGWFRRAPGKEREFVASITWSGIDPTYADSVADRFTISRDVANNTLYLQMNSLKHEDTAVYYCAARAPVGQSSSPYDYDYWGQGTQVTVSSAARGKGEELFTGVVPILVELDGDVNGHKFSVSGEGEGDATYGKLTLKFICTTGKLPVPWPTLVTTLTYGVQCFSRYPDHMKRHDFFKSAMPEGYVQERTIFFKDDGNYKTRAEVKFEGDTLVNRIELKGIDFKEDGNILGHKLEYNYNSHNVYIMADKQKNGIKANFKIRHNIESGGVQLADHYQQNTPIGDGPVLLPDNHYLSTQSKLSKDPNEKRDHMVLKERVTAAGITHGMDELYKGSGGSGGCMSCKCVLS

SEQ ID NO: 32 - DNA, 6562 bp, artificial
  NB33-meGFP-GSGGSGG-hRas
gacggatcgggagatctcccgatcccctatggtgcactctcagtacaatctgctctgatgccgcatagttaagccagtatctgctccctgcttgtgtgttggaggtcgctgagtagtgcgcgagcaaaatttaagctacaacaaggcaaggcttgaccgacaattgcatgaagaatctgcttagggttaggcgttttgcgctgcttcgcgatgtacgggccagatatacgcgttgacattgattattgactagttattaatagtaatcaattacggggtcattagttcatagcccatatatggagttccgcgttacataacttacggtaaatggcccgcctggctgaccgcccaacgacccccgcccattgacgtcaataatgacgtatgttcccatagtaacgccaatagggactttccattgacgtcaatgggtggagtatttacggtaaactgcccacttggcagtacatcaagtgtatcatatgccaagtacgccccctattgacgtcaatgacggtaaatggcccgcctggcattatgcccagtacatgaccttatgggactttcctacttggcagtacatctacgtattagtcatcgctattaccatggtgatgcggttttggcagtacatcaatgggcgtggatagcggtttgactcacggggatttccaagtctccaccccattgacgtcaatgggagtttgttttggcaccaaaatcaacgggactttccaaaatgtcgtaacaactccgccccattgacgcaaatgggcggtaggcgtgtacggtgggaggtctatataagcagagctctctggctaactagagaacccactgcttactggcttatcgaaattaatacgactcactatagggagacccaagctggctagcggtaccgagctcggatcactagtccagtgtggtggaattcacgcggaccatgtcttctagagcacaggtgcagctggtggagtctgggggaggattggtgcggcctgggggctctcggagactctcctgtgtggactctgagcgcaccagctatcccatgggctggttccgccgggccccagggaaggagcgggagtttgtggcatctattacctggagtggtattgacccaacatatgcagactccgtggccgaccgattcaccatctccagagatgtcgcgaataacacgctgtatctgcaaatgaacagcctgaaacatgaggacacggccgtttattattgtgcagctcgtgcccccgtggggcaatcctcttccccatatgactatgactactggggccaggggacccaggtcaccgtctcctcagcggccgctcgaggtaaaggagaagaacttttcactggagttgtcccaattcttgttgaattagatggtgatgttaatgggcacaaattttctgtcagtggagagggtgaaggtgatgcaacatacggaaaacttacccttaaatttatttgcactactggaaaactacctgttccttggccaacacttgtcactactttaacttatggtgttcaatgcttttcaagatacccagatcatatgaaacggcatgactttttcaagagtgccatgcccgaaggttatgtacaggaaagaactatatttttcaaagatgacgggaactacaagacacgtgctgaagtcaagtttgaaggtgatacccttgttaatagaatcgagttaaaaggtattgattttaaagaagatggaaacattcttggacacaaattggaatacaactataactcacacaatgtatacatcatggcagacaaacaaaagaatggaatcaaagctaacttcaaaattagacacaacattgagtccggaggcgttcaactagcagaccattatcaacaaaatactccaattggcgatggccctgtccttttaccagacaaccattacctgtccacacaatctaagctttcgaaagatcccaacgaaaagagagaccacatggtccttaaagagagggtaacagctgctgggattacacatggcatggacgagctgtacaagggatccggtggaagtggaggctgcatgagctgcaagtgtgtgctgtcctaatgagcggccgcactagagggcccgggcccgtttaaacccgctgatcagcctcgactgtgccttctagttgccagccatctgttgtttgcccctcccccgtgccttccttgaccctggaaggtgccactcccactgtcctttcctaataaaatgaggaaattgcatcgcattgtctgagtaggtgtcattctattctggggggtggggtggggcaggacagcaagggggaggattgggaagacaatagcaggcatgctggggatgcggtgggctctatggcttctgaggcggaaagaaccagctggggctctagggggtatccccacgcgccctgtagcggcgcattaagcgcggcgggtgtggtggttacgcgcagcgtgaccgctacacttgccagcgccctagcgcccgctcctttcgctttcttcccttcctttctcgccacgttcgccggctttccccgtcaagctctaaatcgggggctccctttagggttccgatttagtgctttacggcacctcgaccccaaaaaacttgattagggtgatggttcacgtagtgggccatcgccctgatagacggtttttcgccctttgacgttggagtccacgttctttaatagtggactcttgttccaaactggaacaacactcaaccctatctcggtctattcttttgatttataagggattttgccgatttcggcctattggttaaaaaatgagctgatttaacaaaaatttaacgcgaattaattctgtggaatgtgtgtcagttagggtgtggaaagtccccaggctccccagcaggcagaagtatgcaaagcatgcatctcaattagtcagcaaccaggtgtggaaagtccccaggctccccagcaggcagaagtatgcaaagcatgcatctcaattagtcagcaaccatagtcccgcccctaactccgcccatcccgcccctaactccgcccagttccgcccattctccgccccatggctgactaattttttttatttatgcagaggccgaggccgcctctgcctctgagctattccagaagtagtgaggaggcttttttggaggcctaggcttttgcaaaaagctcccgggagcttgtatatccattttcggatctgatcaagagacaggatgaggatcgtttcgcatgattgaacaagatggattgcacgcaggttctccggccgcttgggtggagaggctattcggctatgactgggcacaacagacaatcggctgctctgatgccgccgtgttccggctgtcagcgcaggggcgcccggttctttttgtcaagaccgacctgtccggtgccctgaatgaactgcaggacgaggcagcgcggctatcgtggctggccacgacgggcgttccttgcgcagctgtgctcgacgttgtcactgaagcgggaagggactggctgctattgggcgaagtgccggggcaggatctcctgtcatctcaccttgctcctgccgagaaagtatccatcatggctgatgcaatgcggcggctgcatacgcttgatccggctacctgcccattcgaccaccaagcgaaacatcgcatcgagcgagcacgtactcggatggaagccggtcttgtcgatcaggatgatctggacgaagagcatcaggggctcgcgccagccgaactgttcgccaggctcaaggcgcgcatgcccgacggcgaggatctcgtcgtgacccatggcgatgcctgcttgccgaatatcatggtggaaaatggccgcttttctggattcatcgactgtggccggctgggtgtggcggaccgctatcaggacatagcgttggctacccgtgatattgctgaagagcttggcggcgaatgggctgaccgcttcctcgtgctttacggtatcgccgctcccgattcgcagcgcatcgccttctatcgccttcttgacgagttcttctgagcgggactctggggttcgaaatgaccgaccaagcgacgcccaacctgccatcacgagatttcgattccaccgccgccttctatgaaaggttgggcttcggaatcgttttccgggacgccggctggatgatcctccagcgcggggatctcatgctggagttcttcgcccaccccaacttgtttattgcagcttataatggttacaaataaagcaatagcatcacaaatttcacaaataaagcatttttttcactgcattctagttgtggtttgtccaaactcatcaatgtatcttatcatgtctgtataccgtcgacctctagctagagcttggcgtaatcatggtcatagctgtttcctgtgtgaaattgttatccgctcacaattccacacaacatacgagccggaagcataaagtgtaaagcctggggtgcctaatgagtgagctaactcacattaattgcgttgcgctcactgcccgctttccagtcgggaaacctgtcgtgccagctgcattaatgaatcggccaacgcgcggggagaggcggtttgcgtattgggcgctcttccgcttcctcgctcactgactcgctgcgctcggtcgttcggctgcggcgagcggtatcagctcactcaaaggcggtaatacggttatccacagaatcaggggataacgcaggaaagaacatgtgagcaaaaggccagcaaaaggccaggaaccgtaaaaaggccgcgttgctggcgtttttccataggctccgcccccctgacgagcatcacaaaaatcgacgctcaagtcagaggtggcgaaacccgacaggactataaagataccaggcgtttccccctggaagctccctcgtgcgctctcctgttccgaccctgccgcttaccggatacctgtccgcctttctcccttcgggaagcgtggcgctttctcatagctcacgctgtaggtatctcagttcggtgtaggtcgttcgctccaagctgggctgtgtgcacgaaccccccgttcagcccgaccgctgcgccttatccggtaactatcgtcttgagtccaacccggtaagacacgacttatcgccactggcagcagccactggtaacaggattagcagagcgaggtatgtaggcggtgctacagagttcttgaagtggtggcctaactacggctacactagaagaacagtatttggtatctgcgctctgctgaagccagttaccttcggaaaaagagttggtagctcttgatccggcaaacaaaccaccgctggtagcggtggtttttttgtttgcaagcagcagattacgcgcagaaaaaaaggatctcaagaagatcctttgatcttttctacggggtctgacgctcagtggaacgaaaactcacgttaagggattttggtcatgagattatcaaaaaggatcttcacctagatccttttaaattaaaaatgaagttttaaatcaatctaaagtatatatgagtaaacttggtctgacagttaccaatgcttaatcagtgaggcacctatctcagcgatctgtctatttcgttcatccatagttgcctgactccccgtcgtgtagataactacgatacgggagggcttaccatctggccccagtgctgcaatgataccgcgagacccacgctcaccggctccagatttatcagcaataaaccagccagccggaagggccgagcgcagaagtggtcctgcaactttatccgcctccatccagtctattaattgttgccgggaagctagagtaagtagttcgccagttaatagtttgcgcaacgttgttgccattgctacaggcatcgtggtgtcacgctcgtcgtttggtatggcttcattcagctccggttcccaacgatcaaggcgagttacatgatcccccatgttgtgcaaaaaagcggttagctccttcggtcctccgatcgttgtcagaagtaagttggccgcagtgttatcactcatggttatggcagcactgcataattctcttactgtcatgccatccgtaagatgcttttctgtgactggtgagtactcaaccaagtcattctgagaatagtgtatgcggcgaccgagttgctcttgcccggcgtcaatacgggataataccgcgccacatagcagaactttaaaagtgctcatcattggaaaacgttcttcggggcgaaaactctcaaggatcttaccgctgttgagatccagttcgatgtaacccactcgtgcacccaactgatcttcagcatcttttactttcaccagcgtttctgggtgagcaaaaacaggaaggcaaaatgccgcaaaaaagggaataagggcgacacggaaatgttgaatactcatactcttcctttttcaatattattgaagcatttatcagggttattgtctcatgagcggatacatatttgaatgtatttagaaaaataaacaaataggggttccgcgcacatttccccgaaaagtgccacctgacgtc

SEQ ID NO: 33 - protein, 400 aa, artificial
  opioid receptor
MDSSAAPTNASNCTDALAYSSCSPAPSPGSWVNLSHLDGNLSDPCGPNRTDLGGRDSLCPPTGSPSMITAITIMALYSIVCVVGLFGNFLVMYVIVRYTKMKTATNIYIFNLALADALATSTLPFQSVNYLMGTWPFGTILCKIVISIDYYNMFTSIFTLCTMSVDRYIAVCHPVKALDFRTPRNAKIINVCNWILSSAIGLPVMFMATTKYRQGSIDCTLTFSHPTWYWENLLKICVFIFAFIMPVLIITVCYGLMILRLKSVRMLSGSKEKDRNLRRITRMVLVVVAVFIVCWTPIHIYVIIKALVTIPETTFQTVSWHFCIALGYTNSCLNPVLYAFLDENFKRCFREFCIPTSSNIEQQNSTRIRQNTRDHPSTANTVDRTNHQLENLEAETAPLP

SEQ ID NO: 34 - DNA, 6679 bp, artificial
  opioid receptor
gacggatcgggagatctcccgatcccctatggtcgactctcagtacaatctgctctgatgccgcatagttaagccagtatctgctccctgcttgtgtgttggaggtcgctgagtagtgcgcgagcaaaatttaagctacaacaaggcaaggcttgaccgacaattgcatgaagaatctgcttagggttaggcgttttgcgctgcttcgcgatgtacgggccagatatacgcgttgacattgattattgactagttattaatagtaatcaattacggggtcattagttcatagcccatatatggagttccgcgttacataacttacggtaaatggcccgcctggctgaccgcccaacgacccccgcccattgacgtcaataatgacgtatgttcccatagtaacgccaatagggactttccattgacgtcaatgggtggactatttacggtaaactgcccacttggcagtacatcaagtgtatcatatgccaagtacgccccctattgacgtcaatgacggtaaatggcccgcctggcattatgcccagtacatgaccttatgggactttcctacttggcagtacatctacgtattagtcatcgctattaccatggtgatgcggttttggcagtacatcaatgggcgtggatagcggtttgactcacggggatttccaagtctccaccccattgacgtcaatgggagtttgttttggcaccaaaatcaacgggactttccaaaatgtcgtaacaactccgccccattgacgcaaatgggcggtaggcgtgtacggtgggaggtctatataagcagagctctctggctaactagagaacccactgcttactggcttatcgaaattaatacgactcactatagggagacccaagcttggtaccgagctcggatccactagtaacggccgccagtgtgctggaattctgcagataaacgaattcgcccttctcctggctacctcgcacagcggtgcccgcccggccgtcagtaccatggacagcagcgctgcccccacgaacgccagcaattgcactgatgccttggcgtactcaagttgctccccagcacccagccccggttcctgggtcaacttgtcccacttagatggcaacctgtccgacccatgcggtccgaaccgcaccgacctgggcgggagagacagcctgtgccctccgaccggcagtccctccatgatcacggccatcacgatcatggccctctactccatcgtgtgcgtggtggggctcttcggaaacttcctggtcatgtatgtgattgtcagatacaccaagatgaagactgccaccaacatctacattttcaaccttgctctggcagatgccttagccaccagtaccctgcccttccagagtgtgaattacctaatgggaacatggccatttggaaccatcctttgcaagatagtgatctccatagattactataacatgttcaccagcatattcaccctctgcaccatgagtgttgatcgatacattgcagtctgccaccctgtcaaggccttagatttccgtactccccgaaatgccaaaattatcaatgtctgcaactggatcctctcttcagccattggtcttcctgtaatgttcatggctacaacaaaatacaggcaaggttccatagattgtacactaacattctctcatccaacctggtactgggaaaacctgctgaagatctgtgttttcatcttcgccttcattatgccagtgctcatcattaccgtgtgctatggactgatgatcttgcgcctcaagagtgtccgcatgctctctggctccaaagaaaaggacaggaatcttcgaaggatcaccaggatggtgctggtggtggtggctgtgttcatcgtctgctggactcccattcacatttacgtcatcattaaagccttggttacaatcccagaaactacgttccagactgtttcttggcacttctgcattgctctaggttacacaaacagctgcctcaacccagtcctttatgcatttctggatgaaaacttcaaacgatgcttcagagagttctgtatcccaacctcttccaacattgagcaacaaaactccactcgaattcgtcagaacactagagaccacccctccacggccaatacagtggatagaactaatcatcagctagaaaatctggaagcagaaactgctccgttgcccctcgactagagggccctattctatagtgtcacctaaatgctagagctcgctgatcagcctcgactgtgccttctagttgccagccatctgttgtttgcccctcccccgtgccttccttgaccctggaaggtgccactcccactgtcctttcctaataaaatgaggaaattgcatcgcattgtctgagtaggtgtcattctattctggggggtggggtggggcaggacagcaagggggaggattgggaagacaatagcaggcatgctggggatgcggtgggctctatggcttctgaggcggaaagaaccagctggggctctagggggtatccccacgcgccctgtagcggcgcattaagcgcggcgggtgtggtggttacgcgcagcgtgaccgctacacttgccagcgccctagcgcccgctcctttcgctttcttcccttcctttctcgccacgttcgccggctttccccgtcaagctctaaatcggggcatccctttagggttccgatttagtgctttacggcacctcgaccccaaaaaacttgattagggtgatggttcacgtagtgggccatcgccctgatagacggtttttcgccctttgacgttggagtccacgttctttaatagtggactcttgttccaaactggaacaacactcaaccctatctcggtctattcttttgatttataagggattttggggatttcggcctattggttaaaaaatgagctgatttaacaaaaatttaacgcgaattaattctgtggaatgtgtgtcagttagggtgtggaaagtccccaggctccccaggcaggcagaagtatgcaaagcatgcatctcaattagtcagcaaccaggtgtggaaagtccccaggctccccagcaggcagaagtatgcaaagcatgcatctcaattagtcagcaaccatagtcccgcccctaactccgcccatcccgcccctaactccgcccagttccgcccattctccgccccatggctgactaattttttttatttatgcagaggccgaggccgcctctgcctctgagctattccagaagtagtgaggaggcttttttggaggcctaggcttttgcaaaaagctcccgggagcttgtatatccattttcggatctgatcaagagacaggatgaggatcgtttcgcatgattgaacaagatggattgcacgcaggttctccggccgcttgggtggagaggctattcggctatgactgggcacaacagacaatcggctgctctgatgccgccgtgttccggctgtcagcgcaggggcgcccggttctttttgtcaagaccgacctgtccggtgccctgaatgaactgcaggacgaggcagcgcggctatcgtggctggccacgacgggcgttccttgcgcagctgtgctcgacgttgtcactgaagcgggaagggactggctgctattgggcgaagtgccggggcaggatctcctgtcatctcaccttgctcctgccgagaaagtatccatcatggctgatgcaatgcggcggctgcatacgcttgatccggctacctgcccattcgaccaccaagcgaaacatcgcatcgagcgagcacgtactcggatggaagccggtcttgtcgatcaggatgatctggacgaagagcatcaggggctcgcgccagccgaactgttcgccaggctcaaggcgcgcatgcccgacggcgaggatctcgtcgtgacccatggcgatgcctgcttgccgaatatcatggtggaaaatggccgcttttctggattcatcgactgtggccggctgggtgtggcggaccgctatcaggacatagcgttggctacccgtgatattgctgaagagcttggcggcgaatgggctgaccgcttcctcgtgctttacggtatcgccgctcccgattcgcagcgcatcgccttctatcgccttcttgacgagttcttctgagcgggactctggggttcgaaatgaccgaccaagcgacgcccaacctgccatcacgagatttcgattccaccgccgccttctatgaaaggttgggcttcggaatcgttttccgggacgccggctggatgatcctccagcgcggggatctcatgctggagttcttcgcccaccccaacttgtttattgcagcttataatggttacaaataaagcaatagcatcacaaatttcacaaataaagcatttttttcactgcattctagttgtggtttgtccaaactcatcaatgtatcttatcatgtctgtataccgtcgacctctagctagagcttggcgtaatcatggtcatagctgtttcctgtgtgaaattgttatccgctcacaattccacacaacatacgagccggaagcataaagtgtaaagcctggggtgcctaatgagtgagctaactcacattaattgcgttgcgctcactgcccgctttccagtcgggaaacctgtcgtgccagctgcattaatgaatcggccaacgcgcggggagaggcggtttgcgtattgggcgctcttccgcttcctcgctcactgactcgctgcgctcggtcgttcggctgcggcgagcggtatcagctcactcaaaggcggtaatacggttatccacagaatcaggggataacgcaggaaagaacatgtgagcaaaaggccagcaaaaggccaggaaccgtaaaaaggccgcgttgctggcgtttttccataggctccgcccccctgacgagcatcacaaaaatcgacgctcaagtcagaggtggcgaaacccgacaggactataaagataccaggcgtttccccctggaagctccctcgtgcgctctcctgttccgaccctgccgcttaccggatacctgtccgcctttctcccttcgggaagcgtggcgctttctcaatgctcacgctgtaggtatctcagttcggtgtaggtcgttcgctccaagctgggctgtgtgcacgaaccccccgttcagcccgaccgctgcgccttatccggtaactatcgtcttgagtccaacccggtaagacacgacttatcgccactggcagcagccactggtaacaggattagcagagcgaggtatgtaggcggtgctacagagttcttgaagtggtggcctaactacggctacactagaaggacagtatttggtatctgcgctctgctgaagccagttaccttcggaaaaagagttggtagctcttgatccggcaaacaaaccaccgctggtagcggtggtttttttgtttgcaagcagcagattacgcgcagaaaaaaaggatctcaagaagatcctttgatcttttctacggggtctgacgctcagtggaacgaaaactcacgttaagggattttggtcatgagattatcaaaaaggatcttcacctagatccttttaaattaaaaatgaagttttaaatcaatctaaagtatatatgagtaaacttggtctgacagttaccaatgcttaatcagtgaggcacctatctcagcgatctgtctatttcgttcatccatagttgcctgactccccgtcgtgtagataactacgatacgggagggcttaccatctggccccagtgctgcaatgataccgcgagacccacgctcaccggctccagatttatcagcaataaaccagccagccggaagggccgagcgcagaagtggtcctgcaactttatccgcctccatccagtctattaattgttgccgggaagctagagtaagtagttcgccagttaatagtttgcgcaacgttgttgccattgctacaggcatcgtggtgtcacgctcgtcgtttggtatggcttcattcagctccggttcccaacgatcaaggcgagttacatgatcccccatgttgtgcaaaaaagcggttagctccttcggtcctccgatcgttgtcagaagtaagttggccgcagtgttatcactcatggttatggcagcactgcataattctcttactgtcatgccatccgtaagatgcttttctgtgactggtgagtactcaaccaagtcattctgagaatagtgtatgcggcgaccgagttgctcttgcccggcgtcaatacgggataataccgcgccacatagcagaactttaaaagtgctcatcattggaaaacgttcttcggggcgaaaactctcaaggatcttaccgctgttgagatccagttcgatgtaacccactcgtgcacccaactgatcttcagcatcttttactttcaccagcgtttctgggtgagcaaaaacaggaaggcaaaatgccgcaaaaaagggaataagggcgacacggaaatgttgaatactcatactcttcctttttcaatattattgaagcatttatcagggttattgtctcatgagcggatacatatttgaatgtatttagaaaaataaacaaataggggttccgcgcacatttccccgaaaagtgccacctgacgtc

SEQ ID NO: 35 - protein, 395 aa, artificial
  GAP43-SSGSSGTG-meGFP-NB33
MLCCMRRTKQVEKNDEDQNSSGSSGTGSKGEELFTGVVPILVELDGDVNGHKFSVSGEGEGDATYGKLTLKFICTTGKLPVPWPTLVTTLTYGVQCFSRYPDHMKRHDFFKSAMPEGYVQERTIFFKDDGNYKTRAEVKFEGDTLVNRIELKGIDFKEDGNILGHKLEYNYNSHNVYIMADKQKNGIKANFKIRHNIESGGVQLADHYQQNTPIGDGPVLLPDNHYLSTQSKLSKDPNEKRDHMVLKERVTAAGITHGMDELYKGSSRAQVQLVESGGGLVRPGGSRRLSCVDSERTSYPMGWFRRAPGKEREFVASITWSGIDPTYADSVADRFTISRDVANNTLYLQMNSLKHEDTAVYYCAARAPVGQSSSPYDYDYWGQGTQVTVSSAARG

SEQ ID NO: 36 - DNA, 6583 bp, artificial
  GAP43-SSGSSGTG-meGFP-NB33
gacggatcgggagatctcccgatcccctatggtgcactctcagtacaatctgctctgatgccgcatagttaagccagtatctgctccctgcttgtgtgttggaggtcgctgagtagtgcgcgagcaaaatttaagctacaacaaggcaaggcttgaccgacaattgcatgaagaatctgcttagggttaggcgttttgcgctgcttcgcgatgtacgggccagatatacgcgttgacattgattattgactagttattaatagtaatcaattacggggtcattagttcatagcccatatatggagttccgcgttacataacttacggtaaatggcccgcctggctgaccgcccaacgacccccgcccattgacgtcaataatgacgtatgttcccatagtaacgccaatagggactttccattgacgtcaatgggtggagtatttacggtaaactgcccacttggcagtacatcaagtgtatcatatgccaagtacgccccctattgacgtcaatgacggtaaatggcccgcctggcattatgcccagtacatgaccttatgggactttcctacttggcagtacatctacgtattagtcatcgctattaccatggtgatgcggttttggcagtacatcaatgggcgtggatagcggtttgactcacggggatttccaagtctccaccccattgacgtcaatgggagtttgttttggcaccaaaatcaacgggactttccaaaatgtcgtaacaactccgccccattgacgcaaatgggcggtaggcgtgtacggtgggaggtctatataagcagagctctctggctaactagagaacccactgcttactggcttatcgaaattaatacgactcactatagggagacccaagctggctagcgtttaaacttaagcttggtaccgacggaccatgctgtgctgtatgagaagaaccaaacaggttgaaaagaatgatgaggaccagaattcctccggatcgtctggaaccggttctaaaggagaagaacttttcactggagttgtcccaattcttgttgaattagatggtgatgttaatgggcacaaattttctgtcagtggagagggtgaaggtgatgcaacatacggaaaacttacccttaaatttatttgcactactggaaaactacctgttccttggccaacacttgtcactactttaacttatggtgttcaatgcttttcaagatacccagatcatatgaaacggcatgactttttcaagagtgccatgcccgaaggttatgtacaggaaagaactatatttttcaaagatgacgggaactacaagacacgtgctgaagtcaagtttgaaggtgatacccttgttaatagaatcgagttaaaaggtattgattttaaagaagatggaaacattcttggacacaaattggaatacaactataactcacacaatgtatacatcatggcagacaaacaaaagaatggaatcaaagctaacttcaaaattagacacaacattgagtccggaggcgttcaactagcagaccattatcaacaaaatactccaattggcgatggccctgtccttttaccagacaaccattacctgtccacacaatctaagctttcgaaagatcccaacgaaaagagagaccacatggtccttaaagagagggtaacagctgctgggattacacatggcatggacgagctgtacaagggatcctctagagcacaggtgcagctggtggagtctgggggaggattggtgcggcctgggggctctcggagactctcctgtgtggactctgagcgcaccagctatcccatgggctggttccgccgggccccagggaaggagcgggagtttgtggcatctattacctggagtggtattgacccaacatatgcagactccgtggccgaccgattcaccatctccagagatgtcgcgaataacacgctgtatctgcaaatgaacagcctgaaacatgaggacacggccgtttattattgtgcagctcgtgcccccgtggggcaatcctcttccccatatgactatgactactggggccaggggacccaggtcaccgtctcctcagcggccgctcgaggataatgaaggtggcggccgctcgaaactagagggcccgtttaaacccgctgatcagcctcgactgtgccttctagttgccagccatctgttgtttgcccctcccccgtgccttccttgaccctggaaggtgccactcccactgtcctttcctaataaaatgaggaaattgcatcgcattgtctgagtaggtgtcattctattctggggggtggggtggggcaggacagcaagggggaggattgggaagacaatagcaggcatgctggggatgcggtgggctctatggcttctgaggcggaaagaaccagctggggctctagggggtatccccacgcgccctgtagcggcgcattaagcgcggcgggtgtggtggttacgcgcagcgtgaccgctacacttgccagcgccctagcgcccgctcctttcgctttcttcccttcctttctcgccacgttcgccggctttccccgtcaagctctaaatcgggggctccctttagggttccgatttagtgctttacggcacctcgaccccaaaaaacttgattagggtgatggttcacgtagtgggccatcgccctgatagacggtttttcgccctttgacgttggagtccacgttctttaatagtggactcttgttccaaactggaacaacactcaaccctatctcggtctattcttttgatttataagggattttgccgatttcggcctattggttaaaaaatgagctgatttaacaaaaatttaacgcgaattaattctgtggaatgtgtgtcagttagggtgtggaaagtccccaggctccccagcaggcagaagtatgcaaagcatgcatctcaattagtcagcaaccaggtgtggaaagtccccaggctccccagcaggcagaagtatgcaaagcatgcatctcaattagtcagcaaccatagtcccgcccctaactccgcccatcccgcccctaactccgcccagttccgcccattctccgccccatggctgactaattttttttatttatgcagaggccgaggccgcctctgcctctgagctattccagaagtagtgaggaggcttttttggaggcctaggcttttgcaaaaagctcccgggagcttgtatatccattttcggatctgatcaagagacaggatgaggatcgtttcgcatgattgaacaagatggattgcacgcaggttctccggccgcttgggtggagaggctattcggctatgactgggcacaacagacaatcggctgctctgatgccgccgtgttccggctgtcagcgcaggggcgcccggttctttttgtcaagaccgacctgtccggtgccctgaatgaactgcaggacgaggcagcgcggctatcgtggctggccacgacgggcgttccttgcgcagctgtgctcgacgttgtcactgaagcgggaagggactggctgctattgggcgaagtgccggggcaggatctcctgtcatctcaccttgctcctgccgagaaagtatccatcatggctgatgcaatgcggcggctgcatacgcttgatccggctacctgcccattcgaccaccaagcgaaacatcgcatcgagcgagcacgtactcggatggaagccggtcttgtcgatcaggatgatctggacgaagagcatcaggggctcgcgccagccgaactgttcgccaggctcaaggcgcgcatgcccgacggcgaggatctcgtcgtgacccatggcgatgcctgcttgccgaatatcatggtggaaaatggccgcttttctggattcatcgactgtggccggctgggtgtggcggaccgctatcaggacatagcgttggctacccgtgatattgctgaagagcttggcggcgaatgggctgaccgcttcctcgtgctttacggtatcgccgctcccgattcgcagcgcatcgccttctatcgccttcttgacgagttcttctgagcgggactctggggttcgaaatgaccgaccaagcgacgcccaacctgccatcacgagatttcgattccaccgccgccttctatgaaaggttgggcttcggaatcgttttccgggacgccggctggatgatcctccagcgcggggatctcatgctggagttcttcgcccaccccaacttgtttattgcagcttataatggttacaaataaagcaatagcatcacaaatttcacaaataaagcatttttttcactgcattctagttgtggtttgtccaaactcatcaatgtatcttatcatgtctgtataccgtcgacctctagctagagcttggcgtaatcatggtcatagctgtttcctgtgtgaaattgttatccgctcacaattccacacaacatacgagccggaagcataaagtgtaaagcctggggtgcctaatgagtgagctaactcacattaattgcgttgcgctcactgcccgctttccagtcgggaaacctgtcgtgccagctgcattaatgaatcggccaacgcgcggggagaggcggtttgcgtattgggcgctcttccgcttcctcgctcactgactcgctgcgctcggtcgttcggctgcggcgagcggtatcagctcactcaaaggcggtaatacggttatccacagaatcaggggataacgcaggaaagaacatgtgagcaaaaggccagcaaaaggccaggaaccgtaaaaaggccgcgttgctggcgtttttccataggctccgcccccctgacgagcatcacaaaaatcgacgctcaagtcagaggtggcgaaacccgacaggactataaagataccaggcgtttccccctggaagctccctcgtgcgctctcctgttccgaccctgccgcttaccggatacctgtccgcctttctcccttcgggaagcgtggcgctttctcatagctcacgctgtaggtatctcagttcggtgtaggtcgttcgctccaagctgggctgtgtgcacgaaccccccgttcagcccgaccgctgcgccttatccggtaactatcgtcttgagtccaacccggtaagacacgacttatcgccactggcagcagccactggtaacaggattagcagagcgaggtatgtaggcggtgctacagagttcttgaagtggtggcctaactacggctacactagaagaacagtatttggtatctgcgctctgctgaagccagttaccttcggaaaaagagttggtagctcttgatccggcaaacaaaccaccgctggtagcggtggtttttttgtttgcaagcagcagattacgcgcagaaaaaaaggatctcaagaagatcctttgatcttttctacggggtctgacgctcagtggaacgaaaactcacgttaagggattttggtcatgagattatcaaaaaggatcttcacctagatccttttaaattaaaaatgaagttttaaatcaatctaaagtatatatgagtaaacttggtctgacagttaccaatgcttaatcagtgaggcacctatctcagcgatctgtctatttcgttcatccatagttgcctgactccccgtcgtgtagataactacgatacgggagggcttaccatctggccccagtgctgcaatgataccgcgagacccacgctcaccggctccagatttatcagcaataaaccagccagccggaagggccgagcgcagaagtggtcctgcaactttatccgcctccatccagtctattaattgttgccgggaagctagagtaagtagttcgccagttaatagtttgcgcaacgttgttgccattgctacaggcatcgtggtgtcacgctcgtcgtttggtatggcttcattcagctccggttcccaacgatcaaggcgagttacatgatcccccatgttgtgcaaaaaagcggttagctccttcggtcctccgatcgttgtcagaagtaagttggccgcagtgttatcactcatggttatggcagcactgcataattctcttactgtcatgccatccgtaagatgcttttctgtgactggtgagtactcaaccaagtcattctgagaatagtgtatgcggcgaccgagttgctcttgcccggcgtcaatacgggataataccgcgccacatagcagaactttaaaagtgctcatcattggaaaacgttcttcggggcgaaaactctcaaggatcttaccgctgttgagatccagttcgatgtaacccactcgtgcacccaactgatcttcagcatcttttactttcaccagcgtttctgggtgagcaaaaacaggaaggcaaaatgccgcaaaaaagggaataagggcgacacggaaatgttgaatactcatactcttcctttttcaatattattgaagcatttatcagggttattgtctcatgagcggatacatatttgaatgtatttagaaaaataaacaaataggggttccgcgcacatttccccgaaaagtgccacctgacgtc

SEQ ID NO: 37 - protein, 453 aa, artificial
  GAP43-SSGSSGTG-meGFP-GRK2ct
MLCCMRRTKQVEKNDEDQNSSGSSGTGSKGEELFTGVVPILVELDGDVNGHKFSVSGEGEGDATYGKLTLKFICTTGKLPVPWPTLVTTLTYGVQCFSRYPDHMKRHDFFKSAMPEGYVQERTIFFKDDGNYKTRAEVKFEGDTLVNRIELKGIDFKEDGNILGHKLEYNYNSHNVYIMADKQKNGIKANFKIRHNIESGGVQLADHYQQNTPIGDGPVLLPDNHYLSTQSKLSKDPNEKRDHMVLKERVTAAGITHGMDELYKGSSRNFPLVISERWQQEVAETVYEAVNADTDKIEARKRAKNKQLGHEEDYALGRDCIVHGYMLKLGNPFLTQWQRRYFYLFPNRLEWRGEGESRQSLLTMEQIVSVEETQIKDKKCILLRIKGGKQFVLQCESDPEFVQWKKELTETFMEAQRLLRRAPKFLNKSRSAVVELSKPPLCHRNSNGLGSRG

SEQ ID NO: 38 - DNA, 6754 bp, artificial
  GAP43-SSGSSGTG-meGFP-GRK2ct
gacggatcgggagatctcccgatcccctatggtgcactctcagtacaatctgctctgatgccgcatagttaagccagtatctgctccctgcttgtgtgttggaggtcgctgagtagtgcgcgagcaaaatttaagctacaacaaggcaaggcttgaccgacaattgcatgaagaatctgcttagggttaggcgttttgcgctgcttcgcgatgtacgggccagatatacgcgttgacattgattattgactagttattaatagtaatcaattacggggtcattagttcatagcccatatatggagttccgcgttacataacttacggtaaatggcccgcctggctgaccgcccaacgacccccgcccattgacgtcaataatgacgtatgttcccatagtaacgccaatagggactttccattgacgtcaatgggtggagtatttacggtaaactgcccacttggcagtacatcaagtgtatcatatgccaagtacgccccctattgacgtcaatgacggtaaatggcccgcctggcattatgcccagtacatgaccttatgggactttcctacttggcagtacatctacgtattagtcatcgctattaccatggtgatgcggttttggcagtacatcaatgggcgtggatagcggtttgactcacggggatttccaagtctccaccccattgacgtcaatgggagtttgttttggcaccaaaatcaacgggactttccaaaatgtcgtaacaactccgccccattgacgcaaatgggcggtaggcgtgtacggtgggaggtctatataagcagagctctctggctaactagagaacccactgcttactggcttatcgaaattaatacgactcactatagggagacccaagctggctagcgtttaaacttaagcttggtaccgacggaccatgctgtgctgtatgagaagaaccaaacaggttgaaaagaatgatgaggaccagaattcctccggatcgtctggaaccggttctaaaggagaagaacttttcactggagttgtcccaattcttgttgaattagatggtgatgttaatgggcacaaattttctgtcagtggagagggtgaaggtgatgcaacatacggaaaacttacccttaaatttatttgcactactggaaaactacctgttccttggccaacacttgtcactactttaacttatggtgttcaatgcttttcaagatacccagatcatatgaaacggcatgactttttcaagagtgccatgcccgaaggttatgtacaggaaagaactatatttttcaaagatgacgggaactacaagacacgtgctgaagtcaagtttgaaggtgatacccttgttaatagaatcgagttaaaaggtattgattttaaagaagatggaaacattcttggacacaaattggaatacaactataactcacacaatgtatacatcatggcagacaaacaaaagaatggaatcaaagctaacttcaaaattagacacaacattgagtccggaggcgttcaactagcagaccattatcaacaaaatactccaattggcgatggccctgtccttttaccagacaaccattacctgtccacacaatctaagctttcgaaagatcccaacgaaaagagagaccacatggtccttaaagagagggtaacagctgctgggattacacatggcatggacgagctgtacaagggatcctctagaaacttccctctggtgatctctgagcgctggcagcaggaagtggcggaaacagtttatgaagcagtaaatgcagacacggataaaatcgaggccaggaagagagctaaaaataagcagcttggccacgaagaagattacgccctgggaagagactgcatcgtgcacgggtacatgctgaagctggggaaccctttcctgacccagtggcagcgccgctatttttacctctttccgaacagacttgagtggagaggagaaggcgagtcgcgacaaagtttactgacaatggaacagattgtgtccgtggaagaaactcagattaaagacaaaaagtgcattttgttgagaataaaaggagggaagcagttcgttttgcagtgtgagagtgacccagagtttgtgcagtggaagaaagagctgacggagacattcatggaggcccagcggctgctacggcgagcccccaagttcctcaacaaatcccgctcagccgtcgtggaactctcaaagcctcccctctgccataggaacagcaacggcctcggatctcgaggataatgaaggtggcggccgctcgaaactagagggcccgtttaaacccgctgatcagcctcgactgtgccttctagttgccagccatctgttgtttgcccctcccccgtgccttccttgaccctggaaggtgccactcccactgtcctttcctaataaaatgaggaaattgcatcgcattgtctgagtaggtgtcattctattctggggggtggggtggggcaggacagcaagggggaggattgggaagacaatagcaggcatgctggggatgcggtgggctctatggcttctgaggcggaaagaaccagctggggctctagggggtatccccacgcgccctgtagcggcgcattaagcgcggcgggtgtggtggttacgcgcagcgtgaccgctacacttgccagcgccctagcgcccgctcctttcgctttcttcccttcctttctcgccacgttcgccggctttccccgtcaagctctaaatcgggggctccctttagggttccgatttagtgctttacggcacctcgaccccaaaaaacttgattagggtgatggttcacgtagtgggccatcgccctgatagacggtttttcgccctttgacgttggagtccacgttctttaatagtggactcttgttccaaactggaacaacactcaaccctatctcggtctattcttttgatttataagggattttgccgatttcggcctattggttaaaaaatgagctgatttaacaaaaatttaacgcgaattaattctgtggaatgtgtgtcagttagggtgtggaaagtccccaggctccccagcaggcagaagtatgcaaagcatgcatctcaattagtcagcaaccaggtgtggaaagtccccaggctccccagcaggcagaagtatgcaaagcatgcatctcaattagtcagcaaccatagtcccgcccctaactccgcccatcccgcccctaactccgcccagttccgcccattctccgccccatggctgactaattttttttatttatgcagaggccgaggccgcctctgcctctgagctattccagaagtagtgaggaggcttttttggaggcctaggcttttgcaaaaagctcccgggagcttgtatatccattttcggatctgatcaagagacaggatgaggatcgtttcgcatgattgaacaagatggattgcacgcaggttctccggccgcttgggtggagaggctattcggctatgactgggcacaacagacaatcggctgctctgatgccgccgtgttccggctgtcagcgcaggggcgcccggttctttttgtcaagaccgacctgtccggtgccctgaatgaactgcaggacgaggcagcgcggctatcgtggctggccacgacgggcgttccttgcgcagctgtgctcgacgttgtcactgaagcgggaagggactggctgctattgggcgaagtgccggggcaggatctcctgtcatctcaccttgctcctgccgagaaagtatccatcatggctgatgcaatgcggcggctgcatacgcttgatccggctacctgcccattcgaccaccaagcgaaacatcgcatcgagcgagcacgtactcggatggaagccggtcttgtcgatcaggatgatctggacgaagagcatcaggggctcgcgccagccgaactgttcgccaggctcaaggcgcgcatgcccgacggcgaggatctcgtcgtgacccatggcgatgcctgcttgccgaatatcatggtggaaaatggccgcttttctggattcatcgactgtggccggctgggtgtggcggaccgctatcaggacatagcgttggctacccgtgatattgctgaagagcttggcggcgaatgggctgaccgcttcctcgtgctttacggtatcgccgctcccgattcgcagcgcatcgccttctatcgccttcttgacgagttcttctgagcgggactctggggttcgaaatgaccgaccaagcgacgcccaacctgccatcacgagatttcgattccaccgccgccttctatgaaaggttgggcttcggaatcgttttccgggacgccggctggatgatcctccagcgcggggatctcatgctggagttcttcgcccaccccaacttgtttattgcagcttataatggttacaaataaagcaatagcatcacaaatttcacaaataaagcatttttttcactgcattctagttgtggtttgtccaaactcatcaatgtatcttatcatgtctgtataccgtcgacctctagctagagcttggcgtaatcatggtcatagctgtttcctgtgtgaaattgttatccgctcacaattccacacaacatacgagccggaagcataaagtgtaaagcctggggtgcctaatgagtgagctaactcacattaattgcgttgcgctcactgcccgctttccagtcgggaaacctgtcgtgccagctgcattaatgaatcggccaacgcgcggggagaggcggtttgcgtattgggcgctcttccgcttcctcgctcactgactcgctgcgctcggtcgttcggctgcggcgagcggtatcagctcactcaaaggcggtaatacggttatccacagaatcaggggataacgcaggaaagaacatgtgagcaaaaggccagcaaaaggccaggaaccgtaaaaaggccgcgttgctggcgtttttccataggctccgcccccctgacgagcatcacaaaaatcgacgctcaagtcagaggtggcgaaacccgacaggactataaagataccaggcgtttccccctggaagctccctcgtgcgctctcctgttccgaccctgccgcttaccggatacctgtccgcctttctcccttcgggaagcgtggcgctttctcatagctcacgctgtaggtatctcagttcggtgtaggtcgttcgctccaagctgggctgtgtgcacgaaccccccgttcagcccgaccgctgcgccttatccggtaactatcgtcttgagtccaacccggtaagacacgacttatcgccactggcagcagccactggtaacaggattagcagagcgaggtatgtaggcggtgctacagagttcttgaagtggtggcctaactacggctacactagaagaacagtatttggtatctgcgctctgctgaagccagttaccttcggaaaaagagttggtagctcttgatccggcaaacaaaccaccgctggtagcggtggtttttttgtttgcaagcagcagattacgcgcagaaaaaaaggatctcaagaagatcctttgatcttttctacggggtctgacgctcagtggaacgaaaactcacgttaagggattttggtcatgagattatcaaaaaggatcttcacctagatccttttaaattaaaaatgaagttttaaatcaatctaaagtatatatgagtaaacttggtctgacagttaccaatgcttaatcagtgaggcacctatctcagcgatctgtctatttcgttcatccatagttgcctgactccccgtcgtgtagataactacgatacgggagggcttaccatctggccccagtgctgcaatgataccgcgagacccacgctcaccggctccagatttatcagcaataaaccagccagccggaagggccgagcgcagaagtggtcctgcaactttatccgcctccatccagtctattaattgttgccgggaagctagagtaagtagttcgccagttaatagtttgcgcaacgttgttgccattgctacaggcatcgtggtgtcacgctcgtcgtttggtatggcttcattcagctccggttcccaacgatcaaggcgagttacatgatcccccatgttgtgcaaaaaagcggttagctccttcggtcctccgatcgttgtcagaagtaagttggccgcagtgttatcactcatggttatggcagcactgcataattctcttactgtcatgccatccgtaagatgcttttctgtgactggtgagtactcaaccaagtcattctgagaatagtgtatgcggcgaccgagttgctcttgcccggcgtcaatacgggataataccgcgccacatagcagaactttaaaagtgctcatcattggaaaacgttcttcggggcgaaaactctcaaggatcttaccgctgttgagatccagttcgatgtaacccactcgtgcacccaactgatcttcagcatcttttactttcaccagcgtttctgggtgagcaaaaacaggaaggcaaaatgccgcaaaaaagggaataagggcgacacggaaatgttgaatactcatactcttcctttttcaatattattgaagcatttatcagggttattgtctcatgagcggatacatatttgaatgtatttagaaaaataaacaaataggggttccgcgcacatttccccgaaaagtgccacctgacgtc

SEQ ID NO: 39 - protein, 512 aa, artificial
  GAP43-SSGSSGTG-HALO-GRK2ct
MLCCMRRTKQVEKNDEDQNSSGSSGTGAEIGTGFPFDPHYVEVLGERMHYVDVGPRDGTPVLFLHGNPTSSYVWRNIIPHVAPTHRCIAPDLIGMGKSDKPDLGYFFDDHVRFMDAFIEALGLEEVVLVIHDWGSALGFHWAKRNPERVKGIAFMEFIRPIPTWDEWPEFARETFQAFRTTDVGRKLIIDQNVFIEGTLPMGVVRPLTEVEMDHYREPFLNPVDREPLWRFPNELPIAGEPANIVALVEEYMDWLHQSPVPKLLFWGTPGVLIPPAEAARLAKSLPNCKAVDIGPGLNLLQEDNPDLIGSEIARWLSTLEISGGSSRNFPLVISERWQQEVAETVYEAVNADTDKIEARKRAKNKQLGHEEDYALGRDCIVHGYMLKLGNPFLTQWQRRYFYLFPNRLEWRGEGESRQSLLTMEQIVSVEETQIKDKKCILLRIKGGKQFVLQCESDPEFVQWKKELTETFMEAQRLLRRAPKFLNKSRSAVVELSKPPLCHRNSNGLGSRG

SEQ ID NO: 40 - DNA, 6931 bp, artificial
  GAP43-SSGSSGTG-HALO-GRK2ct
gacggatcgggagatctcccgatcccctatggtgcactctcagtacaatctgctctgatgccgcatagttaagccagtatctgctccctgcttgtgtgttggaggtcgctgagtagtgcgcgagcaaaatttaagctacaacaaggcaaggcttgaccgacaattgcatgaagaatctgcttagggttaggcgttttgcgctgcttcgcgatgtacgggccagatatacgcgttgacattgattattgactagttattaatagtaatcaattacggggtcattagttcatagcccatatatggagttccgcgttacataacttacggtaaatggcccgcctggctgaccgcccaacgacccccgcccattgacgtcaataatgacgtatgttcccatagtaacgccaatagggactttccattgacgtcaatgggtggagtatttacggtaaactgcccacttggcagtacatcaagtgtatcatatgccaagtacgccccctattgacgtcaatgacggtaaatggcccgcctggcattatgcccagtacatgaccttatgggactttcctacttggcagtacatctacgtattagtcatcgctattaccatggtgatgcggttttggcagtacatcaatgggcgtggatagcggtttgactcacggggatttccaagtctccaccccattgacgtcaatgggagtttgttttggcaccaaaatcaacgggactttccaaaatgtcgtaacaactccgccccattgacgcaaatgggcggtaggcgtgtacggtgggaggtctatataagcagagctctctggctaactagagaacccactgcttactggcttatcgaaattaatacgactcactatagggagacccaagctggctagcgtttaaacttaagcttggtaccgacggaccatgctgtgctgtatgagaagaaccaaacaggttgaaaagaatgatgaggaccagaattcctccggatcgtctggaaccggtgcagaaatcggtactggctttccattcgacccccattatgtggaagtcctgggcgagcgcatgcactacgtcgatgttggtccgcgcgatggcacccctgtgctgttcctgcacggtaacccgacctcctcctacgtgtggcgcaacatcatcccgcatgttgcaccgacccatcgctgcattgctccagacctgatcggtatgggcaaatccgacaaaccagacctgggttatttcttcgacgaccacgtccgcttcatggatgccttcatcgaagccctgggtctggaagaggtcgtcctggtcattcacgactggggctccgctctgggtttccactgggccaagcgcaatccagagcgcgtcaaaggtattgcatttatggagttcatccgccctatcccgacctgggacgaatggccagaatttgcccgcgagaccttccaggccttccgcaccaccgacgtcggccgcaagctgatcatcgatcagaacgtttttatcgagggtacgctgccgatgggtgtcgtccgcccgctgactgaagtcgagatggaccattaccgcgagccgttcctgaatcctgttgaccgcgagccactgtggcgcttcccaaacgagctgccaatcgccggtgagccagcgaacatcgtcgcgctggtcgaagaatacatggactggctgcaccagtcccctgtcccgaagctgctgttctggggcaccccaggcgttctgatcccaccggccgaagccgctcgcctggccaaaagcctgcctaactgcaaggctgtggacatcggcccgggtctgaatctgctgcaagaagacaacccggacctgatcggcagcgagatcgcgcgctggctgtcgacgctcgagatttccggcggatcctctagaaacttccctctggtgatctctgagcgctggcagcaggaagtggcggaaacagtttatgaagcagtaaatgcagacacggataaaatcgaggccaggaagagagctaaaaataagcagcttggccacgaagaagattacgccctgggaagagactgcatcgtgcacgggtacatgctgaagctggggaaccctttcctgacccagtggcagcgccgctatttttacctctttccgaacagacttgagtggagaggagaaggcgagtcgcgacaaagtttactgacaatggaacagattgtgtccgtggaagaaactcagattaaagacaaaaagtgcattttgttgagaataaaaggagggaagcagttcgttttgcagtgtgagagtgacccagagtttgtgcagtggaagaaagagctgacggagacattcatggaggcccagcggctgctacggcgagcccccaagttcctcaacaaatcccgctcagccgtcgtggaactctcaaagcctcccctctgccataggaacagcaacggcctcggatctcgaggataatgaaggtggcggccgctcgaaactagagggcccgtttaaacccgctgatcagcctcgactgtgccttctagttgccagccatctgttgtttgcccctcccccgtgccttccttgaccctggaaggtgccactcccactgtcctttcctaataaaatgaggaaattgcatcgcattgtctgagtaggtgtcattctattctggggggtggggtggggcaggacagcaagggggaggattgggaagacaatagcaggcatgctggggatgcggtgggctctatggcttctgaggcggaaagaaccagctggggctctagggggtatccccacgcgccctgtagcggcgcattaagcgcggcgggtgtggtggttacgcgcagcgtgaccgctacacttgccagcgccctagcgcccgctcctttcgctttcttcccttcctttctcgccacgttcgccggctttccccgtcaagctctaaatcgggggctccctttagggttccgatttagtgctttacggcacctcgaccccaaaaaacttgattagggtgatggttcacgtagtgggccatcgccctgatagacggtttttcgccctttgacgttggagtccacgttctttaatagtggactcttgttccaaactggaacaacactcaaccctatctcggtctattcttttgatttataagggattttgccgatttcggcctattggttaaaaaatgagctgatttaacaaaaatttaacgcgaattaattctgtggaatgtgtgtcagttagggtgtggaaagtccccaggctccccagcaggcagaagtatgcaaagcatgcatctcaattagtcagcaaccaggtgtggaaagtccccaggctccccagcaggcagaagtatgcaaagcatgcatctcaattagtcagcaaccatagtcccgcccctaactccgcccatcccgcccctaactccgcccagttccgcccattctccgccccatggctgactaattttttttatttatgcagaggccgaggccgcctctgcctctgagctattccagaagtagtgaggaggcttttttggaggcctaggcttttgcaaaaagctcccgggagcttgtatatccattttcggatctgatcaagagacaggatgaggatcgtttcgcatgattgaacaagatggattgcacgcaggttctccggccgcttgggtggagaggctattcggctatgactgggcacaacagacaatcggctgctctgatgccgccgtgttccggctgtcagcgcaggggcgcccggttctttttgtcaagaccgacctgtccggtgccctgaatgaactgcaggacgaggcagcgcggctatcgtggctggccacgacgggcgttccttgcgcagctgtgctcgacgttgtcactgaagcgggaagggactggctgctattgggcgaagtgccggggcaggatctcctgtcatctcaccttgctcctgccgagaaagtatccatcatggctgatgcaatgcggcggctgcatacgcttgatccggctacctgcccattcgaccaccaagcgaaacatcgcatcgagcgagcacgtactcggatggaagccggtcttgtcgatcaggatgatctggacgaagagcatcaggggctcgcgccagccgaactgttcgccaggctcaaggcgcgcatgcccgacggcgaggatctcgtcgtgacccatggcgatgcctgcttgccgaatatcatggtggaaaatggccgcttttctggattcatcgactgtggccggctgggtgtggcggaccgctatcaggacatagcgttggctacccgtgatattgctgaagagcttggcggcgaatgggctgaccgcttcctcgtgctttacggtatcgccgctcccgattcgcagcgcatcgccttctatcgccttcttgacgagttcttctgagcgggactctggggttcgaaatgaccgaccaagcgacgcccaacctgccatcacgagatttcgattccaccgccgccttctatgaaaggttgggcttcggaatcgttttccgggacgccggctggatgatcctccagcgcggggatctcatgctggagttcttcgcccaccccaacttgtttattgcagcttataatggttacaaataaagcaatagcatcacaaatttcacaaataaagcatttttttcactgcattctagttgtggtttgtccaaactcatcaatgtatcttatcatgtctgtataccgtcgacctctagctagagcttggcgtaatcatggtcatagctgtttcctgtgtgaaattgttatccgctcacaattccacacaacatacgagccggaagcataaagtgtaaagcctggggtgcctaatgagtgagctaactcacattaattgcgttgcgctcactgcccgctttccagtcgggaaacctgtcgtgccagctgcattaatgaatcggccaacgcgcggggagaggcggtttgcgtattgggcgctcttccgcttcctcgctcactgactcgctgcgctcggtcgttcggctgcggcgagcggtatcagctcactcaaaggcggtaatacggttatccacagaatcaggggataacgcaggaaagaacatgtgagcaaaaggccagcaaaaggccaggaaccgtaaaaaggccgcgttgctggcgtttttccataggctccgcccccctgacgagcatcacaaaaatcgacgctcaagtcagaggtggcgaaacccgacaggactataaagataccaggcgtttccccctggaagctccctcgtgcgctctcctgttccgaccctgccgcttaccggatacctgtccgcctttctcccttcgggaagcgtggcgctttctcatagctcacgctgtaggtatctcagttcggtgtaggtcgttcgctccaagctgggctgtgtgcacgaaccccccgttcagcccgaccgctgcgccttatccggtaactatcgtcttgagtccaacccggtaagacacgacttatcgccactggcagcagccactggtaacaggattagcagagcgaggtatgtaggcggtgctacagagttcttgaagtggtggcctaactacggctacactagaagaacagtatttggtatctgcgctctgctgaagccagttaccttcggaaaaagagttggtagctcttgatccggcaaacaaaccaccgctggtagcggtggtttttttgtttgcaagcagcagattacgcgcagaaaaaaaggatctcaagaagatcctttgatcttttctacggggtctgacgctcagtggaacgaaaactcacgttaagggattttggtcatgagattatcaaaaaggatcttcacctagatccttttaaattaaaaatgaagttttaaatcaatctaaagtatatatgagtaaacttggtctgacagttaccaatgcttaatcagtgaggcacctatctcagcgatctgtctatttcgttcatccatagttgcctgactccccgtcgtgtagataactacgatacgggagggcttaccatctggccccagtgctgcaatgataccgcgagacccacgctcaccggctccagatttatcagcaataaaccagccagccggaagggccgagcgcagaagtggtcctgcaactttatccgcctccatccagtctattaattgttgccgggaagctagagtaagtagttcgccagttaatagtttgcgcaacgttgttgccattgctacaggcatcgtggtgtcacgctcgtcgtttggtatggcttcattcagctccggttcccaacgatcaaggcgagttacatgatcccccatgttgtgcaaaaaagcggttagctccttcggtcctccgatcgttgtcagaagtaagttggccgcagtgttatcactcatggttatggcagcactgcataattctcttactgtcatgccatccgtaagatgcttttctgtgactggtgagtactcaaccaagtcattctgagaatagtgtatgcggcgaccgagttgctcttgcccggcgtcaatacgggataataccgcgccacatagcagaactttaaaagtgctcatcattggaaaacgttcttcggggcgaaaactctcaaggatcttaccgctgttgagatccagttcgatgtaacccactcgtgcacccaactgatcttcagcatcttttactttcaccagcgtttctgggtgagcaaaaacaggaaggcaaaatgccgcaaaaaagggaataagggcgacacggaaatgttgaatactcatactcttcctttttcaatattattgaagcatttatcagggttattgtctcatgagcggatacatatttgaatgtatttagaaaaataaacaaataggggttccgcgcacatttccccgaaaagtgccacctgacgtc

SEQ ID NO: 41 - protein, 472 aa, artificial
  GAP43-SSGSSGTG-meGFP-PRGrh
MLCCMRRTKQVEKNDEDQNSSGSSGTGSKGEELFTGVVPILVELDGDVNGHKFSVSGEGEGDATYGKLTLKFICTTGKLPVPWPTLVTTLTYGVQCFSRYPDHMKRHDFFKSAMPEGYVQERTIFFKDDGNYKTRAEVKFEGDTLVNRIELKGIDFKEDGNILGHKLEYNYNSHNVYIMADKQKNGIKANFKIRHNIESGGVQLADHYQQNTPIGDGPVLLPDNHYLSTQSKLSKDPNEKRDHMVLKERVTAAGITHGMDELYKGSSRELIIGPEEDYDPGYFNNESDIIFQDLEKLKSHPAYLVVFLRYILSQADPGPLLFYLCSEVYQQTNPKDSRSLGKDIWNIFLEKNAPLRVKIPEMLQAEIDLRLRNNEDPRNVLCEAQEAVMLEIQEQINDYRSKRTLGLGSLYGENDLLGLDGDPLRERQMAEKQLAALGDILSKYEEDRSAPMDFAVNTFMSHAGIRLRESRG

SEQ ID NO: 42 - DNA, 6811 bp, artificial
  GAP43-SSGSSGTG-meGFP-PRGrh
gacggatcgggagatctcccgatcccctatggtgcactctcagtacaatctgctctgatgccgcatagttaagccagtatctgctccctgcttgtgtgttggaggtcgctgagtagtgcgcgagcaaaatttaagctacaacaaggcaaggcttgaccgacaattgcatgaagaatctgcttagggttaggcgttttgcgctgcttcgcgatgtacgggccagatatacgcgttgacattgattattgactagttattaatagtaatcaattacggggtcattagttcatagcccatatatggagttccgcgttacataacttacggtaaatggcccgcctggctgaccgcccaacgacccccgcccattgacgtcaataatgacgtatgttcccatagtaacgccaatagggactttccattgacgtcaatgggtggagtatttacggtaaactgcccacttggcagtacatcaagtgtatcatatgccaagtacgccccctattgacgtcaatgacggtaaatggcccgcctggcattatgcccagtacatgaccttatgggactttcctacttggcagtacatctacgtattagtcatcgctattaccatggtgatgcggttttggcagtacatcaatgggcgtggatagcggtttgactcacggggatttccaagtctccaccccattgacgtcaatgggagtttgttttggcaccaaaatcaacgggactttccaaaatgtcgtaacaactccgccccattgacgcaaatgggcggtaggcgtgtacggtgggaggtctatataagcagagctctctggctaactagagaacccactgcttactggcttatcgaaattaatacgactcactatagggagacccaagctggctagcgtttaaacttaagcttggtaccgacggaccatgctgtgctgtatgagaagaaccaaacaggttgaaaagaatgatgaggaccagaattcctccggatcgtctggaaccggttctaaaggagaagaacttttcactggagttgtcccaattcttgttgaattagatggtgatgttaatgggcacaaattttctgtcagtggagagggtgaaggtgatgcaacatacggaaaacttacccttaaatttatttgcactactggaaaactacctgttccttggccaacacttgtcactactttaacttatggtgttcaatgcttttcaagatacccagatcatatgaaacggcatgactttttcaagagtgccatgcccgaaggttatgtacaggaaagaactatatttttcaaagatgacgggaactacaagacacgtgctgaagtcaagtttgaaggtgatacccttgttaatagaatcgagttaaaaggtattgattttaaagaagatggaaacattcttggacacaaattggaatacaactataactcacacaatgtatacatcatggcagacaaacaaaagaatggaatcaaagctaacttcaaaattagacacaacattgagtccggaggcgttcaactagcagaccattatcaacaaaatactccaattggcgatggccctgtccttttaccagacaaccattacctgtccacacaatctaagctttcgaaagatcccaacgaaaagagagaccacatggtccttaaagagagggtaacagctgctgggattacacatggcatggacgagctgtacaagggatcctctagagagctgattattggcccagaggaagattatgacccaggttatttcaacaatgagagtgacatcatcttccaagatcttgaaaaactgaagtcacatccagcttacttggtagtttttctacgttacatcctctctcaggcagaccctggccccctgcttttttatttgtgttcagaagtttatcaacagacaaatcccaaagattcccgaagtctggggaaagacatctggaacattttcctggagaaaaatgcgcctctcagagtgaagatccctgagatgttgcaggctgaaattgacctacgcctgcggaacaatgaggaccctcgcaatgtgctctgtgaagctcaggaggcagtcatgctggaaatccaggagcagatcaacgactacagatccaagcgtactctgggcctgggcagcctctatggtgaaaatgacctgctaggcctggatggggaccctcttcgagaacgccaaatggctgagaagcagctggctgcccttggagatatcttgtccaaatatgaggaagatcggagtgcccccatggactttgctgttaatacctttatgagccacgctgggatccgtcttcgggagtctcgaggataatgaaggtggcggccgctcgaaactagagggcccgtttaaacccgctgatcagcctcgactgtgccttctagttgccagccatctgttgtttgcccctcccccgtgccttccttgaccctggaaggtgccactcccactgtcctttcctaataaaatgaggaaattgcatcgcattgtctgagtaggtgtcattctattctggggggtggggtggggcaggacagcaagggggaggattgggaagacaatagcaggcatgctggggatgcggtgggctctatggcttctgaggcggaaagaaccagctggggctctagggggtatccccacgcgccctgtagcggcgcattaagcgcggcgggtgtggtggttacgcgcagcgtgaccgctacacttgccagcgccctagcgcccgctcctttcgctttcttcccttcctttctcgccacgttcgccggctttccccgtcaagctctaaatcgggggctccctttagggttccgatttagtgctttacggcacctcgaccccaaaaaacttgattagggtgatggttcacgtagtgggccatcgccctgatagacggtttttcgccctttgacgttggagtccacgttctttaatagtggactcttgttccaaactggaacaacactcaaccctatctcggtctattcttttgatttataagggattttgccgatttcggcctattggttaaaaaatgagctgatttaacaaaaatttaacgcgaattaattctgtggaatgtgtgtcagttagggtgtggaaagtccccaggctccccagcaggcagaagtatgcaaagcatgcatctcaattagtcagcaaccaggtgtggaaagtccccaggctccccagcaggcagaagtatgcaaagcatgcatctcaattagtcagcaaccatagtcccgcccctaactccgcccatcccgcccctaactccgcccagttccgcccattctccgccccatggctgactaattttttttatttatgcagaggccgaggccgcctctgcctctgagctattccagaagtagtgaggaggcttttttggaggcctaggcttttgcaaaaagctcccgggagcttgtatatccattttcggatctgatcaagagacaggatgaggatcgtttcgcatgattgaacaagatggattgcacgcaggttctccggccgcttgggtggagaggctattcggctatgactgggcacaacagacaatcggctgctctgatgccgccgtgttccggctgtcagcgcaggggcgcccggttctttttgtcaagaccgacctgtccggtgccctgaatgaactgcaggacgaggcagcgcggctatcgtggctggccacgacgggcgttccttgcgcagctgtgctcgacgttgtcactgaagcgggaagggactggctgctattgggcgaagtgccggggcaggatctcctgtcatctcaccttgctcctgccgagaaagtatccatcatggctgatgcaatgcggcggctgcatacgcttgatccggctacctgcccattcgaccaccaagcgaaacatcgcatcgagcgagcacgtactcggatggaagccggtcttgtcgatcaggatgatctggacgaagagcatcaggggctcgcgccagccgaactgttcgccaggctcaaggcgcgcatgcccgacggcgaggatctcgtcgtgacccatggcgatgcctgcttgccgaatatcatggtggaaaatggccgcttttctggattcatcgactgtggccggctgggtgtggcggaccgctatcaggacatagcgttggctacccgtgatattgctgaagagcttggcggcgaatgggctgaccgcttcctcgtgctttacggtatcgccgctcccgattcgcagcgcatcgccttctatcgccttcttgacgagttcttctgagcgggactctggggttcgaaatgaccgaccaagcgacgcccaacctgccatcacgagatttcgattccaccgccgccttctatgaaaggttgggcttcggaatcgttttccgggacgccggctggatgatcctccagcgcggggatctcatgctggagttcttcgcccaccccaacttgtttattgcagcttataatggttacaaataaagcaatagcatcacaaatttcacaaataaagcatttttttcactgcattctagttgtggtttgtccaaactcatcaatgtatcttatcatgtctgtataccgtcgacctctagctagagcttggcgtaatcatggtcatagctgtttcctgtgtgaaattgttatccgctcacaattccacacaacatacgagccggaagcataaagtgtaaagcctggggtgcctaatgagtgagctaactcacattaattgcgttgcgctcactgcccgctttccagtcgggaaacctgtcgtgccagctgcattaatgaatcggccaacgcgcggggagaggcggtttgcgtattgggcgctcttccgcttcctcgctcactgactcgctgcgctcggtcgttcggctgcggcgagcggtatcagctcactcaaaggcggtaatacggttatccacagaatcaggggataacgcaggaaagaacatgtgagcaaaaggccagcaaaaggccaggaaccgtaaaaaggccgcgttgctggcgtttttccataggctccgcccccctgacgagcatcacaaaaatcgacgctcaagtcagaggtggcgaaacccgacaggactataaagataccaggcgtttccccctggaagctccctcgtgcgctctcctgttccgaccctgccgcttaccggatacctgtccgcctttctcccttcgggaagcgtggcgctttctcatagctcacgctgtaggtatctcagttcggtgtaggtcgttcgctccaagctgggctgtgtgcacgaaccccccgttcagcccgaccgctgcgccttatccggtaactatcgtcttgagtccaacccggtaagacacgacttatcgccactggcagcagccactggtaacaggattagcagagcgaggtatgtaggcggtgctacagagttcttgaagtggtggcctaactacggctacactagaagaacagtatttggtatctgcgctctgctgaagccagttaccttcggaaaaagagttggtagctcttgatccggcaaacaaaccaccgctggtagcggtggtttttttgtttgcaagcagcagattacgcgcagaaaaaaaggatctcaagaagatcctttgatcttttctacggggtctgacgctcagtggaacgaaaactcacgttaagggattttggtcatgagattatcaaaaaggatcttcacctagatccttttaaattaaaaatgaagttttaaatcaatctaaagtatatatgagtaaacttggtctgacagttaccaatgcttaatcagtgaggcacctatctcagcgatctgtctatttcgttcatccatagttgcctgactccccgtcgtgtagataactacgatacgggagggcttaccatctggccccagtgctgcaatgataccgcgagacccacgctcaccggctccagatttatcagcaataaaccagccagccggaagggccgagcgcagaagtggtcctgcaactttatccgcctccatccagtctattaattgttgccgggaagctagagtaagtagttcgccagttaatagtttgcgcaacgttgttgccattgctacaggcatcgtggtgtcacgctcgtcgtttggtatggcttcattcagctccggttcccaacgatcaaggcgagttacatgatcccccatgttgtgcaaaaaagcggttagctccttcggtcctccgatcgttgtcagaagtaagttggccgcagtgttatcactcatggttatggcagcactgcataattctcttactgtcatgccatccgtaagatgcttttctgtgactggtgagtactcaaccaagtcattctgagaatagtgtatgcggcgaccgagttgctcttgcccggcgtcaatacgggataataccgcgccacatagcagaactttaaaagtgctcatcattggaaaacgttcttcggggcgaaaactctcaaggatcttaccgctgttgagatccagttcgatgtaacccactcgtgcacccaactgatcttcagcatcttttactttcaccagcgtttctgggtgagcaaaaacaggaaggcaaaatgccgcaaaaaagggaataagggcgacacggaaatgttgaatactcatactcttcctttttcaatattattgaagcatttatcagggttattgtctcatgagcggatacatatttgaatgtatttagaaaaataaacaaataggggttccgcgcacatttccccgaaaagtgccacctgacgtc

SEQ ID NO: 43 - protein, 377 aa, artificial
  G 13(Q226L)
MADFLPSRSVLSVCFPGCLLTSGEAEQQRKSKEIDKCLSREKTYVKRLVKILLLGAGESGKSTFLKQMRIIHGQDFDQRAREEFRPTIYSNVIKGMRVLVDAREKLHIPWGDNSNQQHGDKMMSFDTRAPMAAQGMVETRVFLQYLPAIRALWADSGIQNAYDRRREFQLGESVKYFLDNLDKLGEPDYIPSQQDILLARRPTKGIHEYDFEIKNVPFKMVDVGGLRSERKRWFECFDSVTSILFLVSSSEFDQVLMEDRLTNRLTESLNIFETIVNNRVFSNVSIILFLNKTDLLEEKVQIVSIKDYFLEFEGDPHCLRDVQKFLVECFRNKRRDQQQKPLYHHFTTAINTENIRLVFRDVKDTILHDNLKQLMLQ

SEQ ID NO: 44 - DNA, 6507 bp, artificial
  Galfa13(Q226L)
gacggatcgggagatctcccgatcccctatggtgcactctcagtacaatctgctctgatgccgcatagttaagccagtatctgctccctgcttgtgtgttggaggtcgctgagtagtgcgcgagcaaaatttaagctacaacaaggcaaggcttgaccgacaattgcatgaagaatctgcttagggttaggcgttttgcgctgcttcgcgatgtacgggccagatatacgcgttgacattgattattgactagttattaatagtaatcaattacggggtcattagttcatagcccatatatggagttccgcgttacataacttacggtaaatggcccgcctggctgaccgcccaacgacccccgcccattgacgtcaataatgacgtatgttcccatagtaacgccaatagggactttccattgacgtcaatgggtggagtatttacggtaaactgcccacttggcagtacatcaagtgtatcatatgccaagtacgccccctattgacgtcaatgacggtaaatggcccgcctggcattatgcccagtacatgaccttatgggactttcctacttggcagtacatctacgtattagtcatcgctattaccatggtgatgcggttttggcagtacatcaatgggcgtggatagcggtttgactcacggggatttccaagtctccaccccattgacgtcaatgggagtttgttttggcaccaaaatcaacgggactttccaaaatgtcgtaacaactccgccccattgacgcaaatgggcggtaggcgtgtacggtgggaggtctatataagcagagctctctggctaactagagaacccactgcttactggcttatcgaaattaatacgactcactatagggagacccaagctggctagcgtttaaacttaagcttggtaccaccatggcggacttcctgccgtcgcggtccgtgctgtccgtgtgcttccccggctgcctgctgacgagtggcgaggccgagcagcaacgcaagtccaaggagatcgacaaatgcctgtctcgggaaaagacctatgtgaagcggctggtgaagatcctgctgctgggcgcgggcgagagcggcaagtccaccttcctgaagcagatgcggatcatccacgggcaggacttcgaccagcgcgcgcgcgaggagttccgccccaccatctacagcaacgtgatcaaaggtatgagggtgctggttgatgctcgagagaagcttcatattccctggggagacaactcaaaccaacaacatggagataagatgatgtcgtttgatacccgggcccccatggcagcccaaggaatggtggaaacaagggttttcttacaatatcttcctgctataagagcattatgggcagacagcggcatacagaatgcctatgaccggcgtcgagaatttcaactgggtgaatctgtaaaatatttcctggataacttggataaacttggagaaccagattatattccatcacaacaagatattctgcttgccagaagacccaccaaaggcatccatgaatacgactttgaaataaaaaatgttcctttcaaaatggttgatgtaggtggtctgagatcagaaaggaaacgttggtttgaatgtttcgacagtgtgacatcaatacttttccttgtttcctcaagtgaatttgaccaggtgcttatggaagatcgactgaccaatcgccttacagagtctctgaacatttttgaaacaatcgtcaataaccgggttttcagcaatgtctccataattctgttcttaaacaagacagacttgcttgaggagaaggtgcaaattgtgagcatcaaagactatttcctagaatttgaaggggatccccactgcttaagagacgtccaaaaattcctggtggaatgtttccggaacaaacgccgggaccagcaacagaagcccttataccaccacttcaccactgctatcaacacggagaacatccgccttgttttccgtgacgtgaaggatactattctgcatgacaacctcaagcagcttatgctacagtgatctagagatctctagagggcccgtttaaacccgctgatcagcctcgactgtgccttctagttgccagccatctgttgtttgcccctcccccgtgccttccttgaccctggaaggtgccactcccactgtcctttcctaataaaatgaggaaattgcatcgcattgtctgagtaggtgtcattctattctggggggtggggtggggcaggacagcaagggggaggattgggaagacaatagcaggcatgctggggatgcggtgggctctatggcttctgaggcggaaagaaccagctggggctctagggggtatccccacgcgccctgtagcggcgcattaagcgcggcgggtgtggtggttacgcgcagcgtgaccgctacacttgccagcgccctagcgcccgctcctttcgctttcttcccttcctttctcgccacgttcgccggctttccccgtcaagctctaaatcgggggctccctttagggttccgatttagtgctttacggcacctcgaccccaaaaaacttgattagggtgatggttcacgtagtgggccatcgccctgatagacggtttttcgccctttgacgttggagtccacgttctttaatagtggactcttgttccaaactggaacaacactcaaccctatctcggtctattcttttgatttataagggattttgccgatttcggcctattggttaaaaaatgagctgatttaacaaaaatttaacgcgaattaattctgtggaatgtgtgtcagttagggtgtggaaagtccccaggctccccagcaggcagaagtatgcaaagcatgcatctcaattagtcagcaaccaggtgtggaaagtccccaggctccccagcaggcagaagtatgcaaagcatgcatctcaattagtcagcaaccatagtcccgcccctaactccgcccatcccgcccctaactccgcccagttccgcccattctccgccccatggctgactaattttttttatttatgcagaggccgaggccgcctctgcctctgagctattccagaagtagtgaggaggcttttttggaggcctaggcttttgcaaaaagctcccgggagcttgtatatccattttcggatctgatcaagagacaggatgaggatcgtttcgcatgattgaacaagatggattgcacgcaggttctccggccgcttgggtggagaggctattcggctatgactgggcacaacagacaatcggctgctctgatgccgccgtgttccggctgtcagcgcaggggcgcccggttctttttgtcaagaccgacctgtccggtgccctgaatgaactgcaggacgaggcagcgcggctatcgtggctggccacgacgggcgttccttgcgcagctgtgctcgacgttgtcactgaagcgggaagggactggctgctattgggcgaagtgccggggcaggatctcctgtcatctcaccttgctcctgccgagaaagtatccatcatggctgatgcaatgcggcggctgcatacgcttgatccggctacctgcccattcgaccaccaagcgaaacatcgcatcgagcgagcacgtactcggatggaagccggtcttgtcgatcaggatgatctggacgaagagcatcaggggctcgcgccagccgaactgttcgccaggctcaaggcgcgcatgcccgacggcgaggatctcgtcgtgacccatggcgatgcctgcttgccgaatatcatggtggaaaatggccgcttttctggattcatcgactgtggccggctgggtgtggcggaccgctatcaggacatagcgttggctacccgtgatattgctgaagagcttggcggcgaatgggctgaccgcttcctcgtgctttacggtatcgccgctcccgattcgcagcgcatcgccttctatcgccttcttgacgagttcttctgagcgggactctggggttcgaaatgaccgaccaagcgacgcccaacctgccatcacgagatttcgattccaccgccgccttctatgaaaggttgggcttcggaatcgttttccgggacgccggctggatgatcctccagcgcggggatctcatgctggagttcttcgcccaccccaacttgtttattgcagcttataatggttacaaataaagcaatagcatcacaaatttcacaaataaagcatttttttcactgcattctagttgtggtttgtccaaactcatcaatgtatcttatcatgtctgtataccgtcgacctctagctagagcttggcgtaatcatggtcatagctgtttcctgtgtgaaattgttatccgctcacaattccacacaacatacgagccggaagcataaagtgtaaagcctggggtgcctaatgagtgagctaactcacattaattgcgttgcgctcactgcccgctttccagtcgggaaacctgtcgtgccagctgcattaatgaatcggccaacgcgcggggagaggcggtttgcgtattgggcgctcttccgcttcctcgctcactgactcgctgcgctcggtcgttcggctgcggcgagcggtatcagctcactcaaaggcggtaatacggttatccacagaatcaggggataacgcaggaaagaacatgtgagcaaaaggccagcaaaaggccaggaaccgtaaaaaggccgcgttgctggcgtttttccataggctccgcccccctgacgagcatcacaaaaatcgacgctcaagtcagaggtggcgaaacccgacaggactataaagataccaggcgtttccccctggaagctccctcgtgcgctctcctgttccgaccctgccgcttaccggatacctgtccgcctttctcccttcgggaagcgtggcgctttctcatagctcacgctgtaggtatctcagttcggtgtaggtcgttcgctccaagctgggctgtgtgcacgaaccccccgttcagcccgaccgctgcgccttatccggtaactatcgtcttgagtccaacccggtaagacacgacttatcgccactggcagcagccactggtaacaggattagcagagcgaggtatgtaggcggtgctacagagttcttgaagtggtggcctaactacggctacactagaagaacagtatttggtatctgcgctctgctgaagccagttaccttcggaaaaagagttggtagctcttgatccggcaaacaaaccaccgctggtagcggtttttttgtttgcaagcagcagattacgcgcagaaaaaaaggatctcaagaagatcctttgatcttttctacggggtctgacgctcagtggaacgaaaactcacgttaagggattttggtcatgagattatcaaaaaggatcttcacctagatccttttaaattaaaaatgaagttttaaatcaatctaaagtatatatgagtaaacttggtctgacagttaccaatgcttaatcagtgaggcacctatctcagcgatctgtctatttcgttcatccatagttgcctgactccccgtcgtgtagataactacgatacgggagggcttaccatctggccccagtgctgcaatgataccgcgagacccacgctcaccggctccagatttatcagcaataaaccagccagccggaagggccgagcgcagaagtggtcctgcaactttatccgcctccatccagtctattaattgttgccgggaagctagagtaagtagttcgccagttaatagtttgcgcaacgttgttgccattgctacaggcatcgtggtgtcacgctcgtcgtttggtatggcttcattcagctccggttcccaacgatcaaggcgagttacatgatcccccatgttgtgcaaaaaagcggttagctccttcggtcctccgatcgttgtcagaagtaagttggccgcagtgttatcactcatggttatggcagcactgcataattctcttactgtcatgccatccgtaagatgcttttctgtgactggtgagtactcaaccaagtcattctgagaatagtgtatgcggcgaccgagttgctcttgcccggcgtcaatacgggataataccgcgccacatagcagaactttaaaagtgctcatcattggaaaacgttcttcggggcgaaaactctcaaggatcttaccgctgttgagatccagttcgatgtaacccactcgtgcacccaactgatcttcagcatcttttactttcaccagcgtttctgggtgagcaaaaacaggaaggcaaaatgccgcaaaaaagggaataagggcgacacggaaatgttgaatactcatactcttcctttttcaatattattgaagcatttatcagggttattgtctcatgagcggatacatatttgaatgtatttagaaaaataaacaaataggggttccgcgcacatttccccgaaaagtgccacctgacgtc

SEQ ID NO: 45 - protein, 342 aa, artificial
  rhotekin-meGFP-GSGGSGG-hRas
MSSRGILEDLNMLYIRQMALSLEDTELQRKLDHEIRMRDGACKLLAACSQREQALEATKSLLVCNSRILSYMGELQRRKEAQVLEKTSRGKGEELFTGVVPILVELDGDVNGHKFSVSGEGEGDATYGKLTLKFICTTGKLPVPWPTLVTTLTYGVQCFSRYPDHMKRHDFFKSAMPEGYVQERTIFFKDDGNYKTRAEVKFEGDTLVNRIELKGIDFKEDGNILGHKLEYNYNSHNVYIMADKQKNGIKANFKIRHNIESGGVQLADHYQQNTPIGDGPVLLPDNHYLSTQSKLSKDPNEKRDHMVLKERVTAAGITHGMDELYKGSGGSGGCMSCKCVLS

SEQ ID NO: 46 - DNA, 6436 bp, artificial
  rhotekinRBD-meGFP-GSGGSGG-hRas
gacggatcgggagatctcccgatcccctatggtgcactctcagtacaatctgctctgatgccgcatagttaagccagtatctgctccctgcttgtgtgttggaggtcgctgagtagtgcgcgagcaaaatttaagctacaacaaggcaaggcttgaccgacaattgcatgaagaatctgcttagggttaggcgttttgcgctgcttcgcgatgtacgggccagatatacgcgttgacattgattattgactagttattaatagtaatcaattacggggtcattagttcatagcccatatatggagttccgcgttacataacttacggtaaatggcccgcctggctgaccgcccaacgacccccgcccattgacgtcaataatgacgtatgttcccatagtaacgccaatagggactttccattgacgtcaatgggtggagtatttacggtaaactgcccacttggcagtacatcaagtgtatcatatgccaagtacgccccctattgacgtcaatgacggtaaatggcccgcctggcattatgcccagtacatgaccttatgggactttcctacttggcagtacatctacgtattagtcatcgctattaccatggtgatgcggttttggcagtacatcaatgggcgtggatagcggtttgactcacggggatttccaagtctccaccccattgacgtcaatgggagtttgttttggcaccaaaatcaacgggactttccaaaatgtcgtaacaactccgccccattgacgcaaatgggcggtaggcgtgtacggtgggaggtctatataagcagagctctctggctaactagagaacccactgcttactggcttatcgaaattaatacgactcactatagggagacccaagctggctagcggtaccgagctcggatcactagtccagtgtggtggaattcacgcggaccatgtcttctagaggaatcctggaggacctcaatatgctctacatccggcagatggcactcagcctggaggacacagagctgcagaggaaactagatcatgagatccggatgagggatggggcctgcaagctgctggcagcctgctcccagcgagaacaggctctggaagccaccaagagcctgctggtgtgcaacagccgtattctcagctacatgggtgagctgcagcggcgaaaggaggcccaggtgctggagaagacatctcgaggtaaaggagaagaacttttcactggagttgtcccaattcttgttgaattagatggtgatgttaatgggcacaaattttctgtcagtggagagggtgaaggtgatgcaacatacggaaaacttacccttaaatttatttgcactactggaaaactacctgttccttggccaacacttgtcactactttaacttatggtgttcaatgcttttcaagatacccagatcatatgaaacggcatgactttttcaagagtgccatgcccgaaggttatgtacaggaaagaactatatttttcaaagatgacgggaactacaagacacgtgctgaagtcaagtttgaaggtgatacccttgttaatagaatcgagttaaaaggtattgattttaaagaagatggaaacattcttggacacaaattggaatacaactataactcacacaatgtatacatcatggcagacaaacaaaagaatggaatcaaagctaacttcaaaattagacacaacattgagtccggaggcgttcaactagcagaccattatcaacaaaatactccaattggcgatggccctgtccttttaccagacaaccattacctgtccacacaatctaagctttcgaaagatcccaacgaaaagagagaccacatggtccttaaagagagggtaacagctgctgggattacacatggcatggacgagctgtacaagggatccggtggaagtggaggctgcatgagctgcaagtgtgtgctgtcctaatgagcggccgcactagagggcccgggcccgtttaaacccgctgatcagcctcgactgtgccttctagttgccagccatctgttgtttgcccctcccccgtgccttccttgaccctggaaggtgccactcccactgtcctttcctaataaaatgaggaaattgcatcgcattgtctgagtaggtgtcattctattctggggggtggggtggggcaggacagcaagggggaggattgggaagacaatagcaggcatgctggggatgcggtgggctctatggcttctgaggcggaaagaaccagctggggctctagggggtatccccacgcgccctgtagcggcgcattaagcgcggcgggtgtggtggttacgcgcagcgtgaccgctacacttgccagcgccctagcgcccgctcctttcgctttcttcccttcctttctcgccacgttcgccggctttccccgtcaagctctaaatcgggggctccctttagggttccgatttagtgctttacggcacctcgaccccaaaaaacttgattagggtgatggttcacgtagtgggccatcgccctgatagacggtttttcgccctttgacgttggagtccacgttctttaatagtggactcttgttccaaactggaacaacactcaaccctatctcggtctattcttttgatttataagggattttgccgatttcggcctattggttaaaaaatgagctgatttaacaaaaatttaacgcgaattaattctgtggaatgtgtgtcagttagggtgtggaaagtccccaggctccccagcaggcagaagtatgcaaagcatgcatctcaattagtcagcaaccaggtgtggaaagtccccaggctccccagcaggcagaagtatgcaaagcatgcatctcaattagtcagcaaccatagtcccgcccctaactccgcccatcccgcccctaactccgcccagttccgcccattctccgccccatggctgactaattttttttatttatgcagaggccgaggccgcctctgcctctgagctattccagaagtagtgaggaggcttttttggaggcctaggcttttgcaaaaagctcccgggagcttgtatatccattttcggatctgatcaagagacaggatgaggatcgtttcgcatgattgaacaagatggattgcacgcaggttctccggccgcttgggtggagaggctattcggctatgactgggcacaacagacaatcggctgctctgatgccgccgtgttccggctgtcagcgcaggggcgcccggttctttttgtcaagaccgacctgtccggtgccctgaatgaactgcaggacgaggcagcgcggctatcgtggctggccacgacgggcgttccttgcgcagctgtgctcgacgttgtcactgaagcgggaagggactggctgctattgggcgaagtgccggggcaggatctcctgtcatctcaccttgctcctgccgagaaagtatccatcatggctgatgcaatgcggcggctgcatacgcttgatccggctacctgcccattcgaccaccaagcgaaacatcgcatcgagcgagcacgtactcggatggaagccggtcttgtcgatcaggatgatctggacgaagagcatcaggggctcgcgccagccgaactgttcgccaggctcaaggcgcgcatgcccgacggcgaggatctcgtcgtgacccatggcgatgcctgcttgccgaatatcatggtggaaaatggccgcttttctggattcatcgactgtggccggctgggtgtggcggaccgctatcaggacatagcgttggctacccgtgatattgctgaagagcttggcggcgaatgggctgaccgcttcctcgtgctttacggtatcgccgctcccgattcgcagcgcatcgccttctatcgccttcttgacgagttcttctgagcgggactctggggttcgaaatgaccgaccaagcgacgcccaacctgccatcacgagatttcgattccaccgccgccttctatgaaaggttgggcttcggaatcgttttccgggacgccggctggatgatcctccagcgcggggatctcatgctggagttcttcgcccaccccaacttgtttattgcagcttataatggttacaaataaagcaatagcatcacaaatttcacaaataaagcatttttttcactgcattctagttgtggtttgtccaaactcatcaatgtatcttatcatgtctgtataccgtcgacctctagctagagcttggcgtaatcatggtcatagctgtttcctgtgtgaaattgttatccgctcacaattccacacaacatacgagccggaagcataaagtgtaaagcctggggtgcctaatgagtgagctaactcacattaattgcgttgcgctcactgcccgctttccagtcgggaaacctgtcgtgccagctgcattaatgaatcggccaacgcgcggggagaggcggtttgcgtattgggcgctcttccgcttcctcgctcactgactcgctgcgctcggtcgttcggctgcggcgagcggtatcagctcactcaaaggcggtaatacggttatccacagaatcaggggataacgcaggaaagaacatgtgagcaaaaggccagcaaaaggccaggaaccgtaaaaaggccgcgttgctggcgtttttccataggctccgcccccctgacgagcatcacaaaaatcgacgctcaagtcagaggtggcgaaacccgacaggactataaagataccaggcgtttccccctggaagctccctcgtgcgctctcctgttccgaccctgccgcttaccggatacctgtccgcctttctcccttcgggaagcgtggcgctttctcatagctcacgctgtaggtatctcagttcggtgtaggtcgttcgctccaagctgggctgtgtgcacgaaccccccgttcagcccgaccgctgcgccttatccggtaactatcgtcttgagtccaacccggtaagacacgacttatcgccactggcagcagccactggtaacaggattagcagagcgaggtatgtaggcggtgctacagagttcttgaagtggtggcctaactacggctacactagaagaacagtatttggtatctgcgctctgctgaagccagttaccttcggaaaaagagttggtagctcttgatccggcaaacaaaccaccgctggtagcggtggtttttttgtttgcaagcagcagattacgcgcagaaaaaaaggatctcaagaagatcctttgatcttttctacggggtctgacgctcagtggaacgaaaactcacgttaagggattttggtcatgagattatcaaaaaggatcttcacctagatccttttaaattaaaaatgaagttttaaatcaatctaaagtatatatgagtaaacttggtctgacagttaccaatgcttaatcagtgaggcacctatctcagcgatctgtctatttcgttcatccatagttgcctgactccccgtcgtgtagataactacgatacgggagggcttaccatctggccccagtgctgcaatgataccgcgagacccacgctcaccggctccagatttatcagcaataaaccagccagccggaagggccgagcgcagaagtggtcctgcaactttatccgcctccatccagtctattaattgttgccgggaagctagagtaagtagttcgccagttaatagtttgcgcaacgttgttgccattgctacaggcatcgtggtgtcacgctcgtcgtttggtatggcttcattcagctccggttcccaacgatcaaggcgagttacatgatcccccatgttgtgcaaaaaagcggttagctccttcggtcctccgatcgttgtcagaagtaagttggccgcagtgttatcactcatggttatggcagcactgcataattctcttactgtcatgccatccgtaagatgcttttctgtgactggtgagtactcaaccaagtcattctgagaatagtgtatgcggcgaccgagttgctcttgcccggcgtcaatacgggataataccgcgccacatagcagaactttaaaagtgctcatcattggaaaacgttcttcggggcgaaaactctcaaggatcttaccgctgttgagatccagttcgatgtaacccactcgtgcacccaactgatcttcagcatcttttactttcaccagcgtttctgggtgagcaaaaacaggaaggcaaaatgccgcaaaaaagggaataagggcgacacggaaatgttgaatactcatactcttcctttttcaatattattgaagcatttatcagggttattgtctcatgagcggatacatatttgaatgtatttagaaaaataaacaaataggggttccgcgcacatttccccgaaaagtgccacctgacgtc

SEQ ID NO: 47 - protein, 193 aa, artificial
  RhoA(Q63L)
MAAIRKKLVIVGDGACGKTCLLIVFSKDQFPEVYVPTVFENYVADIEVDGKQVELALWDTAGLEDYDRLRPLSYPDTDVILMCFSIDSPDSLENIPEKWTPEVKHFCPNVPIILVGNKKDLRNDEHTRRELAKMKQEPVKPEEGRDMANRIGAFGYMECSAKTKDGVREVFEMATRAALQARRGKKKSGCLVL

SEQ ID NO: 48 - DNA, 6565 bp, artificial
  RhoA(Q63L)
tagttattaatagtaatcaattacggggtcattagttcatagcccatatatggagttccgcgttacataacttacggtaaatggcccgcctggctgaccgcccaacgacccccgcccattgacgtcaataatgacgtatgttcccatagtaacgccaatagggactttccattgacgtcaatgggtggagtatttacggtaaactgcccacttggcagtacatcaagtgtatcatatgccaagtacgccccctattgacgtcaatgacggtaaatggcccgcctggcattatgcccagtacatgaccttatgggactttcctacttggcagtacatctacgtattagtcatcgctattaccatggtgatgcggttttggcagtacatcaatgggcgtggatagcggtttgactcacggggatttccaagtctccaccccattgacgtcaatgggagtttgttttggcaccaaaatcaacgggactttccaaaatgtcgtaacaactccgccccattgacgcaaatgggcggtaggcgtgtacggtgggaggtctatataagcagagctggtttagtgaaccgtcagatccgctagcctcgacttgagctcggatccggtggttctggttctggtggtaccatggctgccatccggaagaaactggtgattgttggtgatggagcctgtggaaagacatgcttgctcatagtcttcagcaaggaccagttcccagaggtgtatgtgcccacagtgtttgagaactatgtggcagatatcgaggtggatggaaagcaggtagagttggctttgtgggacacagctgggctggaagattatgatcgcctgaggcccctctcctacccagataccgatgttatactgatgtgtttttccatcgacagccctgatagtttagaaaacatcccagaaaagtggaccccagaagtcaagcatttctgtcccaacgtgcccatcatcctggttgggaataagaaggatcttcggaatgatgagcacacaaggcgggagctagccaagatgaagcaggagccggtgaaacctgaagaaggcagagatatggcaaacaggattggcgcttttgggtacatggagtgttcagcaaagaccaaagatggagtgagagaggtttttgaaatggctacgagagctgctctgcaagctagacgtgggaagaaaaaatctgggtgccttgtcttgtaaaagcttgcggccgctcgagtctagaactagtttgagtcgagccgcggcaattccgcccccccccccccccctctccctcccccccccctaacgttactggccgaagccgcttggaataaggccggtgtgcgtttgtctatatgttattttccaccatattgccgtcttttggcaatgtgagggcccggaaacctggccctgtcttcttgacgagcattcctaggggtctttcccctctcgccaaaggaatgcaaggtctgttgaatgtcgtgaaggaagcagttcctctggaagcttcttgaagacaaacaacgtctgtagcgaccctttgcaggcagcggaaccccccacctggcaacaggtgcctctgcggccaaaagccacgtgtataagatacacctgcaaaggcggcacaaccccagtgccacgttgtgagttggatagttgtggaaagagtcaaatggctctcctcaagcgtattcaacaaggggctgaaggatgcccagaaggtaccccattgtatgggatctgatctggggcctcggtgcacatgctttacatgtgtttagtcgaggttaaaaaaacgtctaggccccccgaaccacggggacgtggttttcctttgaaaaacacgatgataatatggtgagcaagggcgaggaggataacatggccatcatcaaggagttcatgcgcttcaaggtgcacatggagggctccgtgaacggccacgagttcgagatcgagggcgagggcgagggccgcccctacgagggcacccagaccgccaagctgaaggtgaccaagggtggccccctgcccttcgcctgggacatcctgtcccctcagttcatgtacggctccaaggcctacgtgaagcaccccgccgacatccccgactacttgaagctgtccttccccgagggcttcaagtgggagcgcgtgatgaacttcgaggacggcggcgtggtgaccgtgacccaggactcctccctgcaggacggcgagttcatctacaaggtgaagctgcgcggcaccaacttcccctccgacggccccgtaatgcagaagaagaccatgggctgggaggcctcctccgagcggatgtaccccgaggacggcgccctgaagggcgagatcaagcagaggctgaagctgaaggacggcggccactacgacgctgaggtcaagaccacctacaaggccaagaagcccgtgcagctgcccggcgcctacaacgtcaacatcaagttggacatcacctcccacaacgaggactacaccatcgtggaacagtacgaacgcgccgagggccgccactccaccggcggcatggacgagctgtacaagtaaccgcggtcgacggtaccgcgggcccgggatctaagcttatcgataatcaacctctggattacaaaatttgtgaaagattgactggtattcttaactatgttgctccttttacgctatgtggatacgctgctttaatgcctttgtatcatgctattgcttcccgtatggctttcattttctcctccttgtataaatcctggttgctgtctctttatgaggagttgtggcccgttgtcaggcaacgtggcgtggtgtgcactgtgtttgctgacgcaacccccactggttggggcattgccaccacctgtcagctcctttccgggactttcgctttccccctccctattgccacggcggaactcatcgccgcctgccttgcccgctgctggacaggggctcggctgttgggcactgacaattccgtggtgttgtcggggaaatcatcgtcctttccttggctgctcgcctgtgttgccacctggattctgcgcgggacgtccttctgctacgtcccttcggccctcaatccagcggaccttccttcccgcggcctgctgccggctctgcggcctcttccgcgtcttcgccttcgccctcagacgagtcggatctccctttgggccgcctccccgcatcgataccgtggatcgatccaccggatctagataactgatcataatcagccataccacatttgtagaggttttacttgctttaaaaaacctcccacacctccccctgaacctgaaacataaaatgaatgcaattgttgttgttaacttgtttattgcagcttataatggttacaaataaagcaatagcatcacaaatttcacaaataaagcatttttttcactgcattctagttgtggtttgtccaaactcatcaatgtatcttaacgcgtaaattgtaagcgttaatattttgttaaaattcgcgttaaatttttgttaaatcagctcattttttaaccaataggccgaaatcggcaaaatcccttataaatcaaaagaatagaccgagatagggttgagtgttgttccagtttggaacaagagtccactattaaagaacgtggactccaacgtcaaagggcgaaaaaccgtctatcagggcgatggcccactacgtgaaccatcaccctaatcaagttttttggggtcgaggtgccgtaaagcactaaatcggaaccctaaagggagcccccgatttagagcttgacggggaaagccggcgaacgtggcgagaaaggaagggaagaaagcgaaaggagcgggcgctagggcgctggcaagtgtagcggtcacgctgcgcgtaaccaccacacccgccgcgcttaatgcgccgctacagggcgcgtcaggtggcacttttcggggaaatgtgcgcggaacccctatttgtttatttttctaaatacattcaaatatgtatccgctcatgagacaataaccctgataaatgcttcaataatattgaaaaaggaagagtcctgaggcggaaagaaccagctgtggaatgtgtgtcagttagggtgtggaaagtccccaggctccccagcaggcagaagtatgcaaagcatgcatctcaattagtcagcaaccaggtgtggaaagtccccaggctccccagcaggcagaagtatgcaaagcatgcatctcaattagtcagcaaccatagtcccgcccctaactccgcccatcccgcccctaactccgcccagttccgcccattctccgccccatggctgactaattttttttatttatgcagaggccgaggccgcctcggcctctgagctattccagaagtagtgaggaggcttttttggaggcctaggcttttgcaaagatcgatcaagagacaggatgaggatcgtttcgcatgattgaacaagatggattgcacgcaggttctccggccgcttgggtggagaggctattcggctatgactgggcacaacagacaatcggctgctctgatgccgccgtgttccggctgtcagcgcaggggcgcccggttctttttgtcaagaccgacctgtccggtgccctgaatgaactgcaagacgaggcagcgcggctatcgtggctggccacgacgggcgttccttgcgcagctgtgctcgacgttgtcactgaagcgggaagggactggctgctattgggcgaagtgccggggcaggatctcctgtcatctcaccttgctcctgccgagaaagtatccatcatggctgatgcaatgcggcggctgcatacgcttgatccggctacctgcccattcgaccaccaagcgaaacatcgcatcgagcgagcacgtactcggatggaagccggtcttgtcgatcaggatgatctggacgaagagcatcaggggctcgcgccagccgaactgttcgccaggctcaaggcgagcatgcccgacggcgaggatctcgtcgtgacccatggcgatgcctgcttgccgaatatcatggtggaaaatggccgcttttctggattcatcgactgtggccggctgggtgtggcggaccgctatcaggacatagcgttggctacccgtgatattgctgaagagcttggcggcgaatgggctgaccgcttcctcgtgctttacggtatcgccgctcccgattcgcagcgcatcgccttctatcgccttcttgacgagttcttctgagcgggactctggggttcgaaatgaccgaccaagcgacgcccaacctgccatcacgagatttcgattccaccgccgccttctatgaaaggttgggcttcggaatcgttttccgggacgccggctggatgatcctccagcgcggggatctcatgctggagttcttcgcccaccctagggggaggctaactgaaacacggaaggagacaataccggaaggaacccgcgctatgacggcaataaaaagacagaataaaacgcacggtgttgggtcgtttgttcataaacgcggggttcggtcccagggctggcactctgtcgataccccaccgagaccccattggggccaatacgcccgcgtttcttccttttccccaccccaccccccaagttcgggtgaaggcccagggctcgcagccaacgtcggggcggcaggccctgccatagcctcaggttactcatatatactttagattgatttaaaacttcatttttaatttaaaaggatctaggtgaagatcctttttgataatctcatgaccaaaatcccttaacgtgagttttcgttccactgagcgtcagaccccgtagaaaagatcaaaggatcttcttgagatcctttttttctgcgcgtaatctgctgcttgcaaacaaaaaaaccaccgctaccagcggtggtttgtttgccggatcaagagctaccaactctttttccgaaggtaactggcttcagcagagcgcagataccaaatactgtccttctagtgtagccgtagttaggccaccacttcaagaactctgtagcaccgcctacatacctcgctctgctaatcctgttaccagtggctgctgccagtggcgataagtcgtgtcttaccgggttggactcaagacgatagttaccggataaggcgcagcggtcgggctgaacggggggttcgtgcacacagcccagcttggagcgaacgacctacaccgaactgagatacctacagcgtgagctatgagaaagcgccacgcttcccgaagggagaaaggcggacaggtatccggtaagcggcagggtcggaacaggagagcgcacgagggagcttccagggggaaacgcctggtatctttatagtcctgtcgggtttcgccacctctgacttgagcgtcgatttttgtgatgctcgtcaggggggcggagcctatggaaaaacgccagcaacgcggcctttttacggttcctggccttttgctggccttttgctcacatgttctttcctgcgttatcccctgattctgtggataaccgtattaccgccatgcat

SEQ ID NO: 49 - protein, 351 aa, artificial
  GAP43-SSGSSGTG-meGFP-PAK1
MLCCMRRTKQVEKNDEDQNSSGSSGTGSKGEELFTGVVPILVELDGDVNGHKFSVSGEGEGDATYGKLTLKFICTTGKLPVPWPTLVTTLTYGVQCFSRYPDHMKRHDFFKSAMPEGYVQERTIFFKDDGNYKTRAEVKFEGDTLVNRIELKGIDFKEDGNILGHKLEYNYNSHNVYIMADKQKNGIKANFKIRHNIESGGVQLADHYQQNTPIGDGPVLLPDNHYLSTQSKLSKDPNEKRDHMVLKERVTAAGITHGMDSRNKKKEKERPEISLPSDFEHTIHVGFDAVTGEFTGMPEQWARLLQTSNITKSEQKKNPQAVLDVLEFYNSKKTSNSQKYMSFTDKSPSRG

SEQ ID NO: 50 - DNA, 6448 bp, artificial
  GAP43-SSGSSGTG-meGFP-PAK1
gacggatcgggagatctcccgatcccctatggtgcactctcagtacaatctgctctgatgccgcatagttaagccagtatctgctccctgcttgtgtgttggaggtcgctgagtagtgcgcgagcaaaatttaagctacaacaaggcaaggcttgaccgacaattgcatgaagaatctgcttagggttaggcgttttgcgctgcttcgcgatgtacgggccagatatacgcgttgacattgattattgactagttattaatagtaatcaattacggggtcattagttcatagcccatatatggagttccgcgttacataacttacggtaaatggcccgcctggctgaccgcccaacgacccccgcccattgacgtcaataatgacgtatgttcccatagtaacgccaatagggactttccattgacgtcaatgggtggagtatttacggtaaactgcccacttggcagtacatcaagtgtatcatatgccaagtacgccccctattgacgtcaatgacggtaaatggcccgcctggcattatgcccagtacatgaccttatgggactttcctacttggcagtacatctacgtattagtcatcgctattaccatggtgatgcggttttggcagtacatcaatgggcgtggatagcggtttgactcacggggatttccaagtctccaccccattgacgtcaatgggagtttgttttggcaccaaaatcaacgggactttccaaaatgtcgtaacaactccgccccattgacgcaaatgggcggtaggcgtgtacggtgggaggtctatataagcagagctctctggctaactagagaacccactgcttactggcttatcgaaattaatacgactcactatagggagacccaagctggctagcgtttaaacttaagcttggtaccgacggaccatgctgtgctgtatgagaagaaccaaacaggttgaaaagaatgatgaggaccagaattcctccggatcgtctggaaccggttctaaaggagaagaacttttcactggagttgtcccaattcttgttgaattagatggtgatgttaatgggcacaaattttctgtcagtggagagggtgaaggtgatgcaacatacggaaaacttacccttaaatttatttgcactactggaaaactacctgttccttggccaacacttgtcactactttaacttatggtgttcaatgcttttcaagatacccagatcatatgaaacggcatgactttttcaagagtgccatgcccgaaggttatgtacaggaaagaactatatttttcaaagatgacgggaactacaagacacgtgctgaagtcaagtttgaaggtgatacccttgttaatagaatcgagttaaaaggtattgattttaaagaagatggaaacattcttggacacaaattggaatacaactataactcacacaatgtatacatcatggcagacaaacaaaagaatggaatcaaagctaacttcaaaattagacacaacattgagtccggaggcgttcaactagcagaccattatcaacaaaatactccaattggcgatggccctgtccttttaccagacaaccattacctgtccacacaatctaagctttcgaaagatcccaacgaaaagagagaccacatggtccttaaagagagggtaacagctgctgggattacacatggcatggactctagaaataagaagaaagagaaagagcggccagagatttctctcccttcagattttgaacacacaattcatgtcggttttgatgctgtcacaggggagtttacgggaatgccagagcagtgggcccgcttgcttcagacatcaaatatcactaagtcggagcagaagaaaaacccgcaggctgttctggatgtgttggagttttacaactcgaagaagacatccaacagccagaaatacatgagctttacagataagtcaccttctcgaggataatgaaggtggcggccgctcgaaactagagggcccgtttaaacccgctgatcagcctcgactgtgccttctagttgccagccatctgttgtttgcccctcccccgtgccttccttgaccctggaaggtgccactcccactgtcctttcctaataaaatgaggaaattgcatcgcattgtctgagtaggtgtcattctattctggggggtggggtggggcaggacagcaagggggaggattgggaagacaatagcaggcatgctggggatgcggtgggctctatggcttctgaggcggaaagaaccagctggggctctagggggtatccccacgcgccctgtagcggcgcattaagcgcggcgggtgtggtggttacgcgcagcgtgaccgctacacttgccagcgccctagcgcccgctcctttcgctttcttcccttcctttctcgccacgttcgccggctttccccgtcaagctctaaatcgggggctccctttagggttccgatttagtgctttacggcacctcgaccccaaaaaacttgattagggtgatggttcacgtagtgggccatcgccctgatagacggtttttcgccctttgacgttggagtccacgttctttaatagtggactcttgttccaaactggaacaacactcaaccctatctcggtctattcttttgatttataagggattttgccgatttcggcctattggttaaaaaatgagctgatttaacaaaaatttaacgcgaattaattctgtggaatgtgtgtcagttagggtgtggaaagtccccaggctccccagcaggcagaagtatgcaaagcatgcatctcaattagtcagcaaccaggtgtggaaagtccccaggctccccagcaggcagaagtatgcaaagcatgcatctcaattagtcagcaaccatagtcccgcccctaactccgcccatcccgcccctaactccgcccagttccgcccattctccgccccatggctgactaattttttttatttatgcagaggccgaggccgcctctgcctctgagctattccagaagtagtgaggaggcttttttggaggcctaggcttttgcaaaaagctcccgggagcttgtatatccattttcggatctgatcaagagacaggatgaggatcgtttcgcatgattgaacaagatggattgcacgcaggttctccggccgcttgggtggagaggctattcggctatgactgggcacaacagacaatcggctgctctgatgccgccgtgttccggctgtcagcgcaggggcgcccggttctttttgtcaagaccgacctgtccggtgccctgaatgaactgcaggacgaggcagcgcggctatcgtggctggccacgacgggcgttccttgcgcagctgtgctcgacgttgtcactgaagcgggaagggactggctgctattgggcgaagtgccggggcaggatctcctgtcatctcaccttgctcctgccgagaaagtatccatcatggctgatgcaatgcggcggctgcatacgcttgatccggctacctgcccattcgaccaccaagcgaaacatcgcatcgagcgagcacgtactcggatggaagccggtcttgtcgatcaggatgatctggacgaagagcatcaggggctcgcgccagccgaactgttcgccaggctcaaggcgcgcatgcccgacggcgaggatctcgtcgtgacccatggcgatgcctgcttgccgaatatcatggtggaaaatggccgcttttctggattcatcgactgtggccggctgggtgtggcggaccgctatcaggacatagcgttggctacccgtgatattgctgaagagcttggcggcgaatgggctgaccgcttcctcgtgctttacggtatcgccgctcccgattcgcagcgcatcgccttctatcgccttcttgacgagttcttctgagcgggactctggggttcgaaatgaccgaccaagcgacgcccaacctgccatcacgagatttcgattccaccgccgccttctatgaaaggttgggcttcggaatcgttttccgggacgccggctggatgatcctccagcgcggggatctcatgctggagttcttcgcccaccccaacttgtttattgcagcttataatggttacaaataaagcaatagcatcacaaatttcacaaataaagcatttttttcactgcattctagttgtggtttgtccaaactcatcaatgtatcttatcatgtctgtataccgtcgacctctagctagagcttggcgtaatcatggtcatagctgtttcctgtgtgaaattgttatccgctcacaattccacacaacatacgagccggaagcataaagtgtaaagcctggggtgcctaatgagtgagctaactcacattaattgcgttgcgctcactgcccgctttccagtcgggaaacctgtcgtgccagctgcattaatgaatcggccaacgcgcggggagaggcggtttgcgtattgggcgctcttccgcttcctcgctcactgactcgctgcgctcggtcgttcggctgcggcgagcggtatcagctcactcaaaggcggtaatacggttatccacagaatcaggggataacgcaggaaagaacatgtgagcaaaaggccagcaaaaggccaggaaccgtaaaaaggccgcgttgctggcgtttttccataggctccgcccccctgacgagcatcacaaaaatcgacgctcaagtcagaggtggcgaaacccgacaggactataaagataccaggcgtttccccctggaagctccctcgtgcgctctcctgttccgaccctgccgcttaccggatacctgtccgcctttctcccttcgggaagcgtggcgctttctcatagctcacgctgtaggtatctcagttcggtgtaggtcgttcgctccaagctgggctgtgtgcacgaaccccccgttcagcccgaccgctgcgccttatccggtaactatcgtcttgagtccaacccggtaagacacgacttatcgccactggcagcagccactggtaacaggattagcagagcgaggtatgtaggcggtgctacagagttcttgaagtggtggcctaactacggctacactagaagaacagtatttggtatctgcgctctgctgaagccagttaccttcggaaaaagagttggtagctcttgatccggcaaacaaaccaccgctggtagcggtggtttttttgtttgcaagcagcagattacgcgcagaaaaaaaggatctcaagaagatcctttgatcttttctacggggtctgacgctcagtggaacgaaaactcacgttaagggattttggtcatgagattatcaaaaaggatcttcacctagatccttttaaattaaaaatgaagttttaaatcaatctaaagtatatatgagtaaacttggtctgacagttaccaatgcttaatcagtgaggcacctatctcagcgatctgtctatttcgttcatccatagttgcctgactccccgtcgtgtagataactacgatacgggagggcttaccatctggccccagtgctgcaatgataccgcgagacccacgctcaccggctccagatttatcagcaataaaccagccagccggaagggccgagcgcagaagtggtcctgcaactttatccgcctccatccagtctattaattgttgccgggaagctagagtaagtagttcgccagttaatagtttgcgcaacgttgttgccattgctacaggcatcgtggtgtcacgctcgtcgtttggtatggcttcattcagctccggttcccaacgatcaaggcgagttacatgatcccccatgttgtgcaaaaaagcggttagctccttcggtcctccgatcgttgtcagaagtaagttggccgcagtgttatcactcatggttatggcagcactgcataattctcttactgtcatgccatccgtaagatgcttttctgtgactggtgagtactcaaccaagtcattctgagaatagtgtatgcggcgaccgagttgctcttgcccggcgtcaatacgggataataccgcgccacatagcagaactttaaaagtgctcatcattggaaaacgttcttcggggcgaaaactctcaaggatcttaccgctgttgagatccagttcgatgtaacccactcgtgcacccaactgatcttcagcatcttttactttcaccagcgtttctgggtgagcaaaaacaggaaggcaaaatgccgcaaaaaagggaataagggcgacacggaaatgttgaatactcatactcttcctttttcaatattattgaagcatttatcagggttattgtctcatgagcggatacatatttgaatgtatttagaaaaataaacaaataggggttccgcgcacatttccccgaaaagtgccacctgacgtc

SEQ ID NO: 51 - protein, 202 aa, artificial
  Rac1(Q61L)
MGYPYDVPDYAQAIKCVVVGDGAVGKTCLLISYTTNAFPGEYIPTVFDNYSANVMVDGKPVNLGLWDTAGLEDYDRLRPLSYPQTDVFLICFSLVSPASFENVRAKWYPEVRHHCPNTPIILVGTKLDLRDDKDTIEKLKEKKLTPITYPQGLAMAKEIGAVKYLECSALTQRGLKTVFDEAIRAVLCPPPVKKRKRKCLLL

SEQ ID NO: 52 - DNA, 6586 bp, artificial
  Rac1(Q61L)
tagttattaatagtaatcaattacggggtcattagttcatagcccatatatggagttccgcgttacataacttacggtaaatggcccgcctggctgaccgcccaacgacccccgcccattgacgtcaataatgacgtatgttcccatagtaacgccaatagggactttccattgacgtcaatgggtggagtatttacggtaaactgcccacttggcagtacatcaagtgtatcatatgccaagtacgccccctattgacgtcaatgacggtaaatggcccgcctggcattatgcccagtacatgaccttatgggactttcctacttggcagtacatctacgtattagtcatcgctattaccatggtgatgcggttttggcagtacatcaatgggcgtggatagcggtttgactcacggggatttccaagtctccaccccattgacgtcaatgggagtttgttttggcaccaaaatcaacgggactttccaaaatgtcgtaacaactccgccccattgacgcaaatgggcggtaggcgtgtacggtgggaggtctatataagcagagctggtttagtgaaccgtcagatccgctagcctcgacttgagctcggatccacggtggaattcctgcagcccgggggatccgccaccatgggctacccatacgatgttcctgactatgctcaggccatcaagtgtgtggtggtgggagacggagctgttggtaaaacctgcctgctcatcagttacacgaccaatgcatttcctggagagtacatccccaccgtctttgacaactattctgccaatgttatggtagatggaaaaccagtgaatctgggcctatgggacacagctggactagaagattatgacagattgcgtcccctctcctacccgcagacagacgtgttcttaatttgcttttcccttgtgagtcctgcatcatttgaaaatgtccgtgcaaagtggtatcctgaagtgcgacaccactgtcccaatactcctatcatcctcgtggggacgaagcttgatcttagggatgataaggacaccattgagaagctgaaggagaagaagctgactcccatcacctacccgcaggggctggccatggcgaaagagatcggtgctgtcaaatacctggagtgctcagctctcacacagcgaggactcaagacagtgtttgacgaagctatccgagcggttctctgtccccctcctgtcaagaagaggaagagaaaatgcctgctgttgtaagcggccgctcgagtctagaactagtttgagtcgagccgcggcaattccgcccctctccctcccccccccctaacgttactggccgaagccgcttggaataaggccggtgtgcgtttgtctatatgttattttccaccatattgccgtcttttggcaatgtgagggcccggaaacctggccctgtcttcttgacgagcattcctaggggtctttcccctctcgccaaaggaatgcaaggtctgttgaatgtcgtgaaggaagcagttcctctggaagcttcttgaagacaaacaacgtctgtagcgaccctttgcaggcagcggaaccccccacctggcaacaggtgcctctgcggccaaaagccacgtgtataagatacacctgcaaaggcggcacaaccccagtgccacgttgtgagttggatagttgtggaaagagtcaaatggctctcctcaagcgtattcaacaaggggctgaaggatgcccagaaggtaccccattgtatgggatctgatctggggcctcggtgcacatgctttacatgtgtttagtcgaggttaaaaaaacgtctaggccccccgaaccacggggacgtggttttcctttgaaaaacacgatgataatatggtgagcaagggcgaggaggataacatggccatcatcaaggagttcatgcgcttcaaggtgcacatggagggctccgtgaacggccacgagttcgagatcgagggcgagggcgagggccgcccctacgagggcacccagaccgccaagctgaaggtgaccaagggtggccccctgcccttcgcctgggacatcctgtcccctcagttcatgtacggctccaaggcctacgtgaagcaccccgccgacatccccgactacttgaagctgtccttccccgagggcttcaagtgggagcgcgtgatgaacttcgaggacggcggcgtggtgaccgtgacccaggactcctccctgcaggacggcgagttcatctacaaggtgaagctgcgcggcaccaacttcccctccgacggccccgtaatgcagaagaagaccatgggctgggaggcctcctccgagcggatgtaccccgaggacggcgccctgaagggcgagatcaagcagaggctgaagctgaaggacggcggccactacgacgctgaggtcaagaccacctacaaggccaagaagcccgtgcagctgcccggcgcctacaacgtcaacatcaagttggacatcacctcccacaacgaggactacaccatcgtggaacagtacgaacgcgccgagggccgccactccaccggcggcatggacgagctgtacaagtaaccgcggtcgacggtaccgcgggcccgggatctaagcttatcgataatcaacctctggattacaaaatttgtgaaagattgactggtattcttaactatgttgctccttttacgctatgtggatacgctgctttaatgcctttgtatcatgctattgcttcccgtatggctttcattttctcctccttgtataaatcctggttgctgtctctttatgaggagttgtggcccgttgtcaggcaacgtggcgtggtgtgcactgtgtttgctgacgcaacccccactggttggggcattgccaccacctgtcagctcctttccgggactttcgctttccccctccctattgccacggcggaactcatcgccgcctgccttgcccgctgctggacaggggctcggctgttgggcactgacaattccgtggtgttgtcggggaaatcatcgtcctttccttggctgctcgcctgtgttgccacctggattctgcgcgggacgtccttctgctacgtcccttcggccctcaatccagcggaccttccttcccgcggcctgctgccggctctgcggcctcttccgcgtcttcgccttcgccctcagacgagtcggatctccctttgggccgcctccccgcatcgataccgtggatcgatccaccggatctagataactgatcataatcagccataccacatttgtagaggttttacttgctttaaaaaacctcccacacctccccctgaacctgaaacataaaatgaatgcaattgttgttgttaacttgtttattgcagcttataatggttacaaataaagcaatagcatcacaaatttcacaaataaagcatttttttcactgcattctagttgtggtttgtccaaactcatcaatgtatcttaacgcgtaaattgtaagcgttaatattttgttaaaattcgcgttaaatttttgttaaatcagctcattttttaaccaataggccgaaatcggcaaaatcccttataaatcaaaagaatagaccgagatagggttgagtgttgttccagtttggaacaagagtccactattaaagaacgtggactccaacgtcaaagggcgaaaaaccgtctatcagggcgatggcccactacgtgaaccatcaccctaatcaagttttttggggtcgaggtgccgtaaagcactaaatcggaaccctaaagggagcccccgatttagagcttgacggggaaagccggcgaacgtggcgagaaaggaagggaagaaagcgaaaggagcgggcgctagggcgctggcaagtgtagcggtcacgctgcgcgtaaccaccacacccgccgcgcttaatgcgccgctacagggcgcgtcaggtggcacttttcggggaaatgtgcgcggaacccctatttgtttatttttctaaatacattcaaatatgtatccgctcatgagacaataaccctgataaatgcttcaataatattgaaaaaggaagagtcctgaggcggaaagaaccagctgtggaatgtgtgtcagttagggtgtggaaagtccccaggctccccagcaggcagaagtatgcaaagcatgcatctcaattagtcagcaaccaggtgtggaaagtccccaggctccccagcaggcagaagtatgcaaagcatgcatctcaattagtcagcaaccatagtcccgcccctaactccgcccatcccgcccctaactccgcccagttccgcccattctccgccccatggctgactaattttttttatttatgcagaggccgaggccgcctcggcctctgagctattccagaagtagtgaggaggcttttttggaggcctaggcttttgcaaagatcgatcaagagacaggatgaggatcgtttcgcatgattgaacaagatggattgcacgcaggttctccggccgcttgggtggagaggctattcggctatgactgggcacaacagacaatcggctgctctgatgccgccgtgttccggctgtcagcgcaggggcgcccggttctttttgtcaagaccgacctgtccggtgccctgaatgaactgcaagacgaggcagcgcggctatcgtggctggccacgacgggcgttccttgcgcagctgtgctcgacgttgtcactgaagcgggaagggactggctgctattgggcgaagtgccggggcaggatctcctgtcatctcaccttgctcctgccgagaaagtatccatcatggctgatgcaatgcggcggctgcatacgcttgatccggctacctgcccattcgaccaccaagcgaaacatcgcatcgagcgagcacgtactcggatggaagccggtcttgtcgatcaggatgatctggacgaagagcatcaggggctcgcgccagccgaactgttcgccaggctcaaggcgagcatgcccgacggcgaggatctcgtcgtgacccatggcgatgcctgcttgccgaatatcatggtggaaaatggccgcttttctggattcatcgactgtggccggctgggtgtggcggaccgctatcaggacatagcgttggctacccgtgatattgctgaagagcttggcggcgaatgggctgaccgcttcctcgtgctttacggtatcgccgctcccgattcgcagcgcatcgccttctatcgccttcttgacgagttcttctgagcgggactctggggttcgaaatgaccgaccaagcgacgcccaacctgccatcacgagatttcgattccaccgccgccttctatgaaaggttgggcttcggaatcgttttccgggacgccggctggatgatcctccagcgcggggatctcatgctggagttcttcgcccaccctagggggaggctaactgaaacacggaaggagacaataccggaaggaacccgcgctatgacggcaataaaaagacagaataaaacgcacggtgttgggtcgtttgttcataaacgcggggttcggtcccagggctggcactctgtcgataccccaccgagaccccattggggccaatacgcccgcgtttcttccttttccccaccccaccccccaagttcgggtgaaggcccagggctcgcagccaacgtcggggcggcaggccctgccatagcctcaggttactcatatatactttagattgatttaaaacttcatttttaatttaaaaggatctaggtgaagatcctttttgataatctcatgaccaaaatcccttaacgtgagttttcgttccactgagcgtcagaccccgtagaaaagatcaaaggatcttcttgagatcctttttttctgcgcgtaatctgctgcttgcaaacaaaaaaaccaccgctaccagcggtggtttgtttgccggatcaagagctaccaactctttttccgaaggtaactggcttcagcagagcgcagataccaaatactgtccttctagtgtagccgtagttaggccaccacttcaagaactctgtagcaccgcctacatacctcgctctgctaatcctgttaccagtggctgctgccagtggcgataagtcgtgtcttaccgggttggactcaagacgatagttaccggataaggcgcagcggtcgggctgaacggggggttcgtgcacacagcccagcttggagcgaacgacctacaccgaactgagatacctacagcgtgagctatgagaaagcgccacgcttcccgaagggagaaaggcggacaggtatccggtaagcggcagggtcggaacaggagagcgcacgagggagcttccagggggaaacgcctggtatctttatagtcctgtcgggtttcgccacctctgacttgagcgtcgatttttgtgatgctcgtcaggggggcggagcctatggaaaaacgccagcaacgcggcctttttacggttcctggccttttgctggccttttgctcacatgttctttcctgcgttatcccctgattctgtggataaccgtattaccgccatgcat

SEQ ID NO: 53 - protein, 1500 aa, artificial
  GAP43-SSGSSGTG-meGFP-IRS1
MLCCMRRTKQVEKNDEDQNSSGSSGTGSKGEELFTGVVPILVELDGDVNGHKFSVSGEGEGDATYGKLTLKFICTTGKLPVPWPTLVTTLTYGVQCFSRYPDHMKRHDFFKSAMPEGYVQERTIFFKDDGNYKTRAEVKFEGDTLVNRIELKGIDFKEDGNILGHKLEYNYNSHNVYIMADKQKNGIKANFKIRHNIESGGVQLADHYQQNTPIGDGPVLLPDNHYLSTQSKLSKDPNEKRDHMVLKERVTAAGITHGMDELYKDIMCPPDTDGFSDVRKVGYLRKPKSMHKRFFVLRAASEAGGPARLEYYENEKKWRHKSSAPKRSIPLESCFNINKRADSKNKHLVALYTRDEHFAIAADSEAEQDSWYQALLQLHNRAKAHHDGAGGGCGGSCSGSSGVGEAGEDLSYDTGPGPAFKEVWQVILKPKGLGQTKNLIGIYRLCLTSKTISFVKLNSEAAAVVLQLMNIRRCGHSENFFFIEVGRSAVTGPGEFWMQVDDSVVAQNMHETILEAMRAMSDEFRPRTKSQSSSSCSNPISVPLRRHHLNNPPPSQVGLTRRSRTESITATSPASMVGGKPGSFRVRASSDGEGTMSRPASVDGSPVSPSTNRTHAHRHRGSSRLHPPLNHSRSIPMPSSRCSPSATSPVSLSSSSTSGHGSTSDCLFPRRSSASVSGSPSDGGFISSDEYGSSPCDFRSSFRSVTPDSLGHTPPARGEEELSNYICMGGKGASTLTAPNGHYILSRGGNGHRYIPGATMGTSPALTGDEAAGAADLDNRFRKRTHSAGTSPTISHQKTPSQSSVVSIEEYTEMMPAAYPPGGGSGGRLPGYRHSAFVPTHSYPEEGLEMHHLERRGGHHRPDSSNLHTDDGYMPMSPGVAPVPSNRKGNGDYMPMSPKSVSAPQQIINPIRRHPQRVDPNGYMMMSPSGSCSPDIGGGSCSSSSISAAPSGSSYGKPWTNGVGGHHTHALPHAKPPVESGGGKLLPCTGDYMNMSPVGDSNTSSPSECYYGPEDPQHKPVLSYYSLPRSFKHTQRPGEPEEGARHQHLRLSSSSGRLRYTATAEDSSSSTSSDSLGGGYCGARPESSVTHPHHHALQPHLPRKVDTAAQTNSRLARPTRLSLGDPKASTLPRVREQQQQQQQQQQSSLHPPEPKSPGEYVNIEFGSGQPGYLAGPATSRSSPSVRCLPQLHPAPREETGSEEYMNMDLGPGRRATWQESGGVELGRVGPAPPGAASICRPTRSVPNSRGDYMTMQIGCPRQSYVDTSPVAPVSYADMRTGIAAEKVSLPRTTGAAPPPSSTASASASVTPQGAAEQAAHSSLLGGPQGPGGMSAFTRVNLSPNHNQSAKVIRADTQGCRRRHSSETFSAPTRAANTVSFGAGAAGGGSGGGSEDVKRHSSASFENVWLRPGDLGGASKESAPGCGAAGGLEKSLNYIDLDLVKDVKQHPQDCPSQQQSLPPPPPHQPLGSNEGSSPRRSSEDLSTYASINFQKQPEDRQ

SEQ ID NO: 54 - DNA, 9892 bp, artificial
  GAP43-SSGSSGTG-meGFP-IRS1
gacggatcgggagatctcccgatcccctatggtgcactctcagtacaatctgctctgatgccgcatagttaagccagtatctgctccctgcttgtgtgttggaggtcgctgagtagtgcgcgagcaaaatttaagctacaacaaggcaaggcttgaccgacaattgcatgaagaatctgcttagggttaggcgttttgcgctgcttcgcgatgtacgggccagatatacgcgttgacattgattattgactagttattaatagtaatcaattacggggtcattagttcatagcccatatatggagttccgcgttacataacttacggtaaatggcccgcctggctgaccgcccaacgacccccgcccattgacgtcaataatgacgtatgttcccatagtaacgccaatagggactttccattgacgtcaatgggtggagtatttacggtaaactgcccacttggcagtacatcaagtgtatcatatgccaagtacgccccctattgacgtcaatgacggtaaatggcccgcctggcattatgcccagtacatgaccttatgggactttcctacttggcagtacatctacgtattagtcatcgctattaccatggtgatgcggttttggcagtacatcaatgggcgtggatagcggtttgactcacggggatttccaagtctccaccccattgacgtcaatgggagtttgttttggcaccaaaatcaacgggactttccaaaatgtcgtaacaactccgccccattgacgcaaatgggcggtaggcgtgtacggtgggaggtctatataagcagagctctctggctaactagagaacccactgcttactggcttatcgaaattaatacgactcactatagggagacccaagctggctagcgtttaaacttaagcttggtaccgacggaccatgctgtgctgtatgagaagaaccaaacaggttgaaaagaatgatgaggaccagaattcctccggatcgtctggaaccggttctaaaggagaagaacttttcactggagttgtcccaattcttgttgaattagatggtgatgttaatgggcacaaattttctgtcagtggagagggtgaaggtgatgcaacatacggaaaacttacccttaaatttatttgcactactggaaaactacctgttccttggccaacacttgtcactactttaacttatggtgttcaatgcttttcaagatacccagatcatatgaaacggcatgactttttcaagagtgccatgcccgaaggttatgtacaggaaagaactatatttttcaaagatgacgggaactacaagacacgtgctgaagtcaagtttgaaggtgatacccttgttaatagaatcgagttaaaaggtattgattttaaagaagatggaaacattcttggacacaaattggaatacaactataactcacacaatgtatacatcatggcagacaaacaaaagaatggaatcaaagctaacttcaaaattagacacaacattgagtccggaggcgttcaactagcagaccattatcaacaaaatactccaattggcgatggccctgtccttttaccagacaaccattacctgtccacacaatctaagctttcgaaagatcccaacgaaaagagagaccacatggtccttaaagagagggtaacagctgctgggattacacatggcatggacgagctgtacaaggatatcatgtgccctccggataccgatggcttctcagacgtgcgcaaggtgggttacctgcgcaaacccaagagtatgcataagcgctttttcgtgctgcgggcggccagcgaggccgggggcccggcgcgcctggagtattatgagaacgagaagaagtggcggcacaagtcgagcgcccccaaacgctcgatccccctcgagagctgtttcaacatcaacaagcgggctgactccaagaacaagcacctggtggctctctacacccgagacgaacactttgccattgcggcggatagcgaggctgaacaagacagctggtaccaggctcttctgcagctgcataatcgggcaaaggcccaccatgacggggctggaggaggctgcggtggtagctgcagcggcagctctggcgtcggagaggcaggggaggacttgagctatgacacgggcccaggacccgcgttcaaggaggtctggcaggttatcctgaaacccaagggcttaggtcagacaaagaacttgattggtatctaccgcctctgcctgaccagcaagaccatcagctttgtgaagctcaactctgaggctgccgctgtggtgctgcagctgatgaacatcagacgctgtggccactcagagaacttcttcttcatcgaggtggggcggtcagctgtgaccgggcccggcgagttctggatgcaagtggatgactccgtggtggcccagaacatgcatgagaccattctagaggccatgcgggccatgagcgatgagtttcgcccgcgcacgaaaagccaatcttcatccagttgctccaaccccatcagtgttcccctgcgcaggcaccatctcaacaatcctccgcccagccaagtggggctgactcggagatctcgaactgagagcatcactgccacctcccctgccagtatggtgggtgggaaaccaggttccttcagggtgcgtgcctccagcgatggcgaaggcaccatgtcccgtccagcatcagtggatggcagtcctgtgagccctagcaccaacaggacccacgcccatcggcatcgaggcagctccaggttgcaccccccactcaaccacagccgctccatccctatgccttcttcacgatgctccccttcagccaccagcccagtgagcctgtcatccagtagtaccagtggccacggctccacttcagactgtctcttcccgaggcgctctagtgcttccgtgtccggttctcctagcgatggcggtttcatctcttctgatgagtatggctctagtccctgcgatttccgaagttccttccgcagtgtcaccccagattccctgggccacaccccaccagccaggggtgaggaggagctgagcaactatatctgcatgggtggcaagggagcctccaccttgacagctcccaatggtcactacattttgtctaggggtggcaacggccatcgctacatcccaggtgctaccatggggacaagcccggcgctgactggagacgaagccgctggtgcagcagatctggataaccggtttcggaagagaactcactcggctggcacgtcccccaccatatcccaccagaagaccccctcgcagtcctcagtggtttctattgaggaatatacagagatgatgcccgctgcctacccaccaggaggtggcagtggaggccgactgcccggctaccggcattccgccttcgtgcccacccactcctatcccgaggagggtctagagatgcaccacttggaacgtcgtgggggccaccaccgtccagactcctccaacctccacaccgatgatggctacatgcccatgtctcccggagtggctccagtgcccagcaaccgcaaaggaaatggggactatatgcccatgagccccaagagtgtatctgccccccagcagatcattaaccccatcaggcgccacccacagagagtggaccccaatggctacatgatgatgtctcccagtggtagttgctctcctgacattggaggtgggtcttgcagcagtagcagcatcagcgcagccccttctgggagcagctatgggaagccatggacaaacggagtaggggggcaccatacccatgcccttccccatgccaaacctcctgttgagagcggtggtggtaagctcttgccttgcactggtgactacatgaacatgtcgccagtgggagattccaacaccagcagcccctcagaatgctactatggcccagaagatccccagcacaagcctgtcctctcctactactcattaccaaggtcctttaagcacacccagcgccctggggagccagaggagggtgccaggcaccagcatcttcgtctctcttcaagctctggacgccttcgctataccgcaactgccgaagattcctcctcttccaccagcagcgacagcctgggtgggggttactgtggggctaggccagagtctagcgtcacacatccccaccaccatgccttgcagccccatctgcctcgaaaggtagacacagctgcacagaccaacagccgcctggctcgacccacaaggctgtccttgggggatcccaaggcaagcactttaccccgggtacgagagcaacagcagcagcagcaacagcagcagcagtcttccctgcaccctcccgagcccaaaagcccaggagaatatgtgaatattgaattcgggagtggccagccaggctatttagctggccctgcaacttcccgtagctccccttcagttcgatgtctaccccagctccacccagctcccagagaagagactggctcggaagagtacatgaacatggacttggggccaggccggagggcaacctggcaggagagtggtggagttgagttgggcagagtaggccctgcacctccaggggctgcttccatttgtaggccaacccggtcggtgccaaatagccgtggtgattacatgaccatgcagataggttgtcctcgtcaaagctatgtggatacctcaccagtggccccagtcagctatgctgacatgcggacaggcattgctgcagagaaggtgagcctgcccagaaccacaggagctgccccccctccatcctccacagcctctgcttctgcttctgttacacctcaaggggccgctgagcaggccgctcactcttccttgctgggaggccctcagggacctgggggcatgagcgcattcaccagggtgaacctaagtcccaaccataaccagagtgccaaagtgattcgtgcagacactcaaggctgccggaggaggcacagctccgagaccttctcggcgcctacgcgggctgccaacacagtgtcttttggagcaggggctgcaggagggggcagcggtggtggcagtgaggatgtgaaacgccacagctctgcatcctttgagaatgtgtggctgagacccggggatctagggggagcatccaaggagtcggctccagggtgcggggctgccgggggattggagaagagtcttaactatatagacttggatttggtcaaggatgttaagcagcaccctcaagactgcccctctcaacagcagtccctgccaccccctccccctcaccaacccttaggcagcaatgagggcagctccccaagacgctccagtgaggatttaagcacctatgccagcatcaacttccagaagcaaccagaggaccgtcaatagaggtggcggccgctcgagtctagagggcccgtttaaacccgctgatcagcctcgactgtgccttctagttgccagccatctgttgtttgcccctcccccgtgccttccttgaccctggaaggtgccactcccactgtcctttcctaataaaatgaggaaattgcatcgcattgtctgagtaggtgtcattctattctggggggtggggtggggcaggacagcaagggggaggattgggaagacaatagcaggcatgctggggatgcggtgggctctatggcttctgaggcggaaagaaccagctggggctctagggggtatccccacgcgccctgtagcggcgcattaagcgcggcgggtgtggtggttacgcgcagcgtgaccgctacacttgccagcgccctagcgcccgctcctttcgctttcttcccttcctttctcgccacgttcgccggctttccccgtcaagctctaaatcgggggctccctttagggttccgatttagtgctttacggcacctcgaccccaaaaaacttgattagggtgatggttcacgtagtgggccatcgccctgatagacggtttttcgccctttgacgttggagtccacgttctttaatagtggactcttgttccaaactggaacaacactcaaccctatctcggtctattcttttgatttataagggattttgccgatttcggcctattggttaaaaaatgagctgatttaacaaaaatttaacgcgaattaattctgtggaatgtgtgtcagttagggtgtggaaagtccccaggctccccagcaggcagaagtatgcaaagcatgcatctcaattagtcagcaaccaggtgtggaaagtccccaggctccccagcaggcagaagtatgcaaagcatgcatctcaattagtcagcaaccatagtcccgcccctaactccgcccatcccgcccctaactccgcccagttccgcccattctccgccccatggctgactaattttttttatttatgcagaggccgaggccgcctctgcctctgagctattccagaagtagtgaggaggcttttttggaggcctaggcttttgcaaaaagctcccgggagcttgtatatccattttcggatctgatcaagagacaggatgaggatcgtttcgcatgattgaacaagatggattgcacgcaggttctccggccgcttgggtggagaggctattcggctatgactgggcacaacagacaatcggctgctctgatgccgccgtgttccggctgtcagcgcaggggcgcccggttctttttgtcaagaccgacctgtccggtgccctgaatgaactgcaggacgaggcagcgcggctatcgtggctggccacgacgggcgttccttgcgcagctgtgctcgacgttgtcactgaagcgggaagggactggctgctattgggcgaagtgccggggcaggatctcctgtcatctcaccttgctcctgccgagaaagtatccatcatggctgatgcaatgcggcggctgcatacgcttgatccggctacctgcccattcgaccaccaagcgaaacatcgcatcgagcgagcacgtactcggatggaagccggtcttgtcgatcaggatgatctggacgaagagcatcaggggctcgcgccagccgaactgttcgccaggctcaaggcgcgcatgcccgacggcgaggatctcgtcgtgacccatggcgatgcctgcttgccgaatatcatggtggaaaatggccgcttttctggattcatcgactgtggccggctgggtgtggcggaccgctatcaggacatagcgttggctacccgtgatattgctgaagagcttggcggcgaatgggctgaccgcttcctcgtgctttacggtatcgccgctcccgattcgcagcgcatcgccttctatcgccttcttgacgagttcttctgagcgggactctggggttcgaaatgaccgaccaagcgacgcccaacctgccatcacgagatttcgattccaccgccgccttctatgaaaggttgggcttcggaatcgttttccgggacgccggctggatgatcctccagcgcggggatctcatgctggagttcttcgcccaccccaacttgtttattgcagcttataatggttacaaataaagcaatagcatcacaaatttcacaaataaagcatttttttcactgcattctagttgtggtttgtccaaactcatcaatgtatcttatcatgtctgtataccgtcgacctctagctagagcttggcgtaatcatggtcatagctgtttcctgtgtgaaattgttatccgctcacaattccacacaacatacgagccggaagcataaagtgtaaagcctggggtgcctaatgagtgagctaactcacattaattgcgttgcgctcactgcccgctttccagtcgggaaacctgtcgtgccagctgcattaatgaatcggccaacgcgcggggagaggcggtttgcgtattgggcgctcttccgcttcctcgctcactgactcgctgcgctcggtcgttcggctgcggcgagcggtatcagctcactcaaaggcggtaatacggttatccacagaatcaggggataacgcaggaaagaacatgtgagcaaaaggccagcaaaaggccaggaaccgtaaaaaggccgcgttgctggcgtttttccataggctccgcccccctgacgagcatcacaaaaatcgacgctcaagtcagaggtggcgaaacccgacaggactataaagataccaggcgtttccccctggaagctccctcgtgcgctctcctgttccgaccctgccgcttaccggatacctgtccgcctttctcccttcgggaagcgtggcgctttctcatagctcacgctgtaggtatctcagttcggtgtaggtcgttcgctccaagctgggctgtgtgcacgaaccccccgttcagcccgaccgctgcgccttatccggtaactatcgtcttgagtccaacccggtaagacacgacttatcgccactggcagcagccactggtaacaggattagcagagcgaggtatgtaggcggtgctacagagttcttgaagtggtggcctaactacggctacactagaagaacagtatttggtatctgcgctctgctgaagccagttaccttcggaaaaagagttggtagctcttgatccggcaaacaaaccaccgctggtagcggtggtttttttgtttgcaagcagcagattacgcgcagaaaaaaaggatctcaagaagatcctttgatcttttctacggggtctgacgctcagtggaacgaaaactcacgttaagggattttggtcatgagattatcaaaaaggatcttcacctagatccttttaaattaaaaatgaagttttaaatcaatctaaagtatatatgagtaaacttggtctgacagttaccaatgcttaatcagtgaggcacctatctcagcgatctgtctatttcgttcatccatagttgcctgactccccgtcgtgtagataactacgatacgggagggcttaccatctggccccagtgctgcaatgataccgcgagacccacgctcaccggctccagatttatcagcaataaaccagccagccggaagggccgagcgcagaagtggtcctgcaactttatccgcctccatccagtctattaattgttgccgggaagctagagtaagtagttcgccagttaatagtttgcgcaacgttgttgccattgctacaggcatcgtggtgtcacgctcgtcgtttggtatggcttcattcagctccggttcccaacgatcaaggcgagttacatgatcccccatgttgtgcaaaaaagcggttagctccttcggtcctccgatcgttgtcagaagtaagttggccgcagtgttatcactcatggttatggcagcactgcataattctcttactgtcatgccatccgtaagatgcttttctgtgactggtgagtactcaaccaagtcattctgagaatagtgtatgcggcgaccgagttgctcttgcccggcgtcaatacgggataataccgcgccacatagcagaactttaaaagtgctcatcattggaaaacgttcttcggggcgaaaactctcaaggatcttaccgctgttgagatccagttcgatgtaacccactcgtgcacccaactgatcttcagcatcttttactttcaccagcgtttctgggtgagcaaaaacaggaaggcaaaatgccgcaaaaaagggaataagggcgacacggaaatgttgaatactcatactcttcctttttcaatattattgaagcatttatcagggttattgtctcatgagcggatacatatttgaatgtatttagaaaaataaacaaataggggttccgcgcacatttccccgaaaagtgccacctgacgtc

SEQ ID NO: 55 - protein, 1391 aa, artificial
  insulin receptor IR1-His6
MCCPGCCATGGRRGAAAAPLLVAVAALLLGAAGHLYPGEVCPGMDIRNNLTRLHELENCSVIEGHLQILLMFKTRPEDFRDLSFPKLIMITDYLLLFRVYGLESLKDLFPNLTVIRGSRLFFNYALVIFEMVHLKELGLYNLMNITRGSVRIEKNNELCYLATIDWSRILDSVEDNYIVLNKDDNEECGDICPGTAKGKTNCPATVINGQFVERCWTHSHCQKVCPTICKSHGCTAEGLCCHSECLGNCSQPDDPTKCVACRNFYLDGRCVETCPPPYYHFQDWRCVNFSFCQDLHHKCKNSRRQGCHQYVIHNNKCIPECPSGYTMNSSNLLCTPCLGPCPKVCHLLEGEKTIDSVTSAQELRGCTVINGSLIINIRGGNNLAAELEANLGLIEEISGYLKIRRSYALVSLSFFRKLRLIRGETLEIGNYSFYALDNQNLRQLWDWSKHNLTITQGKLFFHYNPKLCLSEIHKMEEVSGTKGRQERNDIALKTNGDQASCENELLKFSYIRTSFDKILLRWEPYWPPDFRDLLGFMLFYKEAPYQNVTEFDGQDACGSNSWTVVDIDPPLRSNDPKSQNHPGWLMRGLKPWTQYAIFVKTLVTFSDERRTYGAKSDIIYVQTDATNPSVPLDPISVSNSSSQIILKWKPPSDPNGNITHYLVFWERQAEDSELFELDYCLKGLKLPSRTWSPPFESEDSQKHNQSEYEDSAGECCSCPKTDSQILKELEESSFRKTFEDYLHNVVFVPRPSRKRRSLGDVGNVTVAVPTVAAFPNTSSTSVPTSPEEHRPFEKVVNKESLVISGLRHFTGYRIELQACNQDTPEERCSVAAYVSARTMPEAKADDIVGPVTHEIFENNVVHLMWQEPKEPNGLIVLYEVSYRRYGDEELHLCVSRKHFALERGCRLRGLSPGNYSVRIRATSLAGNGSWTEPTYFYVTDYLDVPSNIAKIIIGPLIFVFLFSVVIGSIYLFLRKRQPDGPLGPLYASSNPEYLSASDVFPCSVYVPDEWEVSREKITLLRELGQGSFGMVYEGNARDIIKGEAETRVAVKTVNESASLRERIEFLNEASVMKGFTCHHVVRLLGVVSKGQPTLVVMELMAHGDLKSYLRSLRPEAENNPGRPPPTLQEMIQMAAEIADGMAYLNAKKFVHRDLAARNCMVAHDFTVKIGDFGMTRDIYETDYYRKGGKGLLPVRWMAPESLKDGVFTTSSDMWSFGVVLWEITSLAEQPYQGLSNEQVLKFVMDGGYLDQPDNCPERVTDLMRMCWQFNPKMRPTFLEIVNLLKDDLHPSFPEVSFFHSEENKAPESEELEMEFEDMENVPLDRSSHCQREEAGGRDGGSSLGFKRSYEEHIPYTHMNGGKKNGRILTLPRSNPSGGGGSHHHHHHHHHH

SEQ ID NO: 56 - DNA, 10124 bp, artificial
  IR1
gacggatcgggagatctcccgatcccctatggtgcactctcagtacaatctgctctgatgccgcatagttaagccagtatctgctccctgcttgtgtgttggaggtcgctgagtagtgcgcgagcaaaatttaagctacaacaaggcaaggcttgaccgacaattgcatgaagaatctgcttagggttaggcgttttgcgctgcttcgcgagtacatttatattggctcatgtccaatatgaccgccatgttgacattgattattgactagttattaatagtaatcaattacggggtcattagttcatagcccatatatggagttccgcgttacataacttacggtaaatggcccgcctggctgaccgcccaacgacccccgcccattgacgtcaataatgacgtatgttcccatagtaacgccaatagggactttccattgacgtcaatgggtggagtatttacggtaaactgcccacttggcagtacatcaagtgtatcatatgccaagtccgccccctattgacgtcaatgacggtaaatggcccgcctggcattatgcccagtacatgaccttacgggactttcctacttggcagtacatctacgtattagtcatcgctattaccatggtgatgcggttttggcagtacaccaatgggcgtggatagcggtttgactcacggggatttccaagtctccaccccattgacgtcaatgggagtttgttttggcaccaaaatcaacgggactttccaaaatgtcgtaataaccccgccccgttgacgcaaatgggcggtaggcgtgtacggtgggaggtctatataagcagagctcgtttagtgaaccgtcagatcctcactctcttccgcatcgctgtctgcgagggccagctgttgggctcgcggttgaggacaaactcttcgcggtctttccagtactcttggatcggaaacccgtcggcctccgaacggtactccgccaccgagggacctgagcgagtccgcatcgaccggatcggaaaacctctcgagaaaggcgtctaaccagtcacagtcgcaaggtaggctgagcaccgtggcgggcggcagcgggtggcggtcggggttgtttctggcggaggtgctgctgatgatgtaattaaagtaggcggtcttgagacggcggatggtcgaggtgaggtgtggcaggcttgagatccagctgttggggtgagtactccctctcaaaagcgggcattacttctgcgctaagattgtcagtttccaaaaacgaggaggatttgatattcacctggcccgatctggccatacacttgagtgacaatgacatccactttgcctttctctccacaggtgtccactcccaggtccaagtttaaactttaatacgactcactataggggccgccaccaagcttggtaccatgtgctgtcccggctgttgcgccaccgggggccggcggggggcggcggccgcgccgctgctggtggcggtggccgcgctgctactgggcgccgcgggccacctgtaccccggagaggtgtgtcccggcatggatatccggaacaacctcactaggttgcatgagctggagaattgctctgtcatcgaaggacacttgcagatactcttgatgttcaaaacgaggcccgaagatttccgagacctcagtttccccaaactcatcatgatcactgattacttgctgctcttccgggtctatgggctcgagagcctgaaggacctgttccccaacctcacggtcatccggggatcacgactgttctttaactacgcgctggtcatcttcgagatggttcacctcaaggaactcggcctctacaacctgatgaacatcacccggggttctgtccgcatcgagaagaacaatgagctctgttacttggccactatcgactggtcccgtatcctggattccgtggaggataattacatcgtgttgaacaaagatgacaacgaggagtgtggagacatctgtccgggtaccgcgaagggcaagaccaactgccccgccaccgtcatcaacgggcagtttgtcgaacgatgttggactcatagtcactgccagaaagtttgcccgaccatctgtaagtcacacggctgcaccgccgaaggcctctgttgccacagcgagtgcctgggcaactgttctcagcccgacgaccccaccaagtgcgtggcctgccgcaacttctacctggacggcaggtgtgtggagacctgcccgcccccgtactaccacttccaggactggcgctgtgtgaacttcagcttctgccaggacctgcaccacaaatgcaagaactcgcggaggcagggctgccaccagtacgtcattcacaacaacaagtgcatccctgagtgtccctccgggtacacgatgaattccagcaacttgctgtgcaccccatgcctgggtccctgtcccaaggtgtgccacctcctagaaggcgagaagaccatcgactcggtgacgtctgcccaggagctccgaggatgcaccgtcatcaacgggagtctgatcatcaacattcgaggaggcaacaatctggcagctgagctagaagccaacctcggcctcattgaagaaatttcagggtatctaaaaatccgccgatcctacgctctggtgtcactttccttcttccggaagttacgtctgattcgaggagagaccttggaaattgggaactactccttctatgccttggacaaccagaacctaaggcagctctgggactggagcaaacacaacctcaccatcactcaggggaaactcttcttccactataaccccaaactctgcttgtcagaaatccacaagatggaagaagtttcaggaaccaaggggcgccaggagagaaacgacattgccctgaagaccaatggggaccaggcatcctgtgaaaatgagttacttaaattttcttacattcggacatcttttgacaagatcttgctgagatgggagccgtactggccccccgacttccgagacctcttggggttcatgctgttctacaaagaggccccttatcagaatgtgacggagttcgacgggcaggatgcatgtggttccaacagttggacggtggtagacattgacccacccctgaggtccaacgaccccaaatcacagaaccacccagggtggctgatgcggggtctcaagccctggacccagtatgccatctttgtgaagaccctggtcaccttttcggatgaacgccggacctatggggccaagagtgacatcatttatgtccagacagatgccaccaacccctctgtgcccctggatccaatctcagtgtctaactcatcatcccagattattctgaagtggaaaccaccctccgaccccaatggcaacatcacccactacctggttttctgggagaggcaggcggaagacagtgagctgttcgagctggattattgcctcaaagggctgaagctgccctcgaggacctggtctccaccattcgagtctgaagattctcagaagcacaaccagagtgagtatgaggattcggccggcgaatgctgctcctgtccaaagacagactctcagatcctgaaggagctggaggagtcctcgtttaggaagacgtttgaggattacctgcacaacgtggttttcgtccccaggccatctcggaaacgcaggtcccttggcgatgttgggaatgtgacggtggccgtgcccacggtggcagctttccccaacacttcctcgaccagcgtgcccacgagtccggaggagcacaggccttttgagaaggtggtgaacaaggagtcgctggtcatctccggcttgcgacacttcacgggctatcgcatcgagctgcaggcttgcaaccaggacacccctgaggaacggtgcagtgtggcagcctacgtcagtgcgaggaccatgcctgaagccaaggctgatgacattgttggccctgtgacgcatgaaatctttgagaacaacgtcgtccacttgatgtggcaggagccgaaggagcccaatggtctgatcgtgctgtatgaagtgagttatcggcgatatggtgatgaggagctgcatctctgcgtctcccgcaagcacttcgctctggaacggggctgcaggctgcgtgggctgtcaccggggaactacagcgtgcgaatccgggccacctcccttgcgggcaacggctcttggacggaacccacctatttctacgtgacagactatttagacgtcccgtcaaatattgcaaaaattatcatcggccccctcatctttgtctttctcttcagtgttgtgattggaagtatttatctattcctgagaaagaggcagccagatgggccgctgggaccgctttacgcttcttcaaaccctgagtatctcagtgccagtgatgtgtttccatgctctgtgtacgtgccggatgagtgggaggtgtctcgagagaagatcaccctccttcgagagctggggcagggctccttcggcatggtgtatgagggcaatgccagggacatcatcaagggtgaggcagagacccgcgtggcggtgaagacggtcaacgagtcagccagtctccgagagcggattgagttcctcaatgaggcctcggtcatgaagggcttcacctgccatcatgtggtgcgcctcctgggagtggtgtccaagggccagcccacgctggtggtgatggagctgatggctcacggagacctgaagagctacctccgttctctgcggccagaggctgagaataatcctggccgccctccccctacccttcaagagatgattcagatggcggcagagattgctgacgggatggcctacctgaacgccaagaagtttgtgcatcgggacctggcagcgagaaactgcatggtcgcccatgattttactgtcaaaattggagactttggaatgaccagagacatctatgaaacggattactaccggaaagggggcaagggtctgctccctgtacggtggatggcaccggagtccctgaaggatggggtcttcaccacttcttctgacatgtggtcctttggcgtggtcctttgggaaatcaccagcttggcagaacagccttaccaaggcctgtctaatgaacaggtgttgaaatttgtcatggatggagggtatctggatcaacccgacaactgtccagagagagtcactgacctcatgcgcatgtgctggcaattcaaccccaagatgaggccaaccttcctggagattgtcaacctgctcaaggacgacctgcaccccagctttccagaggtgtcgttcttccacagcgaggagaacaaggctcccgagagtgaggagctggagatggagtttgaggacatggagaatgtgcccctggaccgttcctcgcactgtcagagggaggaggcggggggccgggatggagggtcctcgctgggtttcaagcggagctacgaggaacacatcccttacacacacatgaacggaggcaagaaaaacgggcggattctgaccttgcctcggtccaatccttccgggggtggaggctctcaccatcaccaccatcatcaccaccatcactaaactcgagtctagagcggccgccgaattcgggcccgtttaaacccgctgatcagcctcgactgtgccttctagttgccagccatctgttgtttgcccctcccccgtgccttccttgaccctggaaggtgccactcccactgtcctttcctaataaaatgaggaaattgcatcgcattgtctgagtaggtgtcattctattctggggggtggggtggggcaggacagcaagggggaggattgggaagacaatagcaggcatgctggggatgcggtgggctctatggcttctgaggcggaaagaaccagctggggctctagggggtatccccacgcgccctgtagcggcgcattaagcgcggcgggtgtggtggttacgcgcagcgtgaccgctacacttgccagcgccctagcgcccgctcctttcgctttcttcccttcctttctcgccacgttcgcaggctttccccgtcaagctctaaatcgggggctccctttagggttccgatttagtgctttacggcacctcgaccccaaaaaacttgattagggtgatggttcacgtagtgggccatcgccctgatagacggtttttcgccctttgacgttggagtccacgttctttaatagtggactcttgttccaaactggaacaacactcaaccctatctcggtctattcttttgatttataagggattttgccgatttcggcctattggttaaaaaatgagctgatttaacaaaaatttaacgcgaattaattctgtggaatgtgtgtcagttagggtgtggaaagtccccaggctccccagcaggcagaagtatgcaaagcatgcatctcaattagtcagcaaccaggtgtggaaagtccccaggctccccagcaggcagaagtatgcaaagcatgcatctcaattagtcagcaaccatagtcccgcccctaactccgcccatcccgcccctaactccgcccagttccgcccattctccgccccatggctgactaattttttttatttatgcagaggccgaggccgcctctgcctctgagctattccagaagtagtgaggaggcttttttggaggcctaggcttttgcaaaaagctctcgggagcttgtatatccattttcggatctgatcagcacgtgatgaaaaagcctgaactcaccgcgacgtctgtcgagaagtttctgatcgaaaagttcgacagcgtctccgacctgatgcagctctcggagggcgaagaatctcgtgctttcagcttcgatgtaggagggcgtggatatgtcctgcgggtaaatagctgcgccgatggtttctacaaagatcgttatgtttatcggcactttgcatcggccgcgctcccgattccggaagtgcttgacattggggaattcagcgagagcctgacctattgcatctcccgccgtgcacagggtgtcacgttgcaagacctgcctgaaaccgaactgcccgctgttctgcagccggtcgcggaggccatggatgcgatcgctgcggccgatcttagccagacgagcgggttcggcccattcggaccgcaaggaatcggtcaatacactacatggcgtgatttcatatgcgcgattgctgatccccatgtgtatcactggcaaactgtgatggacgacaccgtcagtgcgtccgtcgcgcaggctctcgatgagctgatgctttgggccgaggactgccccgaagtccggcacctcgtgcacgcggatttcggctccaacaatgtcctgacggacaatggccgcataacagcggtcattgactggagcgaggcgatgttcggggattcccaatacgaggtcgccaacatcttcttctggaggccgtggttggcttgtatggagcagcagacgcgctacttcgagcggaggcatccggagcttgcaggatcgccgcggctccgggcgtatatgctccgcattggtcttgaccaactctatcagagcttggttgacggcaatttcgatgatgcagcttgggcgcagggtcgatgcgacgcaatcgtccgatccggagccgggactgtcgggcgtacacaaatcgcccgcagaagcgcggccgtctggaccgatggctgtgtagaagtactcgccgatagtggaaaccgacgccccagcactcgtccgagggcaaaggaatagcacgtgctacgagatttcgattccaccgccgccttctatgaaaggttgggcttcggaatcgttttccgggacgctggctggatgatcctccagcgcggggatctcatgctggagttcttcgcccaccccaacttgtttattgcagcttataatggttacaaataaagcaatagcatcacaaatttcacaaataaagcatttttttcactgcattctagttgtggtttgtccaaactcatcaatgtatcttatcatgtctgtataccgtcgacctctagctagagcttggcgtaatcatggtcatagctgtttcctgtgtgaaattgttatccgctcacaattccacacaacatacgagccggaagcataaagtgtaaagcctggggtgcctaatgagtgagctaactcacattaattgcgttgcgctcactgcccgctttccagtcgggaaacctgtcgtgccagctgcattaatgaatcggccaacgcgcggggagaggcggtttgcgtattgggcgctcttccgcttcctcgctcactgactcgctgcgctcggtcgttcggctgcggcgagcggtatcagctcactcaaaggcggtaatacggttatccacagaatcaggggataacgcaggaaagaacatgtgagcaaaaggccagcaaaaggccaggaaccgtaaaaaggccgcgttgctggcgtttttccataggctccgcccccctgacgagcatcacaaaaatcgacgctcaagtcagaggtggcgaaacccgacaggactataaagataccaggcgtttccccctggaagctccctcgtgcgctctcctgttccgaccctgccgcttaccggatacctgtccgcctttctcccttcgggaagcgtggcgctttctcatagctcacgctgtaggtatctcagttcggtgtaggtcgttcgctccaagctgggctgtgtgcacgaaccccccgttcagcccgaccgctgcgccttatccggtaactatcgtcttgagtccaacccggtaagacacgacttatcgccactggcagcagccactggtaacaggattagcagagcgaggtatgtaggcggtgctacagagttcttgaagtggtggcctaactacggctacactagaagaacagtatttggtatctgcgctctgctgaagccagttaccttcggaaaaagagttggtagctcttgatccggcaaacaaaccaccgctggtagcggtggtttttttgtttgcaagcagcagattacgcgcagaaaaaaaggatctcaagaagatcctttgatcttttctacggggtctgagcgcggaacccctatttgtttatttttctaaatacattcaaatatgtatccgctcatgaattaattcttagaaaaactcatcgagcatcaaatgaaactgcaatttattcatatcaggattatcaataccatatttttgaaaaagccgtttctgtaatgaaggagaaaactcaccgaggcagttccataggatggcaagatcctggtatcggtctgcgattccgactcgtccaacatcaatacaacctattaatttcccctcgtcaaaaataaggttatcaagtgagaaatcaccatgagtgacgactgaatccggtgagaatggcaaaagtttatgcatttctttccagacttgttcaacaggccagccattacgctcgtcatcaaaatcactcgcatcaaccaaaccgttattcattcgtgattgcgcctgagcgagacgaaatacgcgatcgctgttaaaaggacaattacaaacaggaatcgaatgcaaccggcgcaggaacactgccagcgcatcaacaatattttcacctgaatcaggatattcttctaatacctggaatgctgttttcccagggatcgcagtggtgagtaaccatgcatcatcaggagtacggataaaatgcttgatggtcggaagaggcataaattccgtcagccagtttagtctgaccatctcatctgtaacatcattggcaacgctacctttgccatgtttcagaaacaactctggcgcatcgggcttcccatacaatcgatagattgtcgcacctgattgcccgacattatcgcgagcccatttatacccatataaatcagcatccatgttggaatttaatcgcggcctagagcaagacgtttcccgttgaatatggctcataacaccccttgtattactgtttatgtaagcagacagttttattgttcatgaccaaaatcccttaacgtgagttttcgttccactgagcgtcagaccccgtagaaatccgcgcacatttccccgaaaagtgccacctgacgtc

SEQ ID NO: 57 - protein, 354 aa, artificial
  Galfa-i1
MGCTLSAEDKAAVERSKMIDRNLREDGEKAAREVKLLLLGAGESGKSTIVKQMKIIHEAGYSEEECKQYKAVVYSNTIQSIIAIIRAMGRLKIDFGDSARADDARQLFVLAGAAEEGFMTAELAGVIKRLWKDSGVQACFNRSREYQLNDSAAYYLNDLDRIAQPNYIPTQQDVLRTRVKTTGIVETHFTFKDLHFKMFDVGGQRSERKKWIHCFEGVTAIIFCVALSDYDLVLAEDEEMNRMHESMKLFDSICNNKWFTDTSIILFLNKKDLFEEKIKKSPLTICYPEYAGSNTYEEAAAYIQCQFEDLNKRKDTKEIYTHFTCATDTKNVQFVFDAVTDVIIKNNLKDCGLF

SEQ ID NO: 58 - DNA, 5771 bp, artificial
  Galfa-i1
tagttattaatagtaatcaattacggggtcattagttcatagcccatatatggagttccgcgttacataacttacggtaaatggcccgcctggctgaccgcccaacgacccccgcccattgacgtcaataatgacgtatgttcccatagtaacgccaatagggactttccattgacgtcaatgggtggagtatttacggtaaactgcccacttggcagtacatcaagtgtatcatatgccaagtacgccccctattgacgtcaatgacggtaaatggcccgcctggcattatgcccagtacatgaccttatgggactttcctacttggcagtacatctacgtattagtcatcgctattaccatggtgatgcggttttggcagtacatcaatgggcgtggatagcggtttgactcacggggatttccaagtctccaccccattgacgtcaatgggagtttgttttggcaccaaaatcaacgggactttccaaaatgtcgtaacaactccgccccattgacgcaaatgggcggtaggcgtgtacggtgggaggtctatataagcagagctggtttagtgaaccgtcagatccgctagcctcgacttgagctctctggctaactagagaacccactgcttactggcttatcgaaattaatacgactcactatagggagacccaagctggctagcgtttaaacttaagcttggtaccaccatgggctgcacgctgagcgccgaggacaaggcggcggtggagcggagtaagatgatcgaccgcaacctccgtgaggacggcgagaaggcggcgcgcgaggtcaagctgctgctgctcggtgctggtgaatctggtaaaagtacaattgtgaagcagatgaaaattatccatgaagctggttattcagaagaggagtgtaaacaatacaaagcagtggtctacagtaacaccatccagtcaattattgctatcattagggctatggggaggttgaagatagactttggtgactcagcccgggcggatgatgcacgccaactctttgtgctagctggagctgctgaagaaggctttatgactgcagaacttgctggagttataaagagattgtggaaagatagtggtgtacaagcctgtttcaacagatcccgagagtaccagcttaatgattctgcagcatactatttgaatgacttggacagaatagctcaaccaaattacatcccgactcaacaagatgttctcagaactagagtgaaaactacaggaattgttgaaacccattttactttcaaagatcttcattttaaaatgtttgatgtgggaggtcagagatctgagcggaagaagtggattcattgcttcgaaggagtgacggcgatcatcttctgtgtagcactgagtgactacgacctggttctagctgaagatgaagaaatgaaccgaatgcatgaaagcatgaaattgtttgacagcatatgtaacaacaagtggtttacagatacatccattatactttttctaaacaagaaggatctctttgaagaaaaaatcaaaaagagccctctcactatatgctatccagaatatgcaggatcaaacacatatgaagaggcagctgcatatattcaatgtcagtttgaagacctcaataaaagaaaggacacaaaggaaatatacacccacttcacatgtgccacagatactaagaatgtgcagtttgtttttgatgctgtaacagatgtcatcataaaaaataatctaaaagattgtggtctcttttaaccgcggtcgacggtaccgcgggcccgggatctaagcttatcgataatcaacctctggattacaaaatttgtgaaagattgactggtattcttaactatgttgctccttttacgctatgtggatacgctgctttaatgcctttgtatcatgctattgcttcccgtatggctttcattttctcctccttgtataaatcctggttgctgtctctttatgaggagttgtggcccgttgtcaggcaacgtggcgtggtgtgcactgtgtttgctgacgcaacccccactggttggggcattgccaccacctgtcagctcctttccgggactttcgctttccccctccctattgccacggcggaactcatcgccgcctgccttgcccgctgctggacaggggctcggctgttgggcactgacaattccgtggtgttgtcggggaaatcatcgtcctttccttggctgctcgcctgtgttgccacctggattctgcgcgggacgtccttctgctacgtcccttcggccctcaatccagcggaccttccttcccgcggcctgctgccggctctgcggcctcttccgcgtcttcgccttcgccctcagacgagtcggatctccctttgggccgcctccccgcatcgataccgtggatcgatccaccggatctagataactgatcataatcagccataccacatttgtagaggttttacttgctttaaaaaacctcccacacctccccctgaacctgaaacataaaatgaatgcaattgttgttgttaacttgtttattgcagcttataatggttacaaataaagcaatagcatcacaaatttcacaaataaagcatttttttcactgcattctagttgtggtttgtccaaactcatcaatgtatcttaacgcgtaaattgtaagcgttaatattttgttaaaattcgcgttaaatttttgttaaatcagctcattttttaaccaataggccgaaatcggcaaaatcccttataaatcaaaagaatagaccgagatagggttgagtgttgttccagtttggaacaagagtccactattaaagaacgtggactccaacgtcaaagggcgaaaaaccgtctatcagggcgatggcccactacgtgaaccatcaccctaatcaagttttttggggtcgaggtgccgtaaagcactaaatcggaaccctaaagggagcccccgatttagagcttgacggggaaagccggcgaacgtggcgagaaaggaagggaagaaagcgaaaggagcgggcgctagggcgctggcaagtgtagcggtcacgctgcgcgtaaccaccacacccgccgcgcttaatgcgccgctacagggcgcgtcaggtggcacttttcggggaaatgtgcgcggaacccctatttgtttatttttctaaatacattcaaatatgtatccgctcatgagacaataaccctgataaatgcttcaataatattgaaaaaggaagagtcctgaggcggaaagaaccagctgtggaatgtgtgtcagttagggtgtggaaagtccccaggctccccagcaggcagaagtatgcaaagcatgcatctcaattagtcagcaaccaggtgtggaaagtccccaggctccccagcaggcagaagtatgcaaagcatgcatctcaattagtcagcaaccatagtcccgcccctaactccgcccatcccgcccctaactccgcccagttccgcccattctccgccccatggctgactaattttttttatttatgcagaggccgaggccgcctcggcctctgagctattccagaagtagtgaggaggcttttttggaggcctaggcttttgcaaagatcgatcaagagacaggatgaggatcgtttcgcatgattgaacaagatggattgcacgcaggttctccggccgcttgggtggagaggctattcggctatgactgggcacaacagacaatcggctgctctgatgccgccgtgttccggctgtcagcgcaggggcgcccggttctttttgtcaagaccgacctgtccggtgccctgaatgaactgcaagacgaggcagcgcggctatcgtggctggccacgacgggcgttccttgcgcagctgtgctcgacgttgtcactgaagcgggaagggactggctgctattgggcgaagtgccggggcaggatctcctgtcatctcaccttgctcctgccgagaaagtatccatcatggctgatgcaatgcggcggctgcatacgcttgatccggctacctgcccattcgaccaccaagcgaaacatcgcatcgagcgagcacgtactcggatggaagccggtcttgtcgatcaggatgatctggacgaagagcatcaggggctcgcgccagccgaactgttcgccaggctcaaggcgagcatgcccgacggcgaggatctcgtcgtgacccatggcgatgcctgcttgccgaatatcatggtggaaaatggccgcttttctggattcatcgactgtggccggctgggtgtggcggaccgctatcaggacatagcgttggctacccgtgatattgctgaagagcttggcggcgaatgggctgaccgcttcctcgtgctttacggtatcgccgctcccgattcgcagcgcatcgccttctatcgccttcttgacgagttcttctgagcgggactctggggttcgaaatgaccgaccaagcgacgcccaacctgccatcacgagatttcgattccaccgccgccttctatgaaaggttgggcttcggaatcgttttccgggacgccggctggatgatcctccagcgcggggatctcatgctggagttcttcgcccaccctagggggaggctaactgaaacacggaaggagacaataccggaaggaacccgcgctatgacggcaataaaaagacagaataaaacgcacggtgttgggtcgtttgttcataaacgcggggttcggtcccagggctggcactctgtcgataccccaccgagaccccattggggccaatacgcccgcgtttcttccttttccccaccccaccccccaagttcgggtgaaggcccagggctcgcagccaacgtcggggcggcaggccctgccatagcctcaggttactcatatatactttagattgatttaaaacttcatttttaatttaaaaggatctaggtgaagatcctttttgataatctcatgaccaaaatcccttaacgtgagttttcgttccactgagcgtcagaccccgtagaaaagatcaaaggatcttcttgagatcctttttttctgcgcgtaatctgctgcttgcaaacaaaaaaaccaccgctaccagcggtggtttgtttgccggatcaagagctaccaactctttttccgaaggtaactggcttcagcagagcgcagataccaaatactgtccttctagtgtagccgtagttaggccaccacttcaagaactctgtagcaccgcctacatacctcgctctgctaatcctgttaccagtggctgctgccagtggcgataagtcgtgtcttaccgggttggactcaagacgatagttaccggataaggcgcagcggtcgggctgaacggggggttcgtgcacacagcccagcttggagcgaacgacctacaccgaactgagatacctacagcgtgagctatgagaaagcgccacgcttcccgaagggagaaaggcggacaggtatccggtaagcggcagggtcggaacaggagagcgcacgagggagcttccagggggaaacgcctggtatctttatagtcctgtcgggtttcgccacctctgacttgagcgtcgatttttgtgatgctcgtcaggggggcggagcctatggaaaaacgccagcaacgcggcctttttacggttcctggccttttgctggccttttgctcacatgttctttcctgcgttatcccctgattctgtggataaccgtattaccgccatgcat

SEQ ID NO: 59 - protein, 340 aa, artificial [sequence omitted]

SEQ ID NO: 60 - DNA, 6390 bp, artificial
  Gbeta1
gacggatcgggagatctcccgatcccctatggtgcactctcagtacaatctgctctgatgccgcatagttaagccagtatctgctccctgcttgtgtgttggaggtcgctgagtagtgcgcgagcaaaatttaagctacaacaaggcaaggcttgaccgacaattgcatgaagaatctgcttagggttaggcgttttgcgctgcttcgcgatgtacgggccagatatacgcgttgacattgattattgactagttattaatagtaatcaattacggggtcattagttcatagcccatatatggagttccgcgttacataacttacggtaaatggcccgcctggctgaccgcccaacgacccccgcccattgacgtcaataatgacgtatgttcccatagtaacgccaatagggactttccattgacgtcaatgggtggagtatttacggtaaactgcccacttggcagtacatcaagtgtatcatatgccaagtacgccccctattgacgtcaatgacggtaaatggcccgcctggcattatgcccagtacatgaccttatgggactttcctacttggcagtacatctacgtattagtcatcgctattaccatggtgatgcggttttggcagtacatcaatgggcgtggatagcggtttgactcacggggatttccaagtctccaccccattgacgtcaatgggagtttgttttggcaccaaaatcaacgggactttccaaaatgtcgtaacaactccgccccattgacgcaaatgggcggtaggcgtgtacggtgggaggtctatataagcagagctctctggctaactagagaacccactgcttactggcttatcgaaattaatacgactcactataggctagcgtttaaacttaagcttggtaccgagctcggatccaccatgagtgagcttgaccagttacggcaggaggccgagcaacttaagaaccagattcgagacgccaggaaagcatgtgcagatgcaactctctctcagatcacaaacaacatcgacccagtgggaagaatccaaatgcgcacgaggaggacactgcgggggcacctggccaagatctacgccatgcactggggcacagactccaggcttctcgtcagtgcctcgcaggatggtaaacttatcatctgggacagctacaccaccaacaaggtccacgccatccctctgcgctcctcctgggtcatgacctgtgcatatgccccttctgggaactatgtggcctgcggtggcctggataacatttgctccatttacaatctgaaaactcgtgaggggaacgtgcgcgtgagtcgtgagctggcaggacacacaggttacctgtcctgctgccgattcctggatgacaatcagatcgtcaccagctctggagacaccacgtgtgccctgtgggacatcgagaccggccagcagacgaccacgtttaccggacacactggagatgtcatgagcctttctcttgctcctgacaccagactgttcgtctctggtgcttgtgatgcttcagccaaactctgggatgtgcgagaaggcatgtgccggcagaccttcactggccacgagtctgacatcaatgccatttgcttctttccaaatggcaatgcatttgccactggctcagacgacgccacctgcaggctgtttgaccttcgtgctgaccaggagctcatgacttactcccatgacaacatcatctgcgggatcacctctgtctccttctccaagagcgggcgcctcctccttgctgggtacgacgacttcaactgcaacgtctgggatgcactcaaagccgaccgggcaggtgtcttggctgggcatgacaaccgcgtcagctgcctgggcgtgactgacgatggcatggctgtggcgacagggtcctgggatagcttcctcaagatctggaactaactcgagtctagagggcccgtttaaacccgctgatcagcctcgactgtgccttctagttgccagccatctgttgtttgcccctcccccgtgccttccttgaccctggaaggtgccactcccactgtcctttcctaataaaatgaggaaattgcatcgcattgtctgagtaggtgtcattctattctggggggtggggtggggcaggacagcaagggggaggattgggaagacaatagcaggcatgctggggatgcggtgggctctatggcttctgaggcggaaagaaccagctggggctctagggggtatccccacgcgccctgtagcggcgcattaagcgcggcgggtgtggtggttacgcgcagcgtgaccgctacacttgccagcgccctagcgcccgctcctttcgctttcttcccttcctttctcgccacgttcgccggctttccccgtcaagctctaaatcgggggctccctttagggttccgatttagtgctttacggcacctcgaccccaaaaaacttgattagggtgatggttcacgtagtgggccatcgccctgatagacggtttttcgccctttgacgttggagtccacgttctttaatagtggactcttgttccaaactggaacaacactcaaccctatctcggtctattcttttgatttataagggattttgccgatttcggcctattggttaaaaaatgagctgatttaacaaaaatttaacgcgaattaattctgtggaatgtgtgtcagttagggtgtggaaagtccccaggctccccagcaggcagaagtatgcaaagcatgcatctcaattagtcagcaaccaggtgtggaaagtccccaggctccccagcaggcagaagtatgcaaagcatgcatctcaattagtcagcaaccatagtcccgcccctaactccgcccatcccgcccctaactccgcccagttccgcccattctccgccccatggctgactaattttttttatttatgcagaggccgaggccgcctctgcctctgagctattccagaagtagtgaggaggcttttttggaggcctaggcttttgcaaaaagctcccgggagcttgtatatccattttcggatctgatcaagagacaggatgaggatcgtttcgcatgattgaacaagatggattgcacgcaggttctccggccgcttgggtggagaggctattcggctatgactgggcacaacagacaatcggctgctctgatgccgccgtgttccggctgtcagcgcaggggcgcccggttctttttgtcaagaccgacctgtccggtgccctgaatgaactgcaggacgaggcagcgcggctatcgtggctggccacgacgggcgttccttgcgcagctgtgctcgacgttgtcactgaagcgggaagggactggctgctattgggcgaagtgccggggcaggatctcctgtcatctcaccttgctcctgccgagaaagtatccatcatggctgatgcaatgcggcggctgcatacgcttgatccggctacctgcccattcgaccaccaagcgaaacatcgcatcgagcgagcacgtactcggatggaagccggtcttgtcgatcaggatgatctggacgaagagcatcaggggctcgcgccagccgaactgttcgccaggctcaaggcgcgcatgcccgacggcgaggatctcgtcgtgacccatggcgatgcctgcttgccgaatatcatggtggaaaatggccgcttttctggattcatcgactgtggccggctgggtgtggcggaccgctatcaggacatagcgttggctacccgtgatattgctgaagagcttggcggcgaatgggctgaccgcttcctcgtgctttacggtatcgccgctcccgattcgcagcgcatcgccttctatcgccttcttgacgagttcttctgagcgggactctggggttcgaaatgaccgaccaagcgacgcccaacctgccatcacgagatttcgattccaccgccgccttctatgaaaggttgggcttcggaatcgttttccgggacgccggctggatgatcctccagcgcggggatctcatgctggagttcttcgcccaccccaacttgtttattgcagcttataatggttacaaataaagcaatagcatcacaaatttcacaaataaagcatttttttcactgcattctagttgtggtttgtccaaactcatcaatgtatcttatcatgtctgtataccgtcgacctctagctagagcttggcgtaatcatggtcatagctgtttcctgtgtgaaattgttatccgctcacaattccacacaacatacgagccggaagcataaagtgtaaagcctggggtgcctaatgagtgagctaactcacattaattgcgttgcgctcactgcccgctttccagtcgggaaacctgtcgtgccagctgcattaatgaatcggccaacgcgcggggagaggcggtttgcgtattgggcgctcttccgcttcctcgctcactgactcgctgcgctcggtcgttcggctgcggcgagcggtatcagctcactcaaaggcggtaatacggttatccacagaatcaggggataacgcaggaaagaacatgtgagcaaaaggccagcaaaaggccaggaaccgtaaaaaggccgcgttgctggcgtttttccataggctccgcccccctgacgagcatcacaaaaatcgacgctcaagtcagaggtggcgaaacccgacaggactataaagataccaggcgtttccccctggaagctccctcgtgcgctctcctgttccgaccctgccgcttaccggatacctgtccgcctttctcccttcgggaagcgtggcgctttctcatagctcacgctgtaggtatctcagttcggtgtaggtcgttcgctccaagctgggctgtgtgcacgaaccccccgttcagcccgaccgctgcgccttatccggtaactatcgtcttgagtccaacccggtaagacacgacttatcgccactggcagcagccactggtaacaggattagcagagcgaggtatgtaggcggtgctacagagttcttgaagtggtggcctaactacggctacactagaagaacagtatttggtatctgcgctctgctgaagccagttaccttcggaaaaagagttggtagctcttgatccggcaaacaaaccaccgctggtagcggtttttttgtttgcaagcagcagattacgcgcagaaaaaaaggatctcaagaagatcctttgatcttttctacggggtctgacgctcagtggaacgaaaactcacgttaagggattttggtcatgagattatcaaaaaggatcttcacctagatccttttaaattaaaaatgaagttttaaatcaatctaaagtatatatgagtaaacttggtctgacagttaccaatgcttaatcagtgaggcacctatctcagcgatctgtctatttcgttcatccatagttgcctgactccccgtcgtgtagataactacgatacgggagggcttaccatctggccccagtgctgcaatgataccgcgagacccacgctcaccggctccagatttatcagcaataaaccagccagccggaagggccgagcgcagaagtggtcctgcaactttatccgcctccatccagtctattaattgttgccgggaagctagagtaagtagttcgccagttaatagtttgcgcaacgttgttgccattgctacaggcatcgtggtgtcacgctcgtcgtttggtatggcttcattcagctccggttcccaacgatcaaggcgagttacatgatcccccatgttgtgcaaaaaagcggttagctccttcggtcctccgatcgttgtcagaagtaagttggccgcagtgttatcactcatggttatggcagcactgcataattctcttactgtcatgccatccgtaagatgcttttctgtgactggtgagtactcaaccaagtcattctgagaatagtgtatgcggcgaccgagttgctcttgcccggcgtcaatacgggataataccgcgccacatagcagaactttaaaagtgctcatcattggaaaacgttcttcggggcgaaaactctcaaggatcttaccgctgttgagatccagttcgatgtaacccactcgtgcacccaactgatcttcagcatcttttactttcaccagcgtttctgggtgagcaaaaacaggaaggcaaaatgccgcaaaaaagggaataagggcgacacggaaatgttgaatactcatactcttcctttttcaatattattgaagcatttatcagggttattgtctcatgagcggatacatatttgaatgtatttagaaaaataaacaaataggggttccgcgcacatttccccgaaaagtgccacctgacgtc

SEQ ID NO: 61 - protein, 71 aa, artificial
  Ggamma2
MASNNTASIAQARKLVEQLKMEANIDRIKVSKAAADLMAYCEAHAKEDPLLTPVPASENPFREKKFFCAIL

SEQ ID NO: 62 - DNA, 6340 bp, artificial
  Ggamma2
gacggatcgggagatctcccgatcccctatggtgcactctcagtacaatctgctctgatgccgcatagttaagccagtatctgctccctgcttgtgtgttggaggtcgctgagtagtgcgcgagcaaaatttaagctacaacaaggcaaggcttgaccgacaattgcatgaagaatctgcttagggttaggcgttttgcgctgcttcgcgatgtacgggccagatatacgcgttgacattgattattgactagttattaatagtaatcaattacggggtcattagttcatagcccatatatggagttccgcgttacataacttacggtaaatggcccgcctggctgaccgcccaacgacccccgcccattgacgtcaataatgacgtatgttcccatagtaacgccaatagggactttccattgacgtcaatgggtggagtatttacggtaaactgcccacttggcagtacatcaagtgtatcatatgccaagtacgccccctattgacgtcaatgacggtaaatggcccgcctggcattatgcccagtacatgaccttatgggactttcctacttggcagtacatctacgtattagtcatcgctattaccatggtgatgcggttttggcagtacatcaatgggcgtggatagcggtttgactcacggggatttccaagtctccaccccattgacgtcaatgggagtttgttttggcaccaaaatcaacgggactttccaaaatgtcgtaacaactccgccccattgacgcaaatgggcggtaggcgtgtacggtgggaggtctatataagcagagctcgtttagtgaccgtcagatcactagaagctttattgcggtagtttatcacagttaaattgctaacgcagtcagtgcttctgacacaacagtctcgaacttaagctgcagaagttggtcgtgaggcactgggcaggtaagtatcaaggttacaagacaggtttaaggagaccaatagaaactgggcttgtcgagacagagaagactcttgcgtttctgataggcacctattggtcttactgacatccactttgcctttctctccacaggtgtccactcccagttcaattacagctcttaaggctagagtacttaatacgactcactataggctagcctcgaggtcgacggtatcgataagcttgatatcgaattccgggagtgcaggcgagctccggcgcagcccgcccagcccagccccgggagccaagccagatctgccagtgagcctcaggctttgggaattgaagagtgtatctgaaacctacccagcattccaatggccagcaacaacaccgccagcatagcacaagccaggaaactggtagaacagctgaagatggaagccaacatcgataggataaaggtgtccaaggcagctgcagatttgatggcctactgtgaagcgcatgccaaggaagatcccctcctgacacctgttccggcttcagaaaacccatttagggagaagaagtttttctgtgctatcctttaagtcttcaggaggaacctgaggagcctcggggctccagggacactgatgtagagtttttagcaaagtgggcgcctttctagtccacagcatttaaagagagggaggagaaccatcctggagtctccaggcttatgcatgtttaaagaacccggaattcctgcagcccgggggatccactagttctagagcggccgcttcgagcagacatgataagatacattggatgagtttggacaaaccacaactagaatgcagtgaaaaaaatgctttatttgtgaaatttgtgatgctattgctttatttgtaaccattataagctgcaataaacaagttaacaacaacaattgcattcttttatgtttcaggtcgagtctagagggcccgtttaaacccgctgatcagcctcgactgtgccttctagttgccagccatctgttgtttgcccctcccccgtgccttccttgaccctggaaggtgccactcccactgtcctttcctaataaaatgaggaaattgcatcgcattgtctgagtaggtgtcattctattctggggggtggggtggggcaggacagcaagggggaggattgggaagacaatagcaggcatgctggggatgcggtgggctctatggcttctgaggcggaaagaaccagctggggctctagggggtatccccacgcgccctgtagcggcgcattaagcgcggcgggtgtggtggttacgcgcagcgtgaccgctacacttgccagcgccctagcgcccgctcctttcgctttcttcccttcctttctcgccacgttcgccggctttccccgtcaagctctaaatcgggggctccctttagggttccgatttagtgctttacggcacctcgaccccaaaaaacttgattagggtgatggttcacgtagtgggccatcgccctgatagacggtttttcgccctttgacgttggagtccacgttctttaatagtggactcttgttccaaactggaacaacactcaaccctatctcggtctattcttttgatttataagggattttgccgatttcggcctattggttaaaaaatgagctgatttaacaaaaatttaacgcgaattaattctgtggaatgtgtgtcagttagggtgtggaaagtccccaggctccccagcaggcagaagtatgcaaagcatgcatctcaattagtcagcaaccaggtgtggaaagtccccaggctccccagcaggcagaagtatgcaaagcatgcatctcaattagtcagcaaccatagtcccgcccctaactccgcccatcccgcccctaactccgcccagttccgcccattctccgccccatggctgactaattttttttatttatgcagaggccgaggccgcctctgcctctgagctattccagaagtagtgaggaggcttttttggaggcctaggcttttgcaaaaagctcccgggagcttgtatatccattttcggatctgatcaagagacaggatgaggatcgtttcgcatgattgaacaagatggattgcacgcaggttctccggccgcttgggtggagaggctattcggctatgactgggcacaacagacaatcggctgctctgatgccgccgtgttccggctgtcagcgcaggggcgcccggttctttttgtcaagaccgacctgtccggtgccctgaatgaactgcaggacgaggcagcgcggctatcgtggctggccacgacgggcgttccttgcgcagctgtgctcgacgttgtcactgaagcgggaagggactggctgctattgggcgaagtgccggggcaggatctcctgtcatctcaccttgctcctgccgagaaagtatccatcatggctgatgcaatgcggcggctgcatacgcttgatccggctacctgcccattcgaccaccaagcgaaacatcgcatcgagcgagcacgtactcggatggaagccggtcttgtcgatcaggatgatctggacgaagagcatcaggggctcgcgccagccgaactgttcgccaggctcaaggcgcgcatgcccgacggcgaggatctcgtcgtgacccatggcgatgcctgcttgccgaatatcatggtggaaaatggccgcttttctggattcatcgactgtggccggctgggtgtggcggaccgctatcaggacatagcgttggctacccgtgatattgctgaagagcttggcggcgaatgggctgaccgcttcctcgtgctttacggtatcgccgctcccgattcgcagcgcatcgccttctatcgccttcttgacgagttcttctgagcgggactctggggttcgaaatgaccgaccaagcgacgcccaacctgccatcacgagatttcgattccaccgccgccttctatgaaaggttgggcttcggaatcgttttccgggacgccggctggatgatcctccagcgcggggatctcatgctggagttcttcgcccaccccaacttgtttattgcagcttataatggttacaaataaagcaatagcatcacaaatttcacaaataaagcatttttttcactgcattctagttgtggtttgtccaaactcatcaatgtatcttatcatgtctgtataccgtcgacctctagctagagcttggcgtaatcatggtcatagctgtttcctgtgtgaaattgttatccgctcacaattccacacaacatacgagccggaagcataaagtgtaaagcctggggtgcctaatgagtgagctaactcacattaattgcgttgcgctcactgcccgctttccagtcgggaaacctgtcgtgccagctgcattaatgaatcggccaacgcgcggggagaggcggtttgcgtattgggcgctcttccgcttcctcgctcactgactcgctgcgctcggtcgttcggctgcggcgagcggtatcagctcactcaaaggcggtaatacggttatccacagaatcaggggataacgcaggaaagaacatgtgagcaaaaggccagcaaaaggccaggaaccgtaaaaaggccgcgttgctggcgtttttccataggctccgcccccctgacgagcatcacaaaaatcgacgctcaagtcagaggtggcgaaacccgacaggactataaagataccaggcgtttccccctggaagctccctcgtgcgctctcctgttccgaccctgccgcttaccggatacctgtccgcctttctcccttcgggaagcgtggcgctttctcatagctcacgctgtaggtatctcagttcggtgtaggtcgttcgctccaagctgggctgtgtgcacgaaccccccgttcagcccgaccgctgcgccttatccggtaactatcgtcttgagtccaacccggtaagacacgacttatcgccactggcagcagccactggtaacaggattagcagagcgaggtatgtaggcggtgctacagagttcttgaagtggtggcctaactacggctacactagaagaacagtatttggtatctgcgctctgctgaagccagttaccttcggaaaaagagttggtagctcttgatccggcaaacaaaccaccgctggtagcggtttttttgtttgcaagcagcagattacgcgcagaaaaaaaggatctcaagaagatcctttgatcttttctacggggtctgacgctcagtggaacgaaaactcacgttaagggattttggtcatgagattatcaaaaaggatcttcacctagatccttttaaattaaaaatgaagttttaaatcaatctaaagtatatatgagtaaacttggtctgacagttaccaatgcttaatcagtgaggcacctatctcagcgatctgtctatttcgttcatccatagttgcctgactccccgtcgtgtagataactacgatacgggagggcttaccatctggccccagtgctgcaatgataccgcgagacccacgctcaccggctccagatttatcagcaataaaccagccagccggaagggccgagcgcagaagtggtcctgcaactttatccgcctccatccagtctattaattgttgccgggaagctagagtaagtagttcgccagttaatagtttgcgcaacgttgttgccattgctacaggcatcgtggtgtcacgctcgtcgtttggtatggcttcattcagctccggttcccaacgatcaaggcgagttacatgatcccccatgttgtgcaaaaaagcggttagctccttcggtcctccgatcgttgtcagaagtaagttggccgcagtgttatcactcatggttatggcagcactgcataattctcttactgtcatgccatccgtaagatgcttttctgtgactggtgagtactcaaccaagtcattctgagaatagtgtatgcggcgaccgagttgctcttgcccggcgtcaatacgggataataccgcgccacatagcagaactttaaaagtgctcatcattggaaaacgttcttcggggcgaaaactctcaaggatcttaccgctgttgagatccagttcgatgtaacccactcgtgcacccaactgatcttcagcatcttttactttcaccagcgtttctgggtgagcaaaaacaggaaggcaaaatgccgcaaaaaagggaataagggcgacacggaaatgttgaatactcatactcttcctttttcaatattattgaagcatttatcagggttattgtctcatgagcggatacatatttgaatgtatttagaaaaataaacaaataggggttccgcgcacatttccccgaaaagtgccacctgacgtc

SEQ ID NO: 63 - protein, 449 aa, artificial
  alfa2-adrenergic receptor
MGSLQPDAGNSSWNGTEAPGGGTRATPYSLQVTLTLVCLAGLLMLFTVFGNVLVIIAVFTSRALKAPQNLFLVSLASADILVATLVIPFSLANEVMGYWYFGKVWCEIYLALDVLFCTSSIVHLCAISLDRYWSITQAIYNLKRTPRRIKAIIITVWVISAVISFPPLISIEKKGGGGGPQPAEPRCEINDQKWYVISSCIGSFFAPCLIMILVYVRIYQIAKRRTRVPPSRRGPDAVAAPPGGTERRPNGLGPERSAGPGGAEAEPLPTQLNGAPGEPAPAGPRDTDALDLEESSSSDHAERPPGPRRPERGPRGKGKARASQVKPGDSLPRRGPGATGIGTPAAGPGEERVGAAKASRWRGRQNREKRFTFVLAVVIGVFVVCWFPFFFTYTLTAVGCSVPRTLFKFFFWFGYCNSSLNPVIYTIFNHDFRRAFKKILCRGDRKRIV

SEQ ID NO: 64 - DNA, 6980 bp, artificial
  alfa2-adrenergic receptor
gacggatcgggagatctcccgatcccctatggtcgactctcagtacaatctgctctgatgccgcatagttaagccagtatctgctccctgcttgtgtgttggaggtcgctgagtagtgcgcgagcaaaatttaagctacaacaaggcaaggcttgaccgacaattgcatgaagaatctgcttagggttaggcgttttgcgctgcttcgcgatgtacgggccagatatacgcgttgacattgattattgactagttattaatagtaatcaattacggggtcattagttcatagcccatatatggagttccgcgttacataacttacggtaaatggcccgcctggctgaccgcccaacgacccccgcccattgacgtcaataatgacgtatgttcccatagtaacgccaatagggactttccattgacgtcaatgggtggactatttacggtaaactgcccacttggcagtacatcaagtgtatcatatgccaagtacgccccctattgacgtcaatgacggtaaatggcccgcctggcattatgcccagtacatgaccttatgggactttcctacttggcagtacatctacgtattagtcatcgctattaccatggtgatgcggttttggcagtacatcaatgggcgtggatagcggtttgactcacggggatttccaagtctccaccccattgacgtcaatgggagtttgttttggcaccaaaatcaacgggactttccaaaatgtcgtaacaactccgccccattgacgcaaatgggcggtaggcgtgtacggtgggaggtctatataagcagagctctctggctaactagagaacccactgcttactggcttatcgaaattaatacgactcactatagggagacccaagcttccatgggctacccatacgacgtcccagactacgccagcatgggctcactgcagccggatgccggcaacagcagctggaacgggaccgaagcgcccggaggcggcacccgagccaccccttactccctgcaggtgacactgacgctggtttgcctggctggcctgctcatgctgttcacagtatttggcaacgtgctggttattatcgcggtgttcaccagtcgcgcgctcaaagctccccaaaacctcttcctggtgtccctggcctcagcggacatcctggtggccacgctggtcattcccttttctttggccaacgaggttatgggttactggtactttggtaaggtgtggtgtgagatctatttggctctcgacgtgctcttttgcacgtcgtccatagtgcacctgtgcgccatcagccttgaccgctactggtccatcacgcaggccatcgagtacaacctgaagcgcacgccgcgccgcatcaaggccatcatcatcaccgtgtgggtcatctcggccgtcatctccttcccgccgctcatctccatcgagaagaagggcggcggcggcggcccgcagccggccgagccgcgctgcgagatcaacgaccagaagtggtacgtcatctcgtcgtgcatcggctccttcttcgctccctgcctcatcatgatcctggtctacgtgcgcatctaccagatcgccaagcgtcgcacccgcgtgccacccagccgccggggtccggacgccgtcgccgcgccgccggggggcaccgagcgcaggcccaacggtctgggccccgagcgcagcgcgggcccggggggcgcagaggccgaaccgctgcccacccagctcaacggcgcccctggcgagcccgcgccggccgggccgcgcgacaccgacgcgctggacctggaggagagctcgtcttccgaccacgccgagcggcctccagggccccgcagacccgagcgcggtccccggggcaaaggcaaggcccgagcgagccaggtgaagccgggcgacagcctgccgcggcgcgggccgggggcgacggggatcgggacgccggctgcagggccgggggaggagcgcgtcggggctgccaaggcgtcgcgctggcgcgggcggcagaaccgcgagaagcgcttcacgttcgtgctggccgtggtcatcggagtgttcgtggtgtgctggttccccttcttcttcacctacacgctcacggccgtcgggtgctccgtgccacgcacgctcttcaaattcttcttctggttcggctactgcaacagctcgttgaacccggtcatctacaccatcttcaaccacgatttccgccgcgccttcaagaagatcctctgtcggggggacaggaagcggatcgtgtgacgcatgggccttgccctgcgtgcagacaatggtcagacgcaggccctgggcttcgagggggtgcgtctacgcatgcagcccctagcactctgaaaccccggacctacccagctgggagggagctccaccgcggtggcggccgctctagaactagtggatccactagtaacggccgccagtgtgctggaattctgcagatatccatcacactggcggccgctcgagcatgcatctagagggccctattctatagtgtcacctaaatgctagagctcgctgatcagcctcgactgtgccttctagttgccagccatctgttgtttgcccctcccccgtgccttccttgaccctggaaggtgccactcccactgtcctttcctaataaaatgaggaaattgcatcgcattgtctgagtaggtgtcattctattctggggggtggggtggggcaggacagcaagggggaggattgggaagacaatagcaggcatgctggggatgcggtgggctctatggcttctgaggcggaaagaaccagctggggctctagggggtatccccacgcgccctgtagcggcgcattaagcgcggcgggtgtggtggttacgcgcagcgtgaccgctacacttgccagcgccctagcgcccgctcctttcgctttcttcccttcctttctcgccacgttcgccggctttccccgtcaagctctaaatcggggcatccctttagggttccgatttagtgctttacggcacctcgaccccaaaaaacttgattagggtgatggttcacgtagtgggccatcgccctgatagacggtttttcgccctttgacgttggagtccacgttctttaatagtggactcttgttccaaactggaacaacactcaaccctatctcggtctattcttttgatttataagggattttggggatttcggcctattggttaaaaaatgagctgatttaacaaaaatttaacgcgaattaattctgtggaatgtgtgtcagttagggtgtggaaagtccccaggctccccaggcaggcagaagtatgcaaagcatgcatctcaattagtcagcaaccaggtgtggaaagtccccaggctccccagcaggcagaagtatgcaaagcatgcatctcaattagtcagcaaccatagtcccgcccctaactccgcccatcccgcccctaactccgcccagttccgcccattctccgccccatggctgactaattttttttatttatgcagaggccgaggccgcctctgcctctgagctattccagaagtagtgaggaggcttttttggaggcctaggcttttgcaaaaagctcccgggagcttgtatatccattttcggatctgatcaagagacaggatgaggatcgtttcgcatgattgaacaagatggattgcacgcaggttctccggccgcttgggtggagaggctattcggctatgactgggcacaacagacaatcggctgctctgatgccgccgtgttccggctgtcagcgcaggggcgcccggttctttttgtcaagaccgacctgtccggtgccctgaatgaactgcaggacgaggcagcgcggctatcgtggctggccacgacgggcgttccttgcgcagctgtgctcgacgttgtcactgaagcgggaagggactggctgctattgggcgaagtgccggggcaggatctcctgtcatctcaccttgctcctgccgagaaagtatccatcatggctgatgcaatgcggcggctgcatacgcttgatccggctacctgcccattcgaccaccaagcgaaacatcgcatcgagcgagcacgtactcggatggaagccggtcttgtcgatcaggatgatctggacgaagagcatcaggggctcgcgccagccgaactgttcgccaggctcaaggcgcgcatgcccgacggcgaggatctcgtcgtgacccatggcgatgcctgcttgccgaatatcatggtggaaaatggccgcttttctggattcatcgactgtggccggctgggtgtggcggaccgctatcaggacatagcgttggctacccgtgatattgctgaagagcttggcggcgaatgggctgaccgcttcctcgtgctttacggtatcgccgctcccgattcgcagcgcatcgccttctatcgccttcttgacgagttcttctgagcgggactctggggttcgaaatgaccgaccaagcgacgcccaacctgccatcacgagatttcgattccaccgccgccttctatgaaaggttgggcttcggaatcgttttccgggacgccggctggatgatcctccagcgcggggatctcatgctggagttcttcgcccaccccaacttgtttattgcagcttataatggttacaaataaagcaatagcatcacaaatttcacaaataaagcatttttttcactgcattctagttgtggtttgtccaaactcatcaatgtatcttatcatgtctgtataccgtcgacctctagctagagcttggcgtaatcatggtcatagctgtttcctgtgtgaaattgttatccgctcacaattccacacaacatacgagccggaagcataaagtgtaaagcctggggtgcctaatgagtgagctaactcacattaattgcgttgcgctcactgcccgctttccagtcgggaaacctgtcgtgccagctgcattaatgaatcggccaacgcgcggggagaggcggtttgcgtattgggcgctcttccgcttcctcgctcactgactcgctgcgctcggtcgttcggctgcggcgagcggtatcagctcactcaaaggcggtaatacggttatccacagaatcaggggataacgcaggaaagaacatgtgagcaaaaggccagcaaaaggccaggaaccgtaaaaaggccgcgttgctggcgtttttccataggctccgcccccctgacgagcatcacaaaaatcgacgctcaagtcagaggtggcgaaacccgacaggactataaagataccaggcgtttccccctggaagctccctcgtgcgctctcctgttccgaccctgccgcttaccggatacctgtccgcctttctcccttcgggaagcgtggcgctttctcaatgctcacgctgtaggtatctcagttcggtgtaggtcgttcgctccaagctgggctgtgtgcacgaaccccccgttcagcccgaccgctgcgccttatccggtaactatcgtcttgagtccaacccggtaagacacgacttatcgccactggcagcagccactggtaacaggattagcagagcgaggtatgtaggcggtgctacagagttcttgaagtggtggcctaactacggctacactagaaggacagtatttggtatctgcgctctgctgaagccagttaccttcggaaaaagagttggtagctcttgatccggcaaacaaaccaccgctggtagcggtggtttttttgtttgcaagcagcagattacgcgcagaaaaaaaggatctcaagaagatcctttgatcttttctacggggtctgacgctcagtggaacgaaaactcacgttaagggattttggtcatgagattatcaaaaaggatcttcacctagatccttttaaattaaaaatgaagttttaaatcaatctaaagtatatatgagtaaacttggtctgacagttaccaatgcttaatcagtgaggcacctatctcagcgatctgtctatttcgttcatccatagttgcctgactccccgtcgtgtagataactacgatacgggagggcttaccatctggccccagtgctgcaatgataccgcgagacccacgctcaccggctccagatttatcagcaataaaccagccagccggaagggccgagcgcagaagtggtcctgcaactttatccgcctccatccagtctattaattgttgccgggaagctagagtaagtagttcgccagttaatagtttgcgcaacgttgttgccattgctacaggcatcgtggtgtcacgctcgtcgtttggtatggcttcattcagctccggttcccaacgatcaaggcgagttacatgatcccccatgttgtgcaaaaaagcggttagctccttcggtcctccgatcgttgtcagaagtaagttggccgcagtgttatcactcatggttatggcagcactgcataattctcttactgtcatgccatccgtaagatgcttttctgtgactggtgagtactcaaccaagtcattctgagaatagtgtatgcggcgaccgagttgctcttgcccggcgtcaatacgggataataccgcgccacatagcagaactttaaaagtgctcatcattggaaaacgttcttcggggcgaaaactctcaaggatcttaccgctgttgagatccagttcgatgtaacccactcgtgcacccaactgatcttcagcatcttttactttcaccagcgtttctgggtgagcaaaaacaggaaggcaaaatgccgcaaaaaagggaataagggcgacacggaaatgttgaatactcatactcttcctttttcaatattattgaagcatttatcagggttattgtctcatgagcggatacatatttgaatgtatttagaaaaataaacaaataggggttccgcgcacatttccccgaaaagtgccacctgacgtc

SEQ ID NO: 65 - protein, 4 aa, artificial
  motif
  VARIANT (2)..(2): aliphatic amino acid
  VARIANT (3)..(3): aliphatic amino acid
  VARIANT (4)..(4): C-terminal amino acid
CXXX